European Patent Application EP 4 549 454 A2, published May 7, 2025. Title: GIP/GLP1 CO-AGONIST COMPOUNDS. Applicant: Eli Lilly and Company. Application JP 2023-145813, filed July 22, 2019. The sequence listing filed with the application follows.

SEQUENCE LISTING (396 sequences)

SEQ ID NO: 1 - protein, 42 aa, Homo sapiens
YAEGTFISDYSIAMDKIHQQDFVNWLLAQKGKKNDWKHNITQ

SEQ ID NO: 2 - protein, 30 aa, Homo sapiens
  MOD_RES 30: note = AMIDATION
HAEGTFTSDVSSYLEGQAAKEFIAWLVKGR

SEQ ID NO: 3 - protein, 31 aa, synthetic construct
  REGION 1..31: note = Synthetic construct; Formula I
  VARIANT 1: note = Xaa at position 1 is selected from the group consisting of Y, H, D-Tyr, F, desH, and desY, or Xaa at position 1 and Xaa at position 2 combine to form desH-psi[NHCO]-Aib
  MOD_RES 1: note = The N-terminus of Xaa at position 1 is modified with R1, wherein the modification is selected from the group consisting of Ac and absent.
  VARIANT 2: note = Xaa at position 2 is selected from the group consisting of Aib, alpha-MeP, A, P, and D-Ala, or Xaa at position 1 combines with Xaa at position 2 to form desH-psi[NHCO]-Aib
  VARIANT 3: note = Xaa at position 3 is selected from the group of E, N, Aad, and cTA
  VARIANT 6: note = Xaa at position 6 is selected from the group consisting of F, alpha-MeF, and alpha-MeF(2F)
  VARIANT 10: note = Xaa at position 10 is selected from the group consisting of A, L, H, 3Pal, 4Pal, V, Y, E, alpha-MeF, alpha-MeF(2F), I, alpha-MeY, Q, D-His, D-Tyr, cTA, and K
  VARIANT 10: note = when Xaa at position 10 is K, then K is chemically modified by conjugation of the epsilon-amino group of the K side chain with (2-[2-(2-amino-ethoxy)-ethoxy]-acetyl)2-(gamma-Glu)-CO-(CH2)q-CO2 H
  REGION 10..31: note = MISC_FEATURE - When Xaa is K(2-[2-(2-amino-ethoxy)-ethoxy]-acetyl)2-(gamma-Glu)-CO-(CH2)q-CO 2H at positions 10, 12, 13, 14, 16, 17, 19, 20, 21, 23, 24, 26, 27, 28, 29, 30 or 31, q is 14, 15, 16, 17, 18, 19 or 20.
  VARIANT 11: note = Xaa at position 11 is selected from the group consisting of S, alpha-MeS, or D-Ser
  VARIANT 12: note = Xaa at position 12 is selected from the group consisting of I, S, D-Ile, and K
  MOD_RES 12: note = when Xaa at position 12 is K, then K is chemically modified by conjugation of the epsilon-amino group of the K side chain with (2-[2-(2-amino-ethoxy)-ethoxy]-acetyl)2-(gamma-Glu)-CO-(CH2)q-CO2 H
  VARIANT 13: note = Xaa at position 13 is selected from the group consisting of Nle, Aib, L, alpha-MeL, and K
  MOD_RES 13: note = when Xaa at position 13 is K, then K is chemically modified by conjugation of the epsilon-amino group of the K side chain with (2-[2-(2-amino-ethoxy)-ethoxy]-acetyl)2-(gamma-Glu)-CO-(CH2)q-CO2 H
  VARIANT 14: note = Xaa at position 14 is selected from the group consisting of L and K, wherein K is conjugated to a C16-C22 fatty acid wherein said fatty acid is optionally conjugated to said K via a linker
  VARIANT 16: note = Xaa at position 16 is selected from the group consisting of E, Orn, Dab, Dap, S, T, H, Aib, alpha-MeK, R, and K
  MOD_RES 16: note = when Xaa at position 16 is K, then K is optionally chemically modified by conjugation of the epsilon-amino group of the K side chain with (2-[2-(2-amino-ethoxy)-ethoxy]-acetyl)2 -(gamma-Glu)-CO-(CH2)q-CO2H
  VARIANT 17: note = Xaa at position 17 is selected from the group consisting of K, Q, I, and an amino acid conjugated to a C16-C22 fatty acid wherein said fatty acid is optionally conjugated to said amino acid via a linker
  VARIANT 19: note = Xaa at position 19 is selected from the group consisting of Q, A, and K
  MOD_RES 19: note = when Xaa at position 19 is K, then K is chemically modified by conjugation of the epsilon-amino group of the K side chain with (2-[2-(2-amino-ethoxy)-ethoxy]-acetyl)2 -(gamma-Glu)-CO-(CH2)q-CO2H
  VARIANT 20: note = Xaa at position 20 is selected from the group consisting of Aib, Q, H, R, K, and alpha-MeK
  MOD_RES 20: note = when Xaa at position 20 is K, then K is optionally chemically modified by conjugation of the epsilon-amino group of the K side chain with (2-[2-(2-amino-ethoxy)-ethoxy]-acetyl)2 -(gamma-Glu)-CO-(CH2)q-CO2H
  VARIANT 21: note = Xaa at position 21 is selected from the group consisting of H, Aad, D, Aib, T, A, E, I, and K
  MOD_RES 21: note = when Xaa at position 21 is K, then K is chemically modified by conjugation of the epsilon-amino group of the K side chain with K(2-[2-(2-amino-ethoxy)-ethoxy]-acetyl)2-(gamma-Glu)-CO-(CH2)q-CO 2H
  VARIANT 22: note = Xaa at position 22 is selected from the group consisting of F and alpha-MeF
  VARIANT 23: note = Xaa at position 23 is selected from the group consisting of I, L, A, G, F, H, E, V, and K
  MOD_RES 23: note = when Xaa at position 23 is K, then K is chemically modified by conjugation of the epsilon-amino group of the K side chain with K(2-[2-(2-amino-ethoxy)-ethoxy]-acetyl)2-(gamma-Glu)-CO-(CH2)q-CO 2H
  VARIANT 24: note = Xaa at position 24 is selected from the group consisting of S, Aad, D-Glu, E, Aib, H, V, A, Q, D, P, and K
  MOD_RES 24: note = when Xaa at position 24 is K, then K is chemically modified by conjugation of the epsilon-amino group of the K side chain with K(2-[2-(2-amino-ethoxy)-ethoxy]-acetyl)2-(gamma-Glu)-CO-(CH2)q-CO 2H
  VARIANT 25: note = Xaa at position 25 is selected from the group consisting of Y or alpha-MeY
  VARIANT 26: note = Xaa at position 26 is selected from the group consisting of L, alpha-MeL, and K
  MOD_RES 26: note = when Xaa at position 26 is K, then K is chemically modified by conjugation of the epsilon-amino group of the K side chain with (2-[2-(2-amino-ethoxy)-ethoxy]-acetyl)2-(gamma-Glu)-CO-(CH2)q-CO2 H
  VARIANT 27: note = Xaa at position 27 is selected from the group consisting of L, I, and K
  MOD_RES 27: note = when Xaa at position 27 is K, then K is chemically modified by conjugation of the epsilon-amino group of the K side chain with (2-[2-(2-amino-ethoxy)-ethoxy]-acetyl)2-(gamma-Glu)-CO-(CH2)q-CO2 H
  VARIANT 28: note = Xaa at position 28 is selected from the group consisting of E, A, S, D-Glu, and K
  MOD_RES 28: note = when Xaa at position 28 is K, then K is chemically modified by conjugation of the epsilon-amino group of the K side chain with (2-[2-(2-amino-ethoxy)-ethoxy]-acetyl)2-(gamma-Glu)-CO-(CH2)q-CO2 H
  VARIANT 29: note = Xaa at position 29 is selected from the group consisting of Aib, G, A, and K
  MOD_RES 29: note = when Xaa at position 29 is K, then K is chemically modified by conjugation of the epsilon-amino group of the K side chain with (2-[2-(2-amino-ethoxy)-ethoxy]-acetyl)2-(gamma-Glu)-CO-(CH2)q-CO2 H
  VARIANT 30: note = Xaa at position 30 is selected from the group consisting of C, G, G-R2, and K, wherein R2 is a modification of the C-terminal group, wherein the modification is NH2 or absent, wherein if X30 is G-R2, then X31 is absent.
  MOD_RES 30: note = when Xaa at position 30 is K, then K is chemically modified by conjugation of the epsilon-amino group of the K side chain with (2-[2-(2-amino-ethoxy)-ethoxy]-acetyl)2-(gamma-Glu)-CO-(CH2)q-CO2 H
  VARIANT 31: note = Xaa at position 31 is absent or is selected from the group consisting of SEQ ID NO:4, SEQ ID NO:5, SEQ ID:6, SEQ ID NO:7, SEQ ID NO:8, and SEQ ID NO:9
  SITE 31: note = MISC_FEATURE - wherein no more than one of X10, X12, X13, X14, X16, X17, X19, X20, X21, X23, X24, X26, X27, X28, X29, X30, X31, X32, X33, X34, X35, X36, X37, X38, X39, and X40 may be a substituent that contains a fatty acid
  SITE 31: note = MISC_FEATURE - wherein no more than one of X30, X34, X39, and X40 may be C
  SITE 31: note = MISC_FEATURE - wherein if one of X30, X34, X39, and X40 is C, then none of X10, X12, X13, X14, X16, X17, X19, X20, X21, X23, X24, X26, X27, X28, X29, X30, X31, X32, X33, X34, X35, X36, X37, X38, X39, and X40 is a substituent that contains a fatty acid
  MOD_RES 31: note = Xaa at position 31 is modified with R2, wherein the modification is NH2 to form a C-terminal amide or absent
XXXGTXTSDXXXXXDXXAXXXXXXXXXXXXX

SEQ ID NO: 4-9 - skipped (6 entries)

SEQ ID NO: 10 - protein, 39 aa, synthetic construct
  REGION 1..39: note = Synthetic Construct
  SITE 2: note = MISC_FEATURE - Xaa at position 2 is Aib
  SITE 6: note = MISC_FEATURE - Xaa at position 6 is alpha-MeF(2F)
  SITE 13: note = MISC_FEATURE - Xaa at position 13 is alpha-MeL
  MOD_RES 17: note = K at position 17 is chemically modified by conjugation of the epsilon-amino group of the K side chain with (2-[2-(2-amino-ethoxy)-ethoxy]-acetyl)2-(gamma-Glu)-CO-(CH2)18-CO 2H
  SITE 20: note = MISC_FEATURE - Xaa at position 20 is Aib
  SITE 24: note = MISC_FEATURE - Xaa at position 24 is D-Glu
  MOD_RES 39: note = The Serine at position 39 is amidated
YXEGTXTSDYSIXLDEKAQXEFIXYLIEGGPSSGAPPPS

SEQ ID NO: 11 - protein, 39 aa, synthetic construct
  REGION 1..39: note = Synthetic Construct
  SITE 2: note = MISC_FEATURE - Xaa at position 2 is Aib
  SITE 6: note = MISC_FEATURE - Xaa at position 6 is alpha-MeF(2F)
  SITE 13: note = MISC_FEATURE - Xaa at position 13 is alpha-MeL
  SITE 16: note = MISC_FEATURE - Xaa at position 16 is Orn
  MOD_RES 17: note = K at position 17 is chemically modified by conjugation of the epsilon-amino group of the K side chain with (2-[2-(2-amino-ethoxy)-ethoxy]-acetyl)2-(gamma-Glu)-CO-(CH2)16-CO 2H
  SITE 20: note = MISC_FEATURE - Xaa at position 20 is Aib
  SITE 24: note = MISC_FEATURE - Xaa at position 24 is D-Glu
  MOD_RES 39: note = The Serine at position 39 is amidated
YXEGTXTSDYSIXLDXKAQXEFIXYLIEGGPSSGAPPPS

SEQ ID NO: 12 - protein, 39 aa, synthetic construct; identical to SEQ ID NO: 11
  REGION 1..39: note = Synthetic Construct
  SITE 2: note = MISC_FEATURE - Xaa at position 2 is Aib
  SITE 6: note = MISC_FEATURE - Xaa at position 6 is alpha-MeF(2F)
  SITE 13: note = MISC_FEATURE - Xaa at position 13 is alpha-MeL
  SITE 16: note = MISC_FEATURE - Xaa at position 16 is Orn
  MOD_RES 17: note = K at position 17 is chemically modified by conjugation of the epsilon-amino group of the K side chain with (2-[2-(2-amino-ethoxy)-ethoxy]-acetyl)2-(gamma-Glu)-CO-(CH2)18-CO 2H
  SITE 20: note = MISC_FEATURE - Xaa at position 20 is Aib
  SITE 24: note = MISC_FEATURE - Xaa at position 24 is D-Glu
  SITE 39: note = MISC_FEATURE - The Serine at position 39 is amidated

SEQ ID NO: 13 - protein, 39 aa, synthetic construct
  REGION 1..39: note = Synthetic Construct
  SITE 2: note = MISC_FEATURE - Xaa at position 2 is Aib
  SITE 6: note = MISC_FEATURE - Xaa at position 6 is alpha-MeF(2F)
  SITE 10: note = MISC_FEATURE - Xaa at position 10 is 4Pal
  SITE 13: note = MISC_FEATURE - Xaa at position 13 is alpha-MeL
  SITE 16: note = MISC_FEATURE - Xaa at position 16 is Orn
  MOD_RES 17: note = K at position 17 is chemically modified by conjugation of the epsilon-amino group of the K side chain with (2-[2-(2-amino-ethoxy)-ethoxy]-acetyl)2-(gamma-Glu)-CO-(CH2)16-CO 2H
  SITE 20: note = MISC_FEATURE - Xaa at position 20 is Aib
  SITE 24: note = MISC_FEATURE - Xaa at position 24 is D-Glu
  SITE 25: note = MISC_FEATURE - Xaa at position 25 is alpha-MeY
  MOD_RES 39: note = The Serine at position 39 is amidated
YXEGTXTSDXSIXLDXKAQXEFIXXLIEGGPSSGAPPPS

SEQ ID NO: 14 - protein, 39 aa, synthetic construct
  REGION 1..39: note = Synthetic Construct
  SITE 2: note = MISC_FEATURE - Xaa at position 2 is Aib
  SITE 6: note = MISC_FEATURE - Xaa at position 6 is alpha-MeF(2F)
  SITE 13: note = MISC_FEATURE - Xaa at position 13 is alpha-MeL
  SITE 16: note = MISC_FEATURE - Xaa at position 16 is Orn
  MOD_RES 17: note = K at position 17 is chemically modified by conjugation of the epsilon-amino group of the K side chain with (2-[2-(2-amino-ethoxy)-ethoxy]-acetyl)2-(gamma-Glu)-CO-(CH2)16-CO 2H
  SITE 20: note = MISC_FEATURE - Xaa at position 20 is Aib
  SITE 24: note = MISC_FEATURE - Xaa at position 24 is D-Glu
  SITE 25: note = MISC_FEATURE - Xaa at position 25 is alpha-MeY
  MOD_RES 39: note = The Serine at position 39 is amidated
YXEGTXTSDVSIXLDXKAQXEFIXXLIEGGPSSGAPPPS

SEQ ID NO: 15 - protein, 39 aa, synthetic construct
  REGION 1..39: note = Synthetic Construct
  SITE 2: note = MISC_FEATURE - Xaa at position 2 is Aib
  MOD_RES 17: note = Lys at position 17 is chemically modified by conjugation of the epsilon-amino group of the Lys side chain with (2-[2-(2-amino-ethoxy)-ethoxy]-acetyl)2-(gamma-Glu)-CO-(CH2)18-CO 2H
  SITE 20: note = MISC_FEATURE - Xaa at position 20 is Aib
  MOD_RES 39: note = Ser at position 39 is amidated
YXEGTFTSDYSILLDKKAQXAFIEYLLEGGPSSGAPPPS

SEQ ID NO: 16 - protein, 39 aa, synthetic construct
  REGION 1..39: note = Synthetic Construct
  SITE 2: note = MISC_FEATURE - Xaa at position 2 is Aib
  MOD_RES 17: note = Lys at position 17 is chemically modified by conjugation of the epsilon-amino group of the Lys side chain with (2-[2-(2-amino-ethoxy)-ethoxy]-acetyl)2-(gamma-Glu)-CO-(CH2)18-CO 2H
  SITE 20: note = MISC_FEATURE - Xaa at position 20 is Aib
  MOD_RES 39: note = Ser at position 39 is amidated
YXEGTFTSDYSILLDSKAQXAFIEYLLEGGPSSGAPPPS

SEQ ID NO: 17 - protein, 39 aa, synthetic construct
  REGION 1..39: note = Synthetic Construct
  SITE 2: note = MISC_FEATURE - Xaa at position 2 is Aib
  MOD_RES 17: note = Lys at position 17 is chemically modified by conjugation of the epsilon-amino group of the Lys side chain with (2-[2-(2-amino-ethoxy)-ethoxy]-acetyl)2-(gamma-Glu)-CO-(CH2)18-CO 2H
  SITE 20: note = MISC_FEATURE - Xaa at position 20 is Aib
  MOD_RES 39: note = Ser at position 39 is amidated
YXEGTFTSDYSILLDKKAQXAFIEYLIEGGPSSGAPPPS

SEQ ID NO: 18 - protein, 39 aa, synthetic construct
  REGION 1..39: note = Synthetic Construct
  SITE 2: note = MISC_FEATURE - Xaa at position 2 is Aib
  MOD_RES 17: note = Lys at position 17 is chemically modified by conjugation of the epsilon-amino group of the Lys side chain with (2-[2-(2-amino-ethoxy)-ethoxy]-acetyl)2-(gamma-Glu)-CO-(CH2)18-CO 2H
  SITE 20: note = MISC_FEATURE - Xaa at position 20 is Aib
  MOD_RES 39: note = Ser at position 39 is amidated
YXEGTFTSDYSILLDSKAQXAFIEYLIEGGPSSGAPPPS

SEQ ID NO: 19 - protein, 39 aa, synthetic construct
  REGION 1..39: note = Synthetic Construct
  SITE 2: note = MISC_FEATURE - Xaa at position 2 is Aib
  SITE 20: note = MISC_FEATURE - Xaa at position 20 is Aib
  MOD_RES 24: note = Lys at position 24 is chemically modified by conjugation of the epsilon-amino group of the Lys side chain with (2-[2-(2-amino-ethoxy)-ethoxy]-acetyl)2-(gamma-Glu)-CO-(CH2)18-CO 2H
  SITE 29: note = MISC_FEATURE - Xaa at position 29 is Aib
  MOD_RES 39: note = Ser at position 39 is amidated
YXEGTFTSDYSILLDSIAQXAFIKYLLAXGPSSGAPPPS

SEQ ID NO: 20 - protein, 39 aa, synthetic construct
  REGION 1..39: note = Synthetic Construct
  SITE 2: note = MISC_FEATURE - Xaa at position 2 is Aib
  SITE 20: note = MISC_FEATURE - Xaa at position 20 is Aib
  MOD_RES 28: note = Lys at position 28 is chemically modified by conjugation of the epsilon-amino group of the Lys side chain with (2-[2-(2-amino-ethoxy)-ethoxy]-acetyl)2-(gamma-Glu)-CO-(CH2)18-CO 2H
  SITE 29: note = MISC_FEATURE - Xaa at position 29 is Aib
  MOD_RES 39: note = Ser at position 39 is amidated
YXEGTFTSDYSILLDSIAQXAFIEYLLKXGPSSGAPPPS

SEQ ID NO: 21 - protein, 39 aa, synthetic construct
  REGION 1..39: note = Synthetic Construct
  SITE 2: note = MISC_FEATURE - Xaa at position 2 is Aib
  MOD_RES 20: note = Lys at position 20 is chemically modified by conjugation of the epsilon-amino group of the Lys side chain with (2-[2-(2-amino-ethoxy)-ethoxy]-acetyl)2-(gamma-Glu)-CO-(CH2)18-CO 2H
  MOD_RES 39: note = Ser at position 39 is amidated
YXEGTFTSDYSILLDKIAQKAFIEYLIEGGPSSGAPPPS

SEQ ID NO: 22 - protein, 39 aa, synthetic construct
  REGION 1..39: note = Synthetic Construct
  SITE 2: note = MISC_FEATURE - Xaa at position 2 is Aib
  SITE 16: note = MISC_FEATURE - Xaa at position 16 is Aib
  MOD_RES 20: note = Lys at position 20 is chemically modified by conjugation of the epsilon-amino group of the Lys side chain with (2-[2-(2-amino-ethoxy)-ethoxy]-acetyl)2-(gamma-Glu)-CO-(CH2)18-CO 2H
  MOD_RES 39: note = Ser at position 39 is amidated
YXEGTFTSDYSILLDXIAQKAFIEYLIEGGPSSGAPPPS

SEQ ID NO: 23 - protein, 39 aa, synthetic construct
  REGION 1..39: note = Synthetic Construct
  SITE 2: note = MISC_FEATURE - Xaa at position 2 is Aib
  MOD_RES 20: note = Lys at position 20 is chemically modified by conjugation of the epsilon-amino group of the Lys side chain with (2-[2-(2-amino-ethoxy)-ethoxy]-acetyl)2-(gamma-Glu)-CO-(CH2)18-CO 2H
  SITE 29: note = MISC_FEATURE - Xaa at position 29 is Aib
  MOD_RES 39: note = Ser at position 39 is amidated
YXEGTFTSDYSILLDKIAQKEFIQYLLEXGPSSGAPPPS

SEQ ID NO: 24 - protein, 39 aa, synthetic construct
  REGION 1..39: note = Synthetic Construct
  SITE 2: note = MISC_FEATURE - Xaa at position 2 is Aib
  MOD_RES 17: note = Lys at position 17 is chemically modified by conjugation of the epsilon-amino group of the Lys side chain with (2-[2-(2-amino-ethoxy)-ethoxy]-acetyl)2-(gamma-Glu)-CO-(CH2)18-CO 2H
  SITE 20: note = MISC_FEATURE - Xaa at position 20 is Aib
  SITE 29: note = MISC_FEATURE - Xaa at position 29 is Aib
  MOD_RES 39: note = Ser at position 39 is amidated
HXEGTFTSDYSILLDKKAQXAFIEYLLEXGPSSGAPPPS

SEQ ID NO: 25 - protein, 39 aa, synthetic construct
  REGION 1..39: note = Synthetic Construct
  SITE 2: note = MISC_FEATURE - Xaa at position 2 is Aib
  MOD_RES 17: note = Lys at position 17 is chemically modified by conjugation of the epsilon-amino group of the Lys side chain with (2-[2-(2-amino-ethoxy)-ethoxy]-acetyl)2-(gamma-Glu)-CO-(CH2)18-CO 2H
  SITE 20: note = MISC_FEATURE - Xaa at position 20 is Aib
  SITE 29: note = MISC_FEATURE - Xaa at position 29 is Aib
  MOD_RES 39: note = Ser at position 39 is amidated
HXEGTFTSDYSILLDKKAQXAFIEYLIEXGPSSGAPPPS

SEQ ID NO: 26 - protein, 34 aa, synthetic construct
  REGION 1..34: note = Synthetic Construct
  SITE 2: note = MISC_FEATURE - Xaa at position 2 is Aib
  MOD_RES 20: note = Lys at position 20 is chemically modified by conjugation of the epsilon-amino group of the Lys side chain with (2-[2-(2-amino-ethoxy)-ethoxy]-acetyl)2-(gamma-Glu)-CO-(CH2)18-CO 2H
  SITE 29: note = MISC_FEATURE - Xaa at position 29 is Aib
  MOD_RES 34: note = Ser at position 34 is amidated
HXEGTFTSDYSILLDKIAQKAFIEYLLEXGPSSG

SEQ ID NO: 27 - protein, 39 aa, synthetic construct
  REGION 1..39: note = Synthetic Construct
  SITE 2: note = MISC_FEATURE - Xaa at position 2 is Aib
  SITE 13: note = MISC_FEATURE - Xaa at position 13 is alpha-methyl-L
  MOD_RES 17: note = Lys at position 17 is chemically modified by conjugation of the epsilon-amino group of the Lys side chain with Dab-(2-[2-(2-Amino-ethoxy)-ethoxy]-acetyl)-Dab-(2-[2-(2-Amino-eth oxy)-ethoxy]-acetyl)-CO-(CH2)18-CO2H
  SITE 20: note = MISC_FEATURE - Xaa at position 20 is alpha-methyl-Lys
  SITE 29: note = MISC_FEATURE - Xaa at position 29 is Aib
  MOD_RES 39: note = Ser at position 39 is amidated
HXEGTFTSDYSIXLDKKAQXAFIQYLLAXGPSSGAPKPS

SEQ ID NO: 28 - protein, 39 aa, synthetic construct
  REGION 1..39: note = Synthetic Construct
  SITE 2: note = MISC_FEATURE - Xaa at position 2 is Aib
  SITE 13: note = MISC_FEATURE - Xaa at position 13 is alpha-methyl-Leu
  MOD_RES 17: note = Lys at position 17 is chemically modified by conjugation of the epsilon-amino group of the Lys side chain with Dab-(2-[2-(2-Amino-ethoxy)-ethoxy]-acetyl)-Dab-(2-[2-(2-Amino-eth oxy)-ethoxy]-acetyl)-CO-(CH2)18-CO2H
  SITE 20: note = MISC_FEATURE - Xaa at position 20 is alpha-methyl-Lys
  SITE 29: note = MISC_FEATURE - Xaa at position 29 is Aib
  MOD_RES 39: note = Ser at position 39 is amidated
HXEGTFTSDYSIXLDKKAQXAFIQYLLAXGPSSGAPPPS

SEQ ID NO: 29 - protein, 39 aa, synthetic construct
  REGION 1..39: note = Synthetic Construct
  SITE 2: note = MISC_FEATURE - Xaa at position 2 is Aib
  SITE 13: note = MISC_FEATURE - Xaa at position 13 is alpha-methyl-Leu
  MOD_RES 17: note = Lys at position 17 is chemically modified by conjugation of the epsilon-amino group of the Lys side chain with (2-[2-(2-amino-ethoxy)-ethoxy]-acetyl)2-(gamma-Glu)-CO-(CH2)18-CO 2H
  SITE 20: note = MISC_FEATURE - Xaa at position 20 is Aib
  MOD_RES 39: note = Ser at position 39 is amidated
YXEGTFTSDYSIXLDKKAQXAFIEYLIEGGPSSGAPPPS

SEQ ID NO: 30 - protein, 39 aa, synthetic construct
  REGION 1..39: note = Synthetic Construct
  SITE 2: note = MISC_FEATURE - Xaa at position 2 is Aib
  SITE 13: note = MISC_FEATURE - Xaa at position 13 is alpha-methyl-Leu
  MOD_RES 17: note = Lys at position 17 is chemically modified by conjugation of the epsilon-amino group of the Lys side chain with (2-[2-(2-amino-ethoxy)-ethoxy]-acetyl)2-(gamma-Glu)-CO-(CH2)18-CO 2H
  SITE 20: note = MISC_FEATURE - Xaa at position 20 is alpha-methyl-Lys
  MOD_RES 39: note = Ser at position 39 is amidated
YXEGTFTSDYSIXLDEKAQXAFIEYLLEGGPSSGAPPPS

SEQ ID NO: 31 - protein, 39 aa, synthetic construct
  REGION 1..39: note = Synthetic Construct
  SITE 2: note = MISC_FEATURE - Xaa at position 2 is Aib
  SITE 13: note = MISC_FEATURE - Xaa at position 13 is alpha-methyl-Leu
  MOD_RES 17: note = Lys at position 17 is chemically modified by conjugation of the epsilon-amino group of the Lys side chain with (2-[2-(2-amino-ethoxy)-ethoxy]-acetyl)2-(gamma-Glu)-CO-(CH2)18-CO 2H
  SITE 20: note = MISC_FEATURE - Xaa at position 20 is alpha-methyl-Lys
  SITE 29: note = MISC_FEATURE - Xaa at position 29 is Aib
  MOD_RES 39: note = Ser at position 39 is amidated
YXEGTFTSDYSIXLDEKAQXAFIEYLLEXGPSSGAPPPS

SEQ ID NO: 32 - protein, 39 aa, synthetic construct
  REGION 1..39: note = Synthetic Construct
  SITE 2: note = MISC_FEATURE - Xaa at position 2 is Aib
  MOD_RES 10: note = Lys at position 10 is chemically modified by conjugation of the epsilon-amino group of the Lys side chain with (2-[2-(2-amino-ethoxy)-ethoxy]-acetyl)2-(gamma-Glu)-CO-(CH2)18-CO 2H
  SITE 20: note = MISC_FEATURE - Xaa at position 20 is Aib
  MOD_RES 39: note = Ser at position 39 is amidated
YXEGTFTSDKSILLDKIAQXAFIEYLIEGGPSSGAPPPS

SEQ ID NO: 33 - protein, 39 aa, synthetic construct
  REGION 1..39: note = Synthetic Construct
  SITE 2: note = MISC_FEATURE - Xaa at position 2 is Aib
  MOD_RES 11: note = Lys at position 11 is chemically modified by conjugation of the epsilon-amino group of the Lys side chain with (2-[2-(2-amino-ethoxy)-ethoxy]-acetyl)2-(gamma-Glu)-CO-(CH2)18-CO 2H
  SITE 20: note = MISC_FEATURE - Xaa at position 20 is Aib
  MOD_RES 39: note = Ser at position 39 is amidated
YXEGTFTSDYKILLDKIAQXAFIEYLIEGGPSSGAPPPS

SEQ ID NO: 34 - protein, 39 aa, synthetic construct
  REGION 1..39: note = Synthetic Construct
  SITE 2: note = MISC_FEATURE - Xaa at position 2 is Aib
  MOD_RES 12: note = Lys at position 12 is chemically modified by conjugation of the epsilon-amino group of the Lys side chain with (2-[2-(2-amino-ethoxy)-ethoxy]-acetyl)2-(gamma-Glu)-CO-(CH2)18-CO 2H
  SITE 20: note = MISC_FEATURE - Xaa at position 20 is Aib
  MOD_RES 39: note = Ser at position 39 is amidated
YXEGTFTSDYSKLLDKIAQXAFIEYLIEGGPSSGAPPPS

SEQ ID NO: 35 - protein, 39 aa, synthetic construct
  REGION 1..39: note = Synthetic Construct
  SITE 2: note = MISC_FEATURE - Xaa at position 2 is Aib
  MOD_RES 13: note = Lys at position 13 is chemically modified by conjugation of the epsilon-amino group of the Lys side chain with (2-[2-(2-amino-ethoxy)-ethoxy]-acetyl)2-(gamma-Glu)-CO-(CH2)18-CO 2H
  SITE 20: note = MISC_FEATURE - Xaa at position 20 is Aib
  MOD_RES 39: note = Ser at position 39 is amidated
YXEGTFTSDYSIKLDKIAQXAFIEYLIEGGPSSGAPPPS

SEQ ID NO: 36 - protein, 39 aa, synthetic construct
  REGION 1..39: note = Synthetic Construct
  SITE 2: note = MISC_FEATURE - Xaa at position 2 is Aib
  MOD_RES 14: note = Lys at position 14 is chemically modified by conjugation of the epsilon-amino group of the Lys side chain with (2-[2-(2-amino-ethoxy)-ethoxy]-acetyl)2-(gamma-Glu)-CO-(CH2)18-CO 2H
  SITE 20: note = MISC_FEATURE - Xaa at position 20 is Aib
  MOD_RES 39: note = Ser at position 39 is amidated
YXEGTFTSDYSILKDKIAQXAFIEYLIEGGPSSGAPPPS

SEQ ID NO: 37 - protein, 39 aa, synthetic construct
  REGION 1..39: note = Synthetic Construct
  SITE 2: note = MISC_FEATURE - Xaa at position 2 is Aib
  MOD_RES 15: note = Lys at position 15 is chemically modified by conjugation of the epsilon-amino group of the Lys side chain with (2-[2-(2-amino-ethoxy)-ethoxy]-acetyl)2-(gamma-Glu)-CO-(CH2)18-CO 2H
  SITE 20: note = MISC_FEATURE - Xaa at position 20 is Aib
  MOD_RES 39: note = Ser at position 39 is amidated
YXEGTFTSDYSILLKKIAQXAFIEYLIEGGPSSGAPPPS

SEQ ID NO: 38 - protein, 39 aa, synthetic construct
  REGION 1..39: note = Synthetic Construct
  SITE 2: note = MISC_FEATURE - Xaa at position 2 is Aib
  MOD_RES 16: note = Lys at position 16 is chemically modified by conjugation of the epsilon-amino group of the Lys side chain with (2-[2-(2-amino-ethoxy)-ethoxy]-acetyl)2-(gamma-Glu)-CO-(CH2)18-CO 2H
  SITE 20: note = MISC_FEATURE - Xaa at position 20 is Aib
  MOD_RES 39: note = Ser at position 39 is amidated
YXEGTFTSDYSILLDKIAQXAFIEYLIEGGPSSGAPPPS

SEQ ID NO: 39 - protein, 39 aa, synthetic construct
  REGION 1..39: note = Synthetic Construct
  SITE 2: note = MISC_FEATURE - Xaa at position 2 is Aib
  MOD_RES 18: note = Lys at position 18 is chemically modified by conjugation of the epsilon-amino group of the Lys side chain with (2-[2-(2-amino-ethoxy)-ethoxy]-acetyl)2-(gamma-Glu)-CO-(CH2)18-CO 2H
  SITE 20: note = MISC_FEATURE - Xaa at position 20 is Aib
  MOD_RES 39: note = Ser at position 39 is amidated
YXEGTFTSDYSILLDKIKQXAFIEYLIEGGPSSGAPPPS

SEQ ID NO: 40 - protein, 39 aa, synthetic construct
  REGION 1..39: note = Synthetic Construct
  SITE 2: note = MISC_FEATURE - Xaa at position 2 is Aib
  MOD_RES 19: note = Lys at position 19 is chemically modified by conjugation of the epsilon-amino group of the Lys side chain with (2-[2-(2-amino-ethoxy)-ethoxy]-acetyl)2-(gamma-Glu)-CO-(CH2)18-CO 2H
  SITE 20: note = MISC_FEATURE - Xaa at position 20 is Aib
  MOD_RES 39: note = Ser at position 39 is amidated
YXEGTFTSDYSILLDKIAKXAFIEYLIEGGPSSGAPPPS

SEQ ID NO: 41 - protein, 39 aa, synthetic construct
  REGION 1..39: note = Synthetic Construct
  SITE 2: note = MISC_FEATURE - Xaa at position 2 is Aib
  SITE 20: note = MISC_FEATURE - Xaa at position 20 is Aib
  MOD_RES 21: note = Lys at position 17 is chemically modified by conjugation of the epsilon-amino group of the Lys side chain with (2-[2-(2-amino-ethoxy)-ethoxy]-acetyl)2-(gamma-Glu)-CO-(CH2)18-CO 2H
  MOD_RES 39: note = Ser at position 39 is amidated
YXEGTFTSDYSILLDKIAQXKFIEYLIEGGPSSGAPPPS

SEQ ID NO: 42 - protein, 39 aa, synthetic construct
  REGION 1..39: note = Synthetic Construct
  SITE 2: note = MISC_FEATURE - Xaa at position 2 is Aib
  SITE 20: note = MISC_FEATURE - Xaa at position 20 is Aib
  MOD_RES 23: note = Lys at position 23 is chemically modified by conjugation of the epsilon-amino group of the Lys side chain with (2-[2-(2-amino-ethoxy)-ethoxy]-acetyl)2-(gamma-Glu)-CO-(CH2)18-CO 2H
  MOD_RES 39: note = Ser at position 39 is amidated
YXEGTFTSDYSILLDKIAQXAFKEYLIEGGPSSGAPPPS

SEQ ID NO: 43 - protein, 39 aa, synthetic construct
  REGION 1..39: note = Synthetic Construct
  SITE 2: note = MISC_FEATURE - Xaa at position 2 is Aib
  SITE 20: note = MISC_FEATURE - Xaa at position 20 is Aib
  MOD_RES 24: note = Lys at position 24 is chemically modified by conjugation of the epsilon-amino group of the Lys side chain with (2-[2-(2-amino-ethoxy)-ethoxy]-acetyl)2-(gamma-Glu)-CO-(CH2)18-CO 2H
  MOD_RES 39: note = Ser at position 39 is amidated
YXEGTFTSDYSILLDKIAQXAFIKYLIEGGPSSGAPPPS

SEQ ID NO: 44 - protein, 39 aa, synthetic construct
  REGION 1..39: note = Synthetic Construct
  SITE 2: note = MISC_FEATURE - Xaa at position 2 is Aib
  SITE 20: note = MISC_FEATURE - Xaa at position 20 is Aib
  MOD_RES 26: note = Lys at position 26 is chemically modified by conjugation of the epsilon-amino group of the Lys side chain with (2-[2-(2-amino-ethoxy)-ethoxy]-acetyl)2-(gamma-Glu)-CO-(CH2)18-CO 2H
  MOD_RES 39: note = Ser at position 39 is amidated
YXEGTFTSDYSILLDKIAQXAFIEYKIEGGPSSGAPPPS

SEQ ID NO: 45 - protein, 39 aa, synthetic construct
  REGION 1..39: note = Synthetic Construct
  SITE 2: note = MISC_FEATURE - Xaa at position 2 is Aib
  SITE 20: note = MISC_FEATURE - Xaa at position 20 is Aib
  MOD_RES 27: note = Lys at position 27 is chemically modified by conjugation of the epsilon-amino group of the Lys side chain with (2-[2-(2-amino-ethoxy)-ethoxy]-acetyl)2-(gamma-Glu)-CO-(CH2)18-CO 2H
  MOD_RES 39: note = Ser at position 39 is amidated
YXEGTFTSDYSILLDKIAQXAFIEYLKEGGPSSGAPPPS

SEQ ID NO: 46 - protein, 39 aa, synthetic construct
  REGION 1..39: note = Synthetic Construct
  SITE 2: note = MISC_FEATURE - Xaa at position 2 is Aib
  SITE 20: note = MISC_FEATURE - Xaa at position 20 is Aib
  MOD_RES 28: note = Lys at position 28 is chemically modified by conjugation of the epsilon-amino group of the Lys side chain with (2-[2-(2-amino-ethoxy)-ethoxy]-acetyl)2-(gamma-Glu)-CO-(CH2)18-CO 2H
  MOD_RES 39: note = Ser at position 39 is amidated
YXEGTFTSDYSILLDKIAQXAFIEYLIKGGPSSGAPPPS

SEQ ID NO: 47 - protein, 39 aa, synthetic construct
  REGION 1..39: note = Synthetic Construct
  SITE 2: note = MISC_FEATURE - Xaa at position 2 is Aib
  SITE 20: note = MISC_FEATURE - Xaa at position 20 is Aib
  MOD_RES 29: note = Lys at position 29 is chemically modified by conjugation of the epsilon-amino group of the Lys side chain with (2-[2-(2-amino-ethoxy)-ethoxy]-acetyl)2-(gamma-Glu)-CO-(CH2)18-CO 2H
  MOD_RES 39: note = Ser at position 39 is amidated
YXEGTFTSDYSILLDKIAQXAFIEYLIEKGPSSGAPPPS

SEQ ID NO: 48 - protein, 39 aa, synthetic construct
  REGION 1..39: note = Synthetic Construct
  SITE 2: note = MISC_FEATURE - Xaa at position 2 is Aib
  SITE 20: note = MISC_FEATURE - Xaa at position 20 is Aib
  MOD_RES 30: note = Lys at position 30 is chemically modified by conjugation of the epsilon-amino group of the Lys side chain with (2-[2-(2-amino-ethoxy)-ethoxy]-acetyl)2-(gamma-Glu)-CO-(CH2)18-CO 2H
  MOD_RES 39: note = Ser at position 39 is amidated
YXEGTFTSDYSILLDKIAQXAFIEYLIEGKPSSGAPPPS

SEQ ID NO: 49 - protein, 39 aa, synthetic construct
  REGION 1..39: note = Synthetic Construct
  SITE 2: note = MISC_FEATURE - Xaa at position 2 is Aib
  SITE 20: note = MISC_FEATURE - Xaa at position 20 is Aib
  MOD_RES 31: note = Lys at position 31 is chemically modified by conjugation of the epsilon-amino group of the Lys side chain with (2-[2-(2-amino-ethoxy)-ethoxy]-acetyl)2-(gamma-Glu)-CO-(CH2)18-CO 2H
  MOD_RES 39: note = Ser at position 39 is amidated
YXEGTFTSDYSILLDKIAQXAFIEYLIEGGKSSGAPPPS

SEQ ID NO: 50 - protein, 39 aa, synthetic construct
  REGION 1..39: note = Synthetic Construct
  SITE 2: note = MISC_FEATURE - Xaa at position 2 is Aib
  SITE 20: note = MISC_FEATURE - Xaa at position 20 is Aib
  MOD_RES 32: note = Lys at position 32 is chemically modified by conjugation of the epsilon-amino group of the Lys side chain with (2-[2-(2-amino-ethoxy)-ethoxy]-acetyl)2-(gamma-Glu)-CO-(CH2)18-CO 2H
  MOD_RES 39: note = Ser at position 39 is amidated
YXEGTFTSDYSILLDKIAQXAFIEYLIEGGPKSGAPPPS

SEQ ID NO: 51 - protein, 39 aa, synthetic construct
  REGION 1..39: note = Synthetic Construct
  SITE 2: note = MISC_FEATURE - Xaa at position 2 is Aib
  SITE 20: note = MISC_FEATURE - Xaa at position 20 is Aib
  MOD_RES 33: note = Lys at position 33 is chemically modified by conjugation of the epsilon-amino group of the Lys side chain with (2-[2-(2-amino-ethoxy)-ethoxy]-acetyl)2-(gamma-Glu)-CO-(CH2)18-CO 2H
  MOD_RES 39: note = Ser at position 39 is amidated
YXEGTFTSDYSILLDKIAQXAFIEYLIEGGPSKGAPPPS

SEQ ID NO: 52 - protein, 39 aa, synthetic construct
  REGION 1..39: note = Synthetic Construct
  SITE 2: note = MISC_FEATURE - Xaa at position 2 is Aib
  SITE 20: note = MISC_FEATURE - Xaa at position 20 is Aib
  MOD_RES 34: note = Lys at position 34 is chemically modified by conjugation of the epsilon-amino group of the Lys side chain with (2-[2-(2-amino-ethoxy)-ethoxy]-acetyl)2-(gamma-Glu)-CO-(CH2)18-CO 2H
  MOD_RES 39: note = Ser at position 39 is amidated
YXEGTFTSDYSILLDKIAQXAFIEYLIEGGPSSKAPPPS

SEQ ID NO: 53 - protein, 39 aa, synthetic construct
  REGION 1..39: note = Synthetic Construct
  SITE 2: note = MISC_FEATURE - Xaa at position 2 is Aib
  SITE 20: note = MISC_FEATURE - Xaa at position 20 is Aib
  MOD_RES 35: note = Lys at position 35 is chemically modified by conjugation of the epsilon-amino group of the Lys side chain with (2-[2-(2-amino-ethoxy)-ethoxy]-acetyl)2-(gamma-Glu)-CO-(CH2)18-CO 2H
  MOD_RES 39: note = Ser at position 39 is amidated
YXEGTFTSDYSILLDKIAQXAFIEYLIEGGPSSGKPPPS

SEQ ID NO: 54 - protein, 39 aa, synthetic construct
  REGION 1..39: note = Synthetic Construct
  SITE 2: note = MISC_FEATURE - Xaa at position 2 is Aib
  SITE 20: note = MISC_FEATURE - Xaa at position 20 is Aib
  MOD_RES 36: note = Lys at position 36 is chemically modified by conjugation of the epsilon-amino group of the Lys side chain with (2-[2-(2-amino-ethoxy)-ethoxy]-acetyl)2-(gamma-Glu)-CO-(CH2)18-CO 2H
  MOD_RES 39: note = Ser at position 39 is amidated
YXEGTFTSDYSILLDKIAQXAFIEYLIEGGPSSGAKPPS

SEQ ID NO: 55 - protein, 39 aa, synthetic construct
  REGION 1..39: note = Synthetic Construct
  SITE 2: note = MISC_FEATURE - Xaa at position 2 is Aib
  SITE 20: note = MISC_FEATURE - Xaa at position 20 is Aib
  MOD_RES 37: note = Lys at position 37 is chemically modified by conjugation of the epsilon-amino group of the Lys side chain with (2-[2-(2-amino-ethoxy)-ethoxy]-acetyl)2-(gamma-Glu)-CO-(CH2)18-CO 2H
  MOD_RES 39: note = Ser at position 39 is amidated
YXEGTFTSDYSILLDKIAQXAFIEYLIEGGPSSGAPKPS

SEQ ID NO: 56 - protein, 39 aa, synthetic construct
  REGION 1..39: note = Synthetic Construct
  SITE 2: note = MISC_FEATURE - Xaa at position 2 is Aib
  SITE 20: note = MISC_FEATURE - Xaa at position 20 is Aib
  MOD_RES 38: note = Lys at position 38 is chemically modified by conjugation of the epsilon-amino group of the Lys side chain with (2-[2-(2-amino-ethoxy)-ethoxy]-acetyl)2-(gamma-Glu)-CO-(CH2)18-CO 2H
  MOD_RES 39: note = Ser at position 39 is amidated
YXEGTFTSDYSILLDKIAQXAFIEYLIEGGPSSGAPPKS

SEQ ID NO: 57 - protein, 39 aa, synthetic construct
  REGION 1..39: note = Synthetic Construct
  SITE 2: note = MISC_FEATURE - Xaa at position 2 is Aib
  SITE 20: note = MISC_FEATURE - Xaa at position 20 is Aib
  MOD_RES 39: note = Lys at position 39 is chemically modified by conjugation of the epsilon-amino group of the Lys side chain with (2-[2-(2-amino-ethoxy)-ethoxy]-acetyl)2-(gamma-Glu)-CO-(CH2)18-CO 2H
  MOD_RES 39: note = Lys at position 39 is amidated
YXEGTFTSDYSILLDKIAQXAFIEYLIEGGPSSGAPPPK

SEQ ID NO: 58 - protein, 40 aa, synthetic construct
  REGION 1..40: note = Synthetic Construct
  SITE 2: note = MISC_FEATURE - Xaa at position 2 is Aib
  SITE 20: note = MISC_FEATURE - Xaa at position 20 is Aib
  MOD_RES 40: note = Lys at position 40 is chemically modified by conjugation of the epsilon-amino group of the Lys side chain with (2-[2-(2-amino-ethoxy)-ethoxy]-acetyl)2-(gamma-Glu)-CO-(CH2)18-CO 2H
  MOD_RES 40: note = Lys at position 40 is amidated
YXEGTFTSDYSILLDKIAQXAFIEYLIEGGPSSGAPPPSK

SEQ ID NO: 59 - protein, 34 aa, synthetic construct
  REGION 1..34: note = Synthetic Construct
  SITE 2: note = MISC_FEATURE - Xaa at position 2 is Aib
  MOD_RES 17: note = Lys at position 17 is chemically modified by conjugation of the epsilon-amino group of the Lys side chain with (2-[2-(2-amino-ethoxy)-ethoxy]-acetyl)2-(gamma-Glu)-CO-(CH2)18-CO 2H
  SITE 20: note = MISC_FEATURE - Xaa at position 20 is Aib
  MOD_RES 34: note = Gly at position 34 is amidated
YXEGTFTSDYSILLDKKAQXAFIEYLIEGGPSSG

SEQ ID NO: 60 - protein, 30 aa, synthetic construct
  REGION 1..30: note = Synthetic Construct
  SITE 2: note = MISC_FEATURE - Xaa at position 2 is Aib
  MOD_RES 17: note = Lys at position 17 is chemically modified by conjugation of the epsilon-amino group of the Lys side chain with (2-[2-(2-amino-ethoxy)-ethoxy]-acetyl)2-(gamma-Glu)-CO-(CH2)18-CO 2H
  SITE 20: note = MISC_FEATURE - Xaa at position 20 is Aib
  MOD_RES 30: note = Gly at position 30 is amidated
YXEGTFTSDYSILLDKKAQXAFIEYLIEGG

SEQ ID NO: 61 - protein, 39 aa, synthetic construct
  REGION 1..39: note = Synthetic Construct
  SITE 2: note = MISC_FEATURE - Xaa at position 2 is Aib
  SITE 13: note = MISC_FEATURE - Xaa at position 13 is alpha-methyl-Leu
  MOD_RES 17: note = Lys at position 17 is chemically modified by conjugation of the epsilon-amino group of the Lys side chain with (2-[2-(2-amino-ethoxy)-ethoxy]-acetyl)2-(gamma-Glu)-CO-(CH2)18-CO 2H
  SITE 20: note = MISC_FEATURE - Xaa at position 20 is Aib
  MOD_RES 39: note = Ser at position 39 is amidated
YXEGTFTSDYSIXLDSKAQXAFIEYLIEGGPSSGAPPPS

SEQ ID NO: 62 - protein, 39 aa, synthetic construct
  REGION 1..39: note = Synthetic Construct
  SITE 2: note = MISC_FEATURE - Xaa at position 2 is Aib
  SITE 13: note = MISC_FEATURE - Xaa at position 13 is alpha-methyl-Leu
  MOD_RES 17: note = Lys at position 17 is chemically modified by conjugation of the epsilon-amino group of the Lys side chain with (2-[2-(2-amino-ethoxy)-ethoxy]-acetyl)2-(gamma-Glu)-CO-(CH2)18-CO 2H
  SITE 20: note = MISC_FEATURE - Xaa at position 20 is Aib
  MOD_RES 39: note = Ser at position 39 is amidated
HXEGTFTSDYSIXLDKKAQXAFIEYLIEGGPSSGAPPPS

SEQ ID NO: 63 - protein, 39 aa, synthetic construct
  REGION 1..39: note = Synthetic Construct
  SITE 2: note = MISC_FEATURE - Xaa at position 2 is Aib
  SITE 13: note = MISC_FEATURE - Xaa at position 13 is alpha-methyl-Leu
  MOD_RES 17: note = Lys at position 17 is chemically modified by conjugation of the epsilon-amino group of the Lys side chain with (2-[2-(2-amino-ethoxy)-ethoxy]-acetyl)2-(gamma-Glu)-CO-(CH2)18-CO 2H
  MOD_RES 39: note = Ser at position 39 is amidated
HXEGTFTSDYSIXLDKKAQHAFIEYLIEGGPSSGAPPPS

SEQ ID NO: 64 - protein, 39 aa, synthetic construct
  REGION 1..39: note = Synthetic Construct
  SITE 2: note = MISC_FEATURE - Xaa at position 2 is Aib
  SITE 13: note = MISC_FEATURE - Xaa at position 13 is alpha-methyl-Leu
  MOD_RES 17: note = Lys at position 17 is chemically modified by conjugation of the epsilon-amino group of the Lys side chain with (2-[2-(2-amino-ethoxy)-ethoxy]-acetyl)2-(gamma-Glu)-CO-(CH2)18-CO 2H
  MOD_RES 39: note = Ser at position 39 is amidated
HXEGTFTSDYSIXLDEKAQHAFIEYLIEGGPSSGAPPPS

SEQ ID NO: 65 - protein, 39 aa, synthetic construct
  REGION 1..39: note = Synthetic Construct
  SITE 2: note = MISC_FEATURE - Xaa at position 2 is Aib
  SITE 13: note = MISC_FEATURE - Xaa at position 13 is alpha-methyl-Leu
  MOD_RES 17: note = Lys at position 17 is chemically modified by conjugation of the epsilon-amino group of the Lys side chain with (2-[2-(2-amino-ethoxy)-ethoxy]-acetyl)2-(gamma-Glu)-CO-(CH2)18-CO 2H
  MOD_RES 39: note = Ser at position 39 is amidated
YXEGTFTSDYSIXLDEKAQHAFIEYLIEGGPSSGAPPPS

SEQ ID NO: 66 - protein, 39 aa, synthetic construct
  REGION 1..39: note = Synthetic Construct
  SITE 2: note = MISC_FEATURE - Xaa at position 2 is Aib
  SITE 6: note = MISC_FEATURE - Xaa at position 6 is alpha-methyl-Phe
  MOD_RES 17: note = Lys at position 17 is chemically modified by conjugation of the epsilon-amino group of the Lys side chain with (2-[2-(2-amino-ethoxy)-ethoxy]-acetyl)2-(gamma-Glu)-CO-(CH2)18-CO 2H
  SITE 20: note = MISC_FEATURE - Xaa at position 20 is Aib
  MOD_RES 39: note = Ser at position 39 is amidated
YXEGTXTSDYSILLDKKAQXAFIEYLIEGGPSSGAPPPS

SEQ ID NO: 67 - protein, 39 aa, synthetic construct
  REGION 1..39: note = Synthetic Construct
  SITE 2: note = MISC_FEATURE - Xaa at position 2 is Aib
  MOD_RES 17: note = Lys at position 17 is chemically modified by conjugation of the epsilon-amino group of the Lys side chain with (2-[2-(2-amino-ethoxy)-ethoxy]-acetyl)2-(gamma-Glu)-CO-(CH2)18-CO 2H
  SITE 20: note = MISC_FEATURE - Xaa at position 20 is Aib
  MOD_RES 39: note = Ser at position 39 is amidated
YXEGTFTSDYSSLLDKKAQXAFIEYLIEGGPSSGAPPPS

SEQ ID NO: 68 - protein, 39 aa, synthetic construct
  REGION 1..39: note = Synthetic Construct
  SITE 2: note = MISC_FEATURE - Xaa at position 2 is Aib
  SITE 13: note = MISC_FEATURE - Xaa at position 13 is alpha-methyl-Leu
  MOD_RES 17: note = Lys at position 17 is chemically modified by conjugation of the epsilon-amino group of the Lys side chain with (2-[2-(2-amino-ethoxy)-ethoxy]-acetyl)2-(gamma-Glu)-CO-(CH2)18-CO 2H
  SITE 20: note = MISC_FEATURE - Xaa at position 20 is Aib
  MOD_RES 39: note = Ser at position 39 is amidated
YXEGTFTSDYSIXLDEKAQXAFIEYLIEGGPSSGAPPPS

SEQ ID NO: 69 - protein, 39 aa, synthetic construct
  REGION 1..39: note = Synthetic Construct
  SITE 2: note = MISC_FEATURE - Xaa at position 2 is Aib
  SITE 13: note = MISC_FEATURE - Xaa at position 13 is alpha-methyl-Leu
  SITE 16: note = MISC_FEATURE - Xaa at position 16 is Aib
  MOD_RES 17: note = Lys at position 17 is chemically modified by conjugation of the epsilon-amino group of the Lys side chain with (2-[2-(2-amino-ethoxy)-ethoxy]-acetyl)2-(gamma-Glu)-CO-(CH2)18-CO 2H
  SITE 20: note = MISC_FEATURE - Xaa at position 20 is Aib
  MOD_RES 39: note = Ser at position 39 is amidated
YXEGTFTSDYSIXLDXKAQXAFIEYLIEGGPSSGAPPPS

SEQ ID NO: 70 - protein, 39 aa, synthetic construct
  REGION 1..39: note = Synthetic Construct
  SITE 2: note = MISC_FEATURE - Xaa at position 2 is Aib
  SITE 13: note = MISC_FEATURE - Xaa at position 13 is alpha-methyl-Leu
  MOD_RES 17: note = Lys at position 17 is chemically modified by conjugation of the epsilon-amino group of the Lys side chain with (2-[2-(2-amino-ethoxy)-ethoxy]-acetyl)2-(gamma-Glu)-CO-(CH2)18-CO 2H
  SITE 20: note = MISC_FEATURE - Xaa at position 20 is Aib
  MOD_RES 39: note = Ser at position 39 is amidated
YXEGTFTSDYSIXLDSKAQXAFIEYLLEGGPSSGAPPPS

SEQ ID NO: 71 - protein, 30 aa, synthetic construct
  REGION 1..30: note = Synthetic Construct
  SITE 2: note = MISC_FEATURE - Xaa at position 2 is Aib
  SITE 13: note = MISC_FEATURE - Xaa at position 13 is alpha-methyl-Leu
  MOD_RES 17: note = Lys at position 17 is chemically modified by conjugation of the epsilon-amino group of the Lys side chain with (2-[2-(2-amino-ethoxy)-ethoxy]-acetyl)2-(gamma-Glu)-CO-(CH2)18-CO 2H
  SITE 20: note = MISC_FEATURE - Xaa at position 20 is Aib
  MOD_RES 30: note = Gly at position 30 is amidated
YXEGTFTSDYSIXLDKKAQXAFIEYLIEGG

SEQ ID NO: 72 - protein, 30 aa, synthetic construct
  REGION 1..30: note = Synthetic Construct
  SITE 2: note = MISC_FEATURE - Xaa at position 2 is Aib
  SITE 13: note = MISC_FEATURE - Xaa at position 13 is alpha-methyl-Leu
  MOD_RES 17: note = Lys at position 17 is chemically modified by conjugation of the epsilon-amino group of the Lys side chain with (2-[2-(2-amino-ethoxy)-ethoxy]-acetyl)2-(gamma-Glu)-CO-(CH2)18-CO 2H
  SITE 20: note = MISC_FEATURE - Xaa at position 20 is Aib
  MOD_RES 30: note = Gly at position 30 is amidated
YXEGTFTSDYSIXLDEKAQXAFIEYLIEGG

SEQ ID NO: 73 - protein, 30 aa, synthetic construct
  REGION 1..30: note = Synthetic Construct
  SITE 2: note = MISC_FEATURE - Xaa at position 2 is Aib
  SITE 13: note = MISC_FEATURE - Xaa at position 13 is alpha-methyl-Leu
  MOD_RES 17: note = Lys at position 17 is chemically modified by conjugation of the epsilon-amino group of the Lys side chain with (2-[2-(2-amino-ethoxy)-ethoxy]-acetyl)2-(gamma-Glu)-CO-(CH2)18-CO 2H
  SITE 20: note = MISC_FEATURE - Xaa at position 20 is Aib
  MOD_RES 30: note = Gly at position 30 is amidated
YXEGTFTSDYSIXLDSKAQXAFIEYLIEGG

SEQ ID NO: 74 - protein, 30 aa, synthetic construct
  REGION 1..30: note = Synthetic Construct
  SITE 2: note = MISC_FEATURE - Xaa at position 2 is Aib
  SITE 13: note = MISC_FEATURE - Xaa at position 13 is alpha-methyl-Leu
  MOD_RES 17: note = Lys at position 17 is chemically modified by conjugation of the epsilon-amino group of the Lys side chain with (2-[2-(2-amino-ethoxy)-ethoxy]-acetyl)2-(gamma-Glu)-CO-(CH2)18-CO 2H
  SITE 20: note = MISC_FEATURE - Xaa at position 20 is Aib
  MOD_RES 30: note = Gly at position 30 is amidated
YXEGTFTSDYSIXLDTKAQXAFIEYLIEGG

SEQ ID NO: 75 - protein, 39 aa, synthetic construct; identical to SEQ ID NO: 30
  REGION 1..39: note = Synthetic Construct
  SITE 2: note = MISC_FEATURE - Xaa at position 2 is Aib
  SITE 13: note = MISC_FEATURE - Xaa at position 13 is alpha-methyl-Leu
  MOD_RES 17: note = Lys at position 17 is chemically modified by conjugation of the epsilon-amino group of the Lys side chain with (2-[2-(2-amino-ethoxy)-ethoxy]-acetyl)2-(gamma-Glu)-CO-(CH2)18-CO 2H
  SITE 20: note = MISC_FEATURE - Xaa at position 20 is Aib
  MOD_RES 39: note = Ser at position 39 is amidated

SEQ ID NO: 76 - protein, 39 aa, synthetic construct
  REGION 1..39: note = Synthetic Construct
  SITE 2: note = MISC_FEATURE - Xaa at position 2 is Aib
  MOD_RES 17: note = Lys at position 17 is chemically modified by conjugation of the epsilon-amino group of the Lys side chain with (2-[2-(2-amino-ethoxy)-ethoxy]-acetyl)2-(gamma-Glu)-CO-(CH2)18-CO 2H
  SITE 20: note = MISC_FEATURE - Xaa at position 20 is Aib
  SITE 22: note = MISC_FEATURE - Xaa at position 22 is alpha-methyl-Phe
  MOD_RES 39: note = Ser at position 39 is amidated
YXEGTFTSDYSILLDKKAQXAXIEYLIEGGPSSGAPPPS

SEQ ID NO: 77 - protein, 39 aa, synthetic construct
  REGION 1..39: note = Synthetic Construct
  SITE 2: note = MISC_FEATURE - Xaa at position 2 is Aib
  SITE 11: note = MISC_FEATURE - Xaa at position 11 is alpha-methyl-Ser
  MOD_RES 17: note = Lys at position 17 is chemically modified by conjugation of the epsilon-amino group of the Lys side chain with (2-[2-(2-amino-ethoxy)-ethoxy]-acetyl)2-(gamma-Glu)-CO-(CH2)18-CO 2H
  SITE 20: note = MISC_FEATURE - Xaa at position 20 is Aib
  MOD_RES 39: note = Ser at position 39 is amidated
YXEGTFTSDYXILLDKKAQXAFIEYLIEGGPSSGAPPPS

SEQ ID NO: 78 - protein, 39 aa, synthetic construct
  REGION 1..39: note = Synthetic Construct
  SITE 2: note = MISC_FEATURE - Xaa at position 2 is Aib
  SITE 6: note = MISC_FEATURE - Xaa at position 6 is alpha-methyl-Phe
  SITE 13: note = MISC_FEATURE - Xaa at position 13 is alpha-methyl-Leu
  MOD_RES 17: note = Lys at position 17 is chemically modified by conjugation of the epsilon-amino group of the Lys side chain with (2-[2-(2-amino-ethoxy)-ethoxy]-acetyl)2-(gamma-Glu)-CO-(CH2)18-CO 2H
  SITE 20: note = MISC_FEATURE - Xaa at position 20 is Aib
  MOD_RES 39: note = Ser at position 39 is amidated
YXEGTXTSDYSIXLDKKAQXAFIEYLIEGGPSSGAPPPS

SEQ ID NO: 79 - protein, 30 aa, synthetic construct
  REGION 1..30: note = Synthetic Construct
  SITE 2: note = MISC_FEATURE - Xaa at position 2 is Aib
  MOD_RES 10: note = Lys at position 10 is chemically modified by conjugation of the epsilon-amino group of the Lys side chain with (2-[2-(2-amino-ethoxy)-ethoxy]-acetyl)2-(gamma-Glu)-CO-(CH2)18-CO 2H
  SITE 20: note = MISC_FEATURE - Xaa at position 20 is Aib
  MOD_RES 30: note = Gly at position 30 is amidated
YXEGTFTSDKSILLDKIAQXAFIEYLIEGG

SEQ ID NO: 80 - protein, 30 aa, synthetic construct
  REGION 1..30: note = Synthetic Construct
  SITE 2: note = MISC_FEATURE - Xaa at position 2 is Aib
  MOD_RES 14: note = Lys at position 14 is chemically modified by conjugation of the epsilon-amino group of the Lys side chain with (2-[2-(2-amino-ethoxy)-ethoxy]-acetyl)2-(gamma-Glu)-CO-(CH2)18-CO 2H
  SITE 20: note = MISC_FEATURE - Xaa at position 20 is Aib
  MOD_RES 30: note = Gly at position 30 is amidated
YXEGTFTSDYSILKDKIAQXAFIEYLIEGG

SEQ ID NO: 81 - protein, 30 aa, synthetic construct
  REGION 1..30: note = Synthetic Construct
  SITE 2: note = MISC_FEATURE - Xaa at position 2 is Aib
  SITE 20: note = MISC_FEATURE - Xaa at position 20 is Aib
  MOD_RES 21: note = Lys at position 21 is chemically modified by conjugation of the epsilon-amino group of the Lys side chain with (2-[2-(2-amino-ethoxy)-ethoxy]-acetyl)2-(gamma-Glu)-CO-(CH2)18-CO 2H
  MOD_RES 30: note = Gly at position 30 is amidated
YXEGTFTSDYSILLDKIAQXKFIEYLIEGG

SEQ ID NO: 82 - protein, 30 aa, synthetic construct
  REGION 1..30: note = Synthetic Construct
  SITE 2: note = MISC_FEATURE - Xaa at position 2 is Aib
  SITE 20: note = MISC_FEATURE - Xaa at position 20 is Aib
  MOD_RES 28: note = Lys at position 28 is chemically modified by conjugation of the epsilon-amino group of the Lys side chain with (2-[2-(2-amino-ethoxy)-ethoxy]-acetyl)2-(gamma-Glu)-CO-(CH2)18-CO 2H
  MOD_RES 30: note = Gly at position 30 is amidated
YXEGTFTSDYSILLDKIAQXAFIEYLIKGG

SEQ ID NO: 83 - protein, 39 aa, synthetic construct
  REGION 1..39: note = Synthetic Construct
  SITE 2: note = MISC_FEATURE - Xaa at position 2 is Aib
  SITE 13: note = MISC_FEATURE - Xaa at position 13 is alpha-methyl-Leu
  MOD_RES 17: note = Lys at position 17 is chemically modified by conjugation of the epsilon-amino group of the Lys side chain with (2-[2-(2-amino-ethoxy)-ethoxy]-acetyl)2-(gamma-Glu)-CO-(CH2)18-CO 2H
  SITE 20: note = MISC_FEATURE - Xaa at position 20 is Aib
  SITE 22: note = MISC_FEATURE - Xaa at position 22 is alpha-methyl-Phe
  MOD_RES 39: note = Ser at position 39 is amidated
YXEGTFTSDYSIXLDKKAQXAXIEYLIEGGPSSGAPPPS

SEQ ID NO: 84 - protein, 39 aa, synthetic construct
  REGION 1..39: note = Synthetic Construct
  SITE 2: note = MISC_FEATURE - Xaa at position 2 is Aib
  SITE 13: note = MISC_FEATURE - Xaa at position 13 is alpha-methyl-Leu
  MOD_RES 17: note = Lys at position 17 is chemically modified by conjugation of the epsilon-amino group of the Lys side chain with (2-[2-(2-amino-ethoxy)-ethoxy]-acetyl)2-(gamma-Glu)-CO-(CH2)18-CO 2H
  SITE 20: note = MISC_FEATURE - Xaa at position 20 is Aib
  SITE 26: note = MISC_FEATURE - Xaa at position 26 is alpha-methyl-Leu
  MOD_RES 39: note = Ser at position 39 is amidated
YXEGTFTSDYSIXLDKKAQXAFIEYXIEGGPSSGAPPPS

SEQ ID NO: 85 - protein, 39 aa, synthetic construct
  REGION 1..39: note = Synthetic Construct
  SITE 2: note = MISC_FEATURE - Xaa at position 2 is Aib
  SITE 6: note = MISC_FEATURE - Xaa at position 6 is alpha-methyl-Phe
  SITE 13: note = MISC_FEATURE - Xaa at position 13 is alpha-methyl-Leu
  MOD_RES 17: note = Lys at position 17 is chemically modified by conjugation of the epsilon-amino group of the Lys side chain with (2-[2-(2-amino-ethoxy)-ethoxy]-acetyl)2-(gamma-Glu)-CO-(CH2)18-CO 2H
  SITE 20: note = MISC_FEATURE - Xaa at position 20 is Aib
  SITE 22: note = MISC_FEATURE - Xaa at position 22 is alpha-methyl-Phe
  MOD_RES 39: note = Ser at position 39 is amidated
YXEGTXTSDYSIXLDKKAQXAXIEYLIEGGPSSGAPPPS

SEQ ID NO: 86 - protein, 38 aa, synthetic construct
  REGION 1..38: note = Synthetic Construct
  SITE 2: note = MISC_FEATURE - Xaa at position 2 is Aib
  SITE 19: note = MISC_FEATURE - Xaa at position 19 is Aib
  MOD_RES 37: note = Lys at position 37 is chemically modified by conjugation of the epsilon-amino group of the Lys side chain with (2-[2-(2-amino-ethoxy)-ethoxy]-acetyl)2-(gamma-Glu)-CO-(CH2)18-CO 2H
  MOD_RES 38: note = Ser at position 38 is amidated
YXEGTFTSDYSILLKIAQXAFIEYLIEGGPSSGAPPKS

SEQ ID NO: 87 - protein, 39 aa, synthetic construct
  REGION 1..39: note = Synthetic Construct
  SITE 1: note = MISC_FEATURE - Xaa at position 1 is D-Tyr
  SITE 2: note = MISC_FEATURE - Xaa at position 2 is Aib
  MOD_RES 17: note = Lys at position 17 is chemically modified by conjugation of the epsilon-amino group of the Lys side chain with (2-[2-(2-amino-ethoxy)-ethoxy]-acetyl)2-(gamma-Glu)-CO-(CH2)18-CO 2H
  SITE 20: note = MISC_FEATURE - Xaa at position 20 is Aib
  MOD_RES 39: note = Ser at position 39 is amidated
XXEGTFTSDYSILLDKKAQXAFIEYLIEGGPSSGAPPPS

SEQ ID NO: 88 - protein, 39 aa, synthetic construct
  REGION 1..39: note = Synthetic Construct
  SITE 1: note = MISC_FEATURE - Xaa at position 1 is D-Tyr
  MOD_RES 1: note = The N-terminal amino is acetylated
  MOD_RES 17: note = Lys at position 17 is chemically modified by conjugation of the epsilon-amino group of the Lys side chain with (2-[2-(2-amino-ethoxy)-ethoxy]-acetyl)2-(gamma-Glu)-CO-(CH2)18-CO 2H
  SITE 20: note = MISC_FEATURE - Xaa at position 20 is Aib
  MOD_RES 39: note = Ser at position 39 is amidated
XAEGTFTSDYSILLDKKAQXAFIEYLIEGGPSSGAPPPS

SEQ ID NO: 89 - protein, 39 aa, synthetic construct; identical to SEQ ID NO: 17
  REGION 1..39: note = Synthetic Construct
  SITE 2: note = MISC_FEATURE - Xaa at position 2 is D-Ala
  MOD_RES 17: note = Lys at position 17 is chemically modified by conjugation of the epsilon-amino group of the Lys side chain with (2-[2-(2-amino-ethoxy)-ethoxy]-acetyl)2-(gamma-Glu)-CO-(CH2)18-CO 2H
  SITE 20: note = MISC_FEATURE - Xaa at position 20 is Aib
  MOD_RES 39: note = Ser at position 39 is amidated

SEQ ID NO: 90 - protein, 39 aa, synthetic construct; identical to SEQ ID NO: 77
  REGION 1..39: note = Synthetic Construct
  SITE 2: note = MISC_FEATURE - Xaa at position 2 is Aib
  SITE 11: note = MISC_FEATURE - Xaa at position 11 is D-Ser
  MOD_RES 17: note = Lys at position 17 is chemically modified by conjugation of the epsilon-amino group of the Lys side chain with (2-[2-(2-amino-ethoxy)-ethoxy]-acetyl)2-(gamma-Glu)-CO-(CH2)18-CO 2H
  SITE 20: note = MISC_FEATURE - Xaa at position 20 is Aib
  MOD_RES 39: note = Ser at position 39 is amidated

SEQ ID NO: 91 - protein, 39 aa, synthetic construct
  REGION 1..39: note = Synthetic Construct
  SITE 2: note = MISC_FEATURE - Xaa at position 2 is Aib
  SITE 12: note = MISC_FEATURE - Xaa at position 12 is D-Ile
  MOD_RES 17: note = Lys at position 17 is chemically modified by conjugation of the epsilon-amino group of the Lys side chain with (2-[2-(2-amino-ethoxy)-ethoxy]-acetyl)2-(gamma-Glu)-CO-(CH2)18-CO 2H
  SITE 20: note = MISC_FEATURE - Xaa at position 20 is Aib
  MOD_RES 39: note = Ser at position 39 is amidated
YXEGTFTSDYSXLLDKKAQXAFIEYLIEGGPSSGAPPPS

SEQ ID NO: 92 - protein, 39 aa, synthetic construct
  REGION 1..39: note = Synthetic Construct
  SITE 2: note = MISC_FEATURE - Xaa at position 2 is Aib
  MOD_RES 17: note = Lys at position 17 is chemically modified by conjugation of the epsilon-amino group of the Lys side chain with (2-[2-(2-amino-ethoxy)-ethoxy]-acetyl)2-(gamma-Glu)-CO-(CH2)18-CO 2H
  SITE 20: note = MISC_FEATURE - Xaa at position 20 is Aib
  SITE 28: note = MISC_FEATURE - Xaa at position 28 is D-Glu
  MOD_RES 39: note = Ser at position 39 is amidated
YXEGTFTSDYSILLDKKAQXAFIEYLIXGGPSSGAPPPS

SEQ ID NO: 93 - protein, 39 aa, synthetic construct
  REGION 1..39: note = Synthetic Construct
  SITE 2: note = MISC_FEATURE - Xaa at position 2 is Aib
  MOD_RES 17: note = Lys at position 17 is chemically modified by conjugation of the epsilon-amino group of the Lys side chain with (2-[2-(2-amino-ethoxy)-ethoxy]-acetyl)2-(gamma-Glu)-CO-(CH2)18-CO 2H
  SITE 20: note = MISC_FEATURE - Xaa at position 20 is Aib
  SITE 24: note = MISC_FEATURE - Xaa at position 24 is D-Glu
  MOD_RES 39: note = Ser at position 39 is amidated
YXEGTFTSDYSILLDKKAQXAFIXYLIEGGPSSGAPPPS

SEQ ID NO: 94 - protein, 39 aa, synthetic construct
  REGION 1..39: note = Synthetic Construct
  SITE 2: note = MISC_FEATURE - Xaa at position 2 is Aib
  MOD_RES 17: note = Lys at position 17 is chemically modified by conjugation of the epsilon-amino group of the Lys side chain with (2-[2-(2-amino-ethoxy)-ethoxy]-acetyl)2-(gamma-Glu)-CO-(CH2)18-CO 2H
  SITE 20: note = MISC_FEATURE - Xaa at position 20 is Aib
  MOD_RES 39: note = Ser at position 39 is amidated
YXEGTFTSDASILLDKKAQXAFIEYLIEGGPSSGAPPPS

SEQ ID NO: 95 - protein, 39 aa, synthetic construct
  REGION 1..39: note = Synthetic Construct
  SITE 2: note = MISC_FEATURE - Xaa at position 2 is Aib
  MOD_RES 17: note = Lys at position 17 is chemically modified by conjugation of the epsilon-amino group of the Lys side chain with (2-[2-(2-amino-ethoxy)-ethoxy]-acetyl)2-(gamma-Glu)-CO-(CH2)18-CO 2H
  SITE 20: note = MISC_FEATURE - Xaa at position 20 is Aib
  MOD_RES 39: note = Ser at position 39 is amidated
YXEGTFTSDYSILLDKKAQXAFIEYLIEAGPSSGAPPPS

SEQ ID NO: 96 - protein, 39 aa, synthetic construct; identical to SEQ ID NO: 17
  REGION 1..39: note = Synthetic Construct
  SITE 2: note = MISC_FEATURE - Xaa at position 2 is alpha-methyl-Pro
  MOD_RES 17: note = Lys at position 17 is chemically modified by conjugation of the epsilon-amino group of the Lys side chain with (2-[2-(2-amino-ethoxy)-ethoxy]-acetyl)2-(gamma-Glu)-CO-(CH2)18-CO 2H
  SITE 20: note = MISC_FEATURE - Xaa at position 20 is Aib
  MOD_RES 39: note = Ser at position 39 is amidated

SEQ ID NO: 97 - protein, 39 aa, synthetic construct
  REGION 1..39: note = Synthetic Construct
  MOD_RES 17: note = Lys at position 17 is chemically modified by conjugation of the epsilon-amino group of the Lys side chain with (2-[2-(2-amino-ethoxy)-ethoxy]-acetyl)2-(gamma-Glu)-CO-(CH2)18-CO 2H
  SITE 20: note = MISC_FEATURE - Xaa at position 20 is Aib
  MOD_RES 39: note = Ser at position 39 is amidated
YPEGTFTSDYSILLDKKAQXAFIEYLIEGGPSSGAPPPS

SEQ ID NO: 98 - protein, 39 aa, synthetic construct
  REGION 1..39: note = Synthetic Construct
  SITE 2: note = MISC_FEATURE - Xaa at position 2 is Aib
  SITE 3: note = MISC_FEATURE - Xaa at position 3 is Aad
  MOD_RES 17: note = Lys at position 17 is chemically modified by conjugation of the epsilon-amino group of the Lys side chain with (2-[2-(2-amino-ethoxy)-ethoxy]-acetyl)2-(gamma-Glu)-CO-(CH2)18-CO 2H
  SITE 20: note = MISC_FEATURE - Xaa at position 20 is Aib
  MOD_RES 39: note = Ser at position 39 is amidated
YXXGTFTSDYSILLDKKAQXAFIEYLIEGGPSSGAPPPS

SEQ ID NO: 99 - protein, 39 aa, synthetic construct
  REGION 1..39: note = Synthetic Construct
  SITE 2: note = MISC_FEATURE - Xaa at position 2 is Aib
  MOD_RES 17: note = Lys at position 17 is chemically modified by conjugation of the epsilon-amino group of the Lys side chain with (2-[2-(2-amino-ethoxy)-ethoxy]-acetyl)2-(gamma-Glu)-CO-(CH2)18-CO 2H
  SITE 20: note = MISC_FEATURE - Xaa at position 20 is Aib
  MOD_RES 39: note = Ser at position 39 is amidated
YXNGTFTSDYSILLDKKAQXAFIEYLIEGGPSSGAPPPS

SEQ ID NO: 100 - protein, 39 aa, synthetic construct; identical to SEQ ID NO: 98
  REGION 1..39: note = Synthetic Construct
  SITE 2: note = MISC_FEATURE - Xaa at position 2 is Aib
  SITE 3: note = MISC_FEATURE - Xaa at position 3 is gamma-Glu
  MOD_RES 17: note = Lys at position 17 is chemically modified by conjugation of the epsilon-amino group of the Lys side chain with (2-[2-(2-amino-ethoxy)-ethoxy]-acetyl)2-(gamma-Glu)-CO-(CH2)18-CO 2H
  SITE 20: note = MISC_FEATURE - Xaa at position 20 is Aib
  MOD_RES 39: note = Ser at position 39 is amidated

SEQ ID NO: 101 - protein, 30 aa, synthetic construct
  REGION 1..30: note = Synthetic Construct
  SITE 2: note = MISC_FEATURE - Xaa at position 2 is Aib
  SITE 6: note = MISC_FEATURE - Xaa at position 6 is alpha-methyl-Phe
  MOD_RES 10: note = Lys at position 10 is chemically modified by conjugation of the epsilon-amino group of the Lys side chain with (2-[2-(2-amino-ethoxy)-ethoxy]-acetyl)2-(gamma-Glu)-CO-(CH2)18-CO 2H
  SITE 20: note = MISC_FEATURE - Xaa at position 20 is Aib
  MOD_RES 30: note = Gly at position 30 is amidated
YXEGTXTSDKSILLDKIAQXAFIEYLIEGG

SEQ ID NO: 102 - protein, 30 aa, synthetic construct
  REGION 1..30: note = Synthetic Construct
  SITE 2: note = MISC_FEATURE - Xaa at position 2 is Aib
  SITE 6: note = MISC_FEATURE - Xaa at position 6 is alpha-methyl-Phe
  MOD_RES 14: note = Lys at position 14 is chemically modified by conjugation of the epsilon-amino group of the Lys side chain with (2-[2-(2-amino-ethoxy)-ethoxy]-acetyl)2-(gamma-Glu)-CO-(CH2)18-CO 2H
  SITE 20: note = MISC_FEATURE - Xaa at position 20 is Aib
  SITE 30: note = MISC_FEATURE - Gly at position 30 is amidated
YXEGTXTSDYSILKDKIAQXAFIEYLIEGG

SEQ ID NO: 103 - protein, 30 aa, synthetic construct
  REGION 1..30: note = Synthetic Construct
  SITE 2: note = MISC_FEATURE - Xaa at position 2 is Aib
  SITE 6: note = MISC_FEATURE - Xaa at position 6 is alpha-methyl-Phe
  SITE 20: note = MISC_FEATURE - Xaa at position 20 is Aib
  MOD_RES 21: note = Lys at position 21 is chemically modified by conjugation of the epsilon-amino group of the Lys side chain with (2-[2-(2-amino-ethoxy)-ethoxy]-acetyl)2-(gamma-Glu)-CO-(CH2)18-CO 2H
  SITE 30: note = MISC_FEATURE - Gly at position 30 is amidated
YXEGTXTSDYSILLDKIAQXKFIEYLIEGG

SEQ ID NO: 104 - protein, 30 aa, synthetic construct
  REGION 1..30: note = Synthetic Construct
  SITE 2: note = MISC_FEATURE - Xaa at position 2 is Aib
  SITE 6: note = MISC_FEATURE - Xaa at position 6 is alpha-methyl-Phe
  SITE 20: note = MISC_FEATURE - Xaa at position 20 is Aib
  MOD_RES 28: note = Lys at position 28 is chemically modified by conjugation of the epsilon-amino group of the Lys side chain with (2-[2-(2-amino-ethoxy)-ethoxy]-acetyl)2-(gamma-Glu)-CO-(CH2)18-CO 2H
  MOD_RES 30: note = Gly at position 30 is amidated
YXEGTXTSDYSILLDKIAQXAFIEYLIKGG

SEQ ID NO: 105 - protein, 30 aa, synthetic construct
  REGION 1..30: note = Synthetic Construct
  SITE 2: note = MISC_FEATURE - Xaa at position 2 is Aib
  MOD_RES 10: note = Lys at position 10 is chemically modified by conjugation of the epsilon-amino group of the Lys side chain with (2-[2-(2-amino-ethoxy)-ethoxy]-acetyl)2-(gamma-Glu)-CO-(CH2)18-CO 2H
  SITE 13: note = MISC_FEATURE - Xaa at position 13 is alpha-methyl-Leu
  SITE 20: note = MISC_FEATURE - Xaa at position 20 is Aib
  MOD_RES 30: note = Gly at position 30 is amidated
YXEGTFTSDKSIXLDKIAQXAFIEYLIEGG

SEQ ID NO: 106 - protein, 30 aa, synthetic construct
  REGION 1..30: note = Synthetic Construct
  SITE 2: note = MISC_FEATURE - Xaa at position 2 is Aib
  SITE 13: note = MISC_FEATURE - Xaa at position 13 is alpha-methyl-Leu
  SITE 20: note = MISC_FEATURE - Xaa at position 20 is Aib
  MOD_RES 28: note = Lys at position 28 is chemically modified by conjugation of the epsilon-amino group of the Lys side chain with (2-[2-(2-amino-ethoxy)-ethoxy]-acetyl)2-(gamma-Glu)-CO-(CH2)18-CO 2H
  MOD_RES 30: note = Gly at position 30 is amidated
YXEGTFTSDYSIXLDKIAQXAFIEYLIKGG

SEQ ID NO: 107 - protein, 30 aa, synthetic construct
  REGION 1..30: note = Synthetic Construct
  SITE 2: note = MISC_FEATURE - Xaa at position 2 is Aib
  SITE 6: note = MISC_FEATURE - Xaa at position 13 is alpha-methyl-Phe
  MOD_RES 17: note = Lys at position 17 is chemically modified by conjugation of the epsilon-amino group of the Lys side chain with (2-[2-(2-amino-ethoxy)-ethoxy]-acetyl)2-(gamma-Glu)-CO-(CH2)18-CO 2H
  SITE 20: note = MISC_FEATURE - Xaa at position 20 is Aib
  MOD_RES 30: note = Gly at position 30 is amidated
YXEGTXTSDYSILLDKKAQXAFIEYLIEGG

SEQ ID NO: 108 - protein, 30 aa, synthetic construct
  REGION 1..30: note = Synthetic Construct
  SITE 2: note = MISC_FEATURE - Xaa at position 2 is Aib
  SITE 6: note = MISC_FEATURE - Xaa at position 6 is alpha-methyl-Phe
  SITE 13: note = MISC_FEATURE - Xaa at position 13 is alpha-methyl-Leu
  MOD_RES 17: note = Lys at position 17 is chemically modified by conjugation of the epsilon-amino group of the Lys side chain with (2-[2-(2-amino-ethoxy)-ethoxy]-acetyl)2-(gamma-Glu)-CO-(CH2)18-CO 2H
  SITE 20: note = MISC_FEATURE - Xaa at position 20 is Aib
  MOD_RES 30: note = Gly at position 30 is amidated
YXEGTXTSDYSIXLDKKAQXAFIEYLIEGG

SEQ ID NO: 109 - protein, 30 aa, synthetic construct
  REGION 1..30: note = Synthetic Construct
  SITE 2: note = MISC_FEATURE - Xaa at position 2 is Aib
  SITE 6: note = MISC_FEATURE - Xaa at position 6 is alpha-methyl-Phe
  SITE 13: note = MISC_FEATURE - Xaa at position 13 is alpha-methyl-Leu
  MOD_RES 17: note = Lys at position 17 is chemically modified by conjugation of the epsilon-amino group of the Lys side chain with (2-[2-(2-amino-ethoxy)-ethoxy]-acetyl)2-(gamma-Glu)-CO-(CH2)18-CO 2H
  SITE 20: note = MISC_FEATURE - Xaa at position 20 is Aib
  MOD_RES 30: note = Gly at position 30 is amidated
YXEGTXTSDYSIXLDEKAQXAFIEYLIEGG

SEQ ID NO: 110 - protein, 30 aa, synthetic construct; identical to SEQ ID NO: 109
  REGION 1..30: note = Synthetic Construct
  SITE 2: note = MISC_FEATURE - Xaa at position 2 is Aib
  SITE 6: note = MISC_FEATURE - Xaa at position 6 is alpha-methyl-Phe(2F)
  SITE 13: note = MISC_FEATURE - Xaa at position 13 is Aib
  MOD_RES 17: note = Lys at position 17 is chemically modified by conjugation of the epsilon-amino group of the Lys side chain with (2-[2-(2-amino-ethoxy)-ethoxy]-acetyl)2-(gamma-Glu)-CO-(CH2)18-CO 2H
  SITE 20: note = MISC_FEATURE - Xaa at position 20 is Aib
  MOD_RES 30: note = Gly at position 30 is amidated

SEQ ID NO: 111 - protein, 30 aa, synthetic construct; identical to SEQ ID NO: 109
  REGION 1..30: note = Synthetic Construct
  SITE 2: note = MISC_FEATURE - Xaa at position 2 is Aib
  SITE 6: note = MISC_FEATURE - Xaa at position 6 is alpha-methyl-Phe
  SITE 13: note = MISC_FEATURE - Xaa at position 13 is Aib
  MOD_RES 17: note = Lys at position 17 is chemically modified by conjugation of the epsilon-amino group of the Lys side chain with (2-[2-(2-amino-ethoxy)-ethoxy]-acetyl)2-(gamma-Glu)-CO-(CH2)18-CO 2H
  SITE 20: note = MISC_FEATURE - Xaa at position 20 is Aib
  MOD_RES 30: note = Gly at position 30 is amidated

SEQ ID NO: 112 - protein, 30 aa, synthetic construct
  REGION 1..30: note = Synthetic Construct
  SITE 2: note = MISC_FEATURE - Xaa at position 2 is Aib
  SITE 6: note = MISC_FEATURE - Xaa at position 6 is alpha-methyl-Phe(2F)
  SITE 13: note = MISC_FEATURE - Xaa at position 13 is alpha-methyl-Leu
  MOD_RES 17: note = Lys at position 17 is chemically modified by conjugation of the epsilon-amino group of the Lys side chain with (2-[2-(2-amino-ethoxy)-ethoxy]-acetyl)2-(gamma-Glu)-CO-(CH2)18-CO 2H
  SITE 20: note = MISC_FEATURE - Xaa at position 20 is Aib
  MOD_RES 30: note = Gly at position 30 is amidated
YXEGTXTSDYSIXLDEKAQXEFIEYLIEGG

SEQ ID NO: 113 - protein, 30 aa, synthetic construct; identical to SEQ ID NO: 112
  REGION 1..30: note = Synthetic Construct
  SITE 2: note = MISC_FEATURE - Xaa at position 2 is Aib
  SITE 6: note = MISC_FEATURE - Xaa at position 6 is alpha-methyl-Phe(2F)
  SITE 13: note = MISC_FEATURE - Xaa at position 13 is alpha-methyl-Leu
  MOD_RES 17: note = Lys at position 17 is chemically modified by conjugation of the epsilon-amino group of the Lys side chain with (2-[2-(2-amino-ethoxy)-ethoxy]-acetyl)2-(gamma-Glu)-CO-(CH2)16-CO 2H
  SITE 20: note = MISC_FEATURE - Xaa at position 20 is Aib
  MOD_RES 30: note = Gly at position 30 is amidated

SEQ ID NO: 114 - protein, 39 aa, synthetic construct; identical to SEQ ID NO: 87
  REGION 1..39: note = Synthetic Construct
  REGION 1..2: note = MISC_FEATURE - Xaa at position 1 combines with Xaa at position 2 to form desHis-psi[NHCO]-Aib
  MOD_RES 17: note = Lys at position 17 is chemically modified by conjugation of the epsilon-amino group of the Lys side chain with (2-[2-(2-amino-ethoxy)-ethoxy]-acetyl)2-(gamma-Glu)-CO-(CH2)18-CO 2H
  SITE 20: note = MISC_FEATURE - Xaa at position 20 is Aib
  MOD_RES 39: note = Ser at position 39 is amidated

SEQ ID NO: 115 - protein, 39 aa, synthetic construct; identical to SEQ ID NO: 87
  REGION 1..39: note = Synthetic Construct
  REGION 1..2: note = MISC_FEATURE - Xaa at position 1 combines with Xaa at position 2 to form desHis-Aib
  MOD_RES 17: note = Lys at position 17 is chemically modified by conjugation of the epsilon-amino group of the Lys side chain with (2-[2-(2-amino-ethoxy)-ethoxy]-acetyl)2-(gamma-Glu)-CO-(CH2)18-CO 2H
  SITE 20: note = MISC_FEATURE - Xaa at position 20 is Aib
  MOD_RES 39: note = Ser at position 39 is amidated

SEQ ID NO: 116 - protein, 39 aa, synthetic construct; identical to SEQ ID NO: 87
  REGION 1..39: note = Synthetic Construct
  SITE 1: note = MISC_FEATURE - Xaa at position 1 is Des-Tyr
  SITE 2: note = MISC_FEATURE - Xaa at position 2 is Aib
  MOD_RES 17: note = Lys at position 17 is chemically modified by conjugation of the epsilon-amino group of the Lys side chain with (2-[2-(2-amino-ethoxy)-ethoxy]-acetyl)2-(gamma-Glu)-CO-(CH2)18-CO 2H
  SITE 20: note = MISC_FEATURE - Xaa at position 20 is Aib
  MOD_RES 39: note = Ser at position 39 is amidated

SEQ ID NO: 117 - protein, 39 aa, synthetic construct; identical to SEQ ID NO: 17
  REGION 1..39: note = Synthetic Construct
  SITE 2: note = MISC_FEATURE - Xaa at position 2 is Aib
  MOD_RES 17: note = Lys at position 17 is chemically modified by conjugation of the epsilon-amino group of the Lys side chain with (2-[2-(2-amino-ethoxy)-ethoxy]-acetyl)-AOC-(gamma-Glu)-CO-(CH2)18 -CO2H
  SITE 20: note = MISC_FEATURE - Xaa at position 20 is Aib
  MOD_RES 39: note = Ser at position 39 is amidated

SEQ ID NO: 118 - protein, 39 aa, synthetic construct; identical to SEQ ID NO: 17
  REGION 1..39: note = Synthetic Construct
  SITE 2: note = MISC_FEATURE - Xaa at position 2 is Aib
  MOD_RES 17: note = Lys at position 17 is chemically modified by conjugation of the epsilon-amino group of the Lys side chain with AOC-(2-[2-(2-amino-ethoxy)-ethoxy]-acetyl)-(gamma-Glu)-CO-(CH2)18 -CO2H
  SITE 20: note = MISC_FEATURE - Xaa at position 20 is Aib
  MOD_RES 39: note = Ser at position 39 is amidated

SEQ ID NO: 119 - protein, 39 aa, synthetic construct; identical to SEQ ID NO: 17
  REGION 1..39: note = Synthetic Construct
  SITE 2: note = MISC_FEATURE - Xaa at position 2 is Aib
  MOD_RES 17: note = Lys at position 17 is chemically modified by conjugation of the epsilon-amino group of the Lys side chain with (2-[2-(2-amino-ethoxy)-ethoxy]-acetyl)-(gamma-Glu)-(Trx)-CO-(CH2) 18-CO2H
  SITE 20: note = MISC_FEATURE - Xaa at position 20 is Aib
  MOD_RES 39: note = Ser at position 39 is amidated

SEQ ID NO: 120 - protein, 39 aa, synthetic construct; identical to SEQ ID NO: 17
  REGION 1..39: note = Synthetic Construct
  SITE 2: note = MISC_FEATURE - Xaa at position 2 is Aib
  MOD_RES 17: note = Lys at position 17 is chemically modified by conjugation of the epsilon-amino group of the Lys side chain with (2-[2-(2-amino-ethoxy)-ethoxy]-acetyl)-(Trx)-(gamma-Glu)-CO-(CH2) 18-CO2H
  SITE 20: note = MISC_FEATURE - Xaa at position 20 is Aib
  MOD_RES 39: note = Ser at position 39 is amidated

SEQ ID NO: 121 - protein, 39 aa, synthetic construct; identical to SEQ ID NO: 17
  REGION 1..39: note = Synthetic Construct
  SITE 2: note = MISC_FEATURE - Xaa at position 2 is Aib
  MOD_RES 17: note = Lys at position 17 is chemically modified by conjugation of the epsilon-amino group of the Lys side chain with (2-[2-(2-amino-ethoxy)-ethoxy]-acetyl)-(epsilon-Lys)-(gamma-Glu)- CO-(CH2)18-CO2H
  SITE 20: note = MISC_FEATURE - Xaa at position 20 is Aib
  MOD_RES 39: note = Ser at position 39 is amidated

SEQ ID NO: 122 - protein, 39 aa, synthetic construct; identical to SEQ ID NO: 17
  REGION 1..39: note = Synthetic Construct
  SITE 2: note = MISC_FEATURE - Xaa at position 2 is Aib
  MOD_RES 17: note = Lys at position 17 is chemically modified by conjugation of the epsilon-amino group of the Lys side chain with (2-[2-(2-amino-ethoxy)-ethoxy]-acetyl)2-(epsilon-Lys)-CO-(CH2)18- CO2H
  SITE 20: note = MISC_FEATURE - Xaa at position 20 is Aib
  MOD_RES 39: note = Ser at position 39 is amidated

SEQ ID NO: 123 - protein, 39 aa, synthetic construct; identical to SEQ ID NO: 17
  REGION 1..39: note = Synthetic Construct
  SITE 2: note = MISC_FEATURE - Xaa at position 2 is Aib
  MOD_RES 17: note = Lys at position 17 is chemically modified by conjugation of the epsilon-amino group of the Lys side chain with (2-[2-(2-amino-ethoxy)-ethoxy]-acetyl)-(epsilon-Lys)-(epsilon-Lys )-CO-(CH2)18-CO2H
  SITE 20: note = MISC_FEATURE - Xaa at position 2 is Aib
  MOD_RES 39: note = Ser at position 39 is amidated

SEQ ID NO: 124 - protein, 39 aa, synthetic construct
  REGION 1..39: note = Synthetic Construct
  SITE 2: note = MISC_FEATURE - Xaa at position 2 is Aib
  SITE 6: note = MISC_FEATURE - Xaa at position 6 is alpha-methyl-Phe
  SITE 13: note = MISC_FEATURE - Xaa at position 13 is alpha-methyl-Leu
  MOD_RES 17: note = Lys at position 17 is chemically modified by conjugation of the epsilon-amino group of the Lys side chain with (2-[2-(2-amino-ethoxy)-ethoxy]-acetyl)2-(gamma-Glu)-CO-(CH2)18-CO 2H
  SITE 20: note = MISC_FEATURE - Xaa at position 20 is Aib
  MOD_RES 39: note = Ser at position 39 is amidated
YXEGTXTSDYSIXLDEKAQXAFIEYLIEGGPSSGAPPPS

SEQ ID NO: 125 - protein, 39 aa, synthetic construct
  REGION 1..39: note = Synthetic Construct
  SITE 2: note = MISC_FEATURE - Xaa at position 2 is Aib
  SITE 6: note = MISC_FEATURE - Xaa at position 6 is alpha-methyl-Phe
  SITE 13: note = MISC_FEATURE - Xaa at position 13 is alpha-methyl-Leu
  MOD_RES 17: note = Lys at position 17 is chemically modified by conjugation of the epsilon-amino group of the Lys side chain with (2-[2-(2-amino-ethoxy)-ethoxy]-acetyl)2-(gamma-Glu)-CO-(CH2)18-CO 2H
  SITE 20: note = MISC_FEATURE - Xaa at position 20 is Aib
  MOD_RES 39: note = Ser at position 39 is amidated
YXEGTXTSDYSIXLDEKAQXEFIEYLIEGGPSSGAPPPS

SEQ ID NO: 126 - protein, 39 aa, synthetic construct; identical to SEQ ID NO: 124
  REGION 1..39: note = Synthetic Construct
  SITE 2: note = MISC_FEATURE - Xaa at position 2 is Aib
  SITE 6: note = MISC_FEATURE - Xaa at position 6 is alpha-methyl-Phe
  SITE 13: note = MISC_FEATURE - Xaa at position 13 is Aib
  MOD_RES 17: note = Lys at position 17 is chemically modified by conjugation of the epsilon-amino group of the Lys side chain with (2-[2-(2-amino-ethoxy)-ethoxy]-acetyl)2-(gamma-Glu)-CO-(CH2)18-CO 2H
  SITE 20: note = MISC_FEATURE - Xaa at position 20 is Aib
  MOD_RES 39: note = Ser at position 39 is amidated

SEQ ID NO: 127 - protein, 39 aa, synthetic construct; identical to SEQ ID NO: 125
  REGION 1..39: note = Synthetic Construct
  SITE 2: note = MISC_FEATURE - Xaa at position 2 is Aib
  SITE 6: note = MISC_FEATURE - Xaa at position 6 is alpha-methyl-Phe(2F)
  SITE 13: note = MISC_FEATURE - Xaa at position 13 is alpha-methyl-Leu
  MOD_RES 17: note = Lys at position 17 is chemically modified by conjugation of the epsilon-amino group of the Lys side chain with (2-[2-(2-amino-ethoxy)-ethoxy]-acetyl)2-(gamma-Glu)-CO-(CH2)18-CO 2H
  SITE 20: note = MISC_FEATURE - Xaa at position 20 is Aib
  MOD_RES 39: note = Ser at position 39 is amidated

SEQ ID NO: 128 - protein, 39 aa, synthetic construct
  REGION 1..39: note = Synthetic Construct
  SITE 2: note = MISC_FEATURE - Xaa at position 2 is Aib
  SITE 6: note = MISC_FEATURE - Xaa at position 6 is alpha-methyl-Phe
  SITE 13: note = MISC_FEATURE - Xaa at position 13 is alpha-methyl-Leu
  MOD_RES 17: note = Lys at position 17 is chemically modified by conjugation of the epsilon-amino group of the Lys side chain with (2-[2-(2-amino-ethoxy)-ethoxy]-acetyl)2-(gamma-Glu)-CO-(CH2)18-CO 2H
  SITE 20: note = MISC_FEATURE - Xaa at position 20 is Aib
  MOD_RES 39: note = Ser at position 39 is amidated
FXEGTXTSDYSIXLDEKAQXAFIEYLIEGGPSSGAPPPS

SEQ ID NO: 129 - protein, 39 aa, synthetic construct
  REGION 1..39: note = Synthetic Construct
  SITE 2: note = MISC_FEATURE - Xaa at position 2 is Aib
  SITE 3: note = MISC_FEATURE - Xaa at position 3 is cTA
  SITE 6: note = MISC_FEATURE - Xaa at position 6 is alpha-methyl-Phe
  SITE 13: note = MISC_FEATURE - Xaa at position 13 is alpha-methyl-Leu
  MOD_RES 17: note = Lys at position 17 is chemically modified by conjugation of the epsilon-amino group of the Lys side chain with (2-[2-(2-amino-ethoxy)-ethoxy]-acetyl)2-(gamma-Glu)-CO-(CH2)18-CO 2H
  SITE 20: note = MISC_FEATURE - Xaa at position 20 is Aib
  MOD_RES 39: note = Ser at position 39 is amidated
YXXGTXTSDYSIXLDEKAQXAFIEYLIEGGPSSGAPPPS

SEQ ID NO: 130 - protein, 39 aa, synthetic construct
  REGION 1..39: note = Synthetic Construct
  SITE 2: note = MISC_FEATURE - Xaa at position 2 is Aib
  SITE 6: note = MISC_FEATURE - Xaa at position 6 is alpha-methyl-Phe
  SITE 13: note = MISC_FEATURE - Xaa at position 13 is alpha-methyl-Leu
  MOD_RES 17: note = Lys at position 17 is chemically modified by conjugation of the epsilon-amino group of the Lys side chain with (2-[2-(2-amino-ethoxy)-ethoxy]-acetyl)2-(gamma-Glu)-CO-(CH2)18-CO 2H
  MOD_RES 39: note = Ser at position 39 is amidated
YXEGTXTSDYSIXLDEKAQQAFIEYLIEGGPSSGAPPPS

SEQ ID NO: 131 - protein, 39 aa, synthetic construct
  REGION 1..39: note = Synthetic Construct
  SITE 2: note = MISC_FEATURE - Xaa at position 2 is Aib
  SITE 6: note = MISC_FEATURE - Xaa at position 6 is alpha-methyl-Phe
  SITE 13: note = MISC_FEATURE - Xaa at position 13 is alpha-methyl-Leu
  MOD_RES 17: note = Lys at position 17 is chemically modified by conjugation of the epsilon-amino group of the Lys side chain with (2-[2-(2-amino-ethoxy)-ethoxy]-acetyl)2-(gamma-Glu)-CO-(CH2)18-CO 2H
  SITE 29: note = MISC_FEATURE - Xaa at position 29 is Aib
  MOD_RES 39: note = Ser at position 39 is amidated
YXEGTXTSDYSIXLDEKAQQAFIEYLIEXGPSSGAPPPS

SEQ ID NO: 132 - protein, 34 aa, synthetic construct
  REGION 1..34: note = Synthetic Construct
  SITE 2: note = MISC_FEATURE - Xaa at position 2 is Aib
  SITE 6: note = MISC_FEATURE - Xaa at position 6 is alpha-methyl-Phe
  SITE 13: note = MISC_FEATURE - Xaa at position 13 is alpha-methyl-Leu
  MOD_RES 17: note = Lys at position 17 is chemically modified by conjugation of the epsilon-amino group of the Lys side chain with (2-[2-(2-amino-ethoxy)-ethoxy]-acetyl)2-(gamma-Glu)-CO-(CH2)18-CO 2H
  SITE 20: note = MISC_FEATURE - Xaa at position 20 is Aib
  MOD_RES 34: note = Gly at position 34 is amidated
YXEGTXTSDYSIXLDKKAQXEFIEYLIEGGPSSG

SEQ ID NO: 133 - protein, 34 aa, synthetic construct
  REGION 1..34: note = Synthetic Construct
  SITE 2: note = MISC_FEATURE - Xaa at position 2 is Aib
  SITE 6: note = MISC_FEATURE - Xaa at position 6 is alpha-methyl-Phe
  SITE 13: note = MISC_FEATURE - Xaa at position 13 is alpha-methyl-Leu
  MOD_RES 17: note = Lys at position 17 is chemically modified by conjugation of the epsilon-amino group of the Lys side chain with (2-[2-(2-amino-ethoxy)-ethoxy]-acetyl)2-(gamma-Glu)-CO-(CH2)18-CO 2H
  SITE 20: note = MISC_FEATURE - Xaa at position 20 is Aib
  MOD_RES 34: note = Gly at position 34 is amidated
YXEGTXTSDYSIXLDEKAQXEFIEYLIEGGPSSG

SEQ ID NO: 134 - protein, 39 aa, synthetic construct; identical to SEQ ID NO: 78
  REGION 1..39: note = Synthetic Construct
  SITE 2: note = MISC_FEATURE - Xaa at position 2 is Aib
  SITE 6: note = MISC_FEATURE - Xaa at position 6 is alpha-methyl-Phe
  SITE 13: note = MISC_FEATURE - Xaa at position 13 is alpha-methyl-Leu
  MOD_RES 17: note = Lys at position 17 is chemically modified by conjugation of the epsilon-amino group of the Lys side chain with (2-[2-(2-amino-ethoxy)-ethoxy]-acetyl)2-(gamma-Glu)2-CO-(CH2)18-C O2H
  SITE 20: note = MISC_FEATURE - Xaa at position 20 is Aib
  MOD_RES 39: note = Ser at position 39 is amidated

SEQ ID NO: 135 - protein, 39 aa, synthetic construct
  REGION 1..39: note = Synthetic Construct
  SITE 2: note = MISC_FEATURE - Xaa at position 2 is Aib
  SITE 6: note = MISC_FEATURE - Xaa at position 6 is alpha-methyl-Phe
  SITE 13: note = MISC_FEATURE - Xaa at position 13 is alpha-methyl-Leu
  MOD_RES 17: note = Lys at position 17 is chemically modified by conjugation of the epsilon-amino group of the Lys side chain with (2-[2-(2-amino-ethoxy)-ethoxy]-acetyl)2-(gamma-Glu)-CO-(CH2)18-CO 2H
  SITE 20: note = MISC_FEATURE - Xaa at position 20 is Aib
  MOD_RES 39: note = Ser at position 39 is amidated
YXEGTXTSDYSIXLDKKAQXAFIEYLIEAGPSSGAPPPS

SEQ ID NO: 136 - protein, 39 aa, synthetic construct
  REGION 1..39: note = Synthetic Construct
  SITE 2: note = MISC_FEATURE - Xaa at position 2 is Aib
  SITE 6: note = MISC_FEATURE - Xaa at position 6 is alpha-methyl-Phe
  MOD_RES 17: note = Lys at position 17 is chemically modified by conjugation of the epsilon-amino group of the Lys side chain with (2-[2-(2-amino-ethoxy)-ethoxy]-acetyl)2-(gamma-Glu)-CO-(CH2)18-CO 2H
  SITE 20: note = MISC_FEATURE - Xaa at position 20 is Aib
  MOD_RES 39: note = Ser at position 39 is amidated
YXEGTXTSDISILLDKKAQXAFIEYLIEGGPSSGAPPPS

SEQ ID NO: 137 - protein, 39 aa, synthetic construct
  REGION 1..39: note = Synthetic Construct
  SITE 2: note = MISC_FEATURE - Xaa at position 2 is Aib
  SITE 6: note = MISC_FEATURE - Xaa at position 6 is alpha-methyl-Phe
  MOD_RES 17: note = Lys at position 17 is chemically modified by conjugation of the epsilon-amino group of the Lys side chain with (2-[2-(2-amino-ethoxy)-ethoxy]-acetyl)2-(gamma-Glu)-CO-(CH2)18-CO 2H
  SITE 20: note = MISC_FEATURE - Xaa at position 20 is Aib
  MOD_RES 39: note = Ser at position 39 is amidated
YXEGTXTSDHSILLDKKAQXAFIEYLIEGGPSSGAPPPS

SEQ ID NO: 138 - protein, 39 aa, synthetic construct
  REGION 1..39: note = Synthetic Construct
  SITE 2: note = MISC_FEATURE - Xaa at position 2 is Aib
  SITE 6: note = MISC_FEATURE - Xaa at position 6 is alpha-methyl-Phe
  MOD_RES 17: note = Lys at position 17 is chemically modified by conjugation of the epsilon-amino group of the Lys side chain with (2-[2-(2-amino-ethoxy)-ethoxy]-acetyl)2-(gamma-Glu)-CO-(CH2)18-CO 2H
  SITE 20: note = MISC_FEATURE - Xaa at position 20 is Aib
  MOD_RES 39: note = Ser at position 39 is amidated
YXEGTXTSDLSILLDKKAQXAFIEYLIEGGPSSGAPPPS

SEQ ID NO: 139 - protein, 39 aa, synthetic construct
  REGION 1..39: note = Synthetic Construct
  SITE 2: note = MISC_FEATURE - Xaa at position 2 is Aib
  SITE 6: note = MISC_FEATURE - Xaa at position 6 is alpha-methyl-Phe
  MOD_RES 17: note = Lys at position 17 is chemically modified by conjugation of the epsilon-amino group of the Lys side chain with (2-[2-(2-amino-ethoxy)-ethoxy]-acetyl)2-(gamma-Glu)-CO-(CH2)18-CO 2H
  SITE 20: note = MISC_FEATURE - Xaa at position 20 is Aib
  MOD_RES 39: note = Ser at position 39 is amidated
YXEGTXTSDESILLDKKAQXAFIEYLIEGGPSSGAPPPS

SEQ ID NO: 140 - protein, 39 aa, synthetic construct
  REGION 1..39: note = Synthetic Construct
  SITE 2: note = MISC_FEATURE - Xaa at position 2 is Aib
  SITE 6: note = MISC_FEATURE - Xaa at position 6 is alpha-methyl-Phe
  SITE 10: note = MISC_FEATURE - Xaa at position 10 is alpha-methyl-Phe
  MOD_RES 17: note = Lys at position 17 is chemically modified by conjugation of the epsilon-amino group of the Lys side chain with (2-[2-(2-amino-ethoxy)-ethoxy]-acetyl)2-(gamma-Glu)-CO-(CH2)18-CO 2H
  SITE 20: note = MISC_FEATURE - Xaa at position 20 is Aib
  MOD_RES 39: note = Ser at position 39 is amidated
YXEGTXTSDXSILLDKKAQXAFIEYLIEGGPSSGAPPPS

SEQ ID NO: 141 - protein, 39 aa, synthetic construct; identical to SEQ ID NO: 140
  REGION 1..39: note = Synthetic Construct
  SITE 2: note = MISC_FEATURE - Xaa at position 2 is Aib
  SITE 6: note = MISC_FEATURE - Xaa at position 6 is alpha-methyl-Phe
  SITE 10: note = MISC_FEATURE - Xaa at position 10 is 3Pal
  MOD_RES 17: note = Lys at position 17 is chemically modified by conjugation of the epsilon-amino group of the Lys side chain with (2-[2-(2-amino-ethoxy)-ethoxy]-acetyl)2-(gamma-Glu)-CO-(CH2)18-CO 2H
  SITE 20: note = MISC_FEATURE - Xaa at position 20 is Aib
  MOD_RES 39: note = Ser at position 39 is amidated

SEQ ID NO: 142 - protein, 39 aa, synthetic construct
  REGION 1..39: note = Synthetic Construct
  SITE 1: note = MISC_FEATURE - Xaa at position 1 is DesTyr
  SITE 2: note = MISC_FEATURE - Xaa at position 2 is Aib
  SITE 6: note = MISC_FEATURE - Xaa at position 6 is alpha-methyl-Phe
  SITE 13: note = MISC_FEATURE - Xaa at position 13 is Aib
  MOD_RES 17: note = Lys at position 17 is chemically modified by conjugation of the epsilon-amino group of the Lys side chain with (2-[2-(2-amino-ethoxy)-ethoxy]-acetyl)2-(gamma-Glu)-CO-(CH2)18-CO 2H
  SITE 20: note = MISC_FEATURE - Xaa at position 20 is Aib
  MOD_RES 39: note = Ser at position 39 is amidated
XXEGTXTSDYSIXLDEKAQXAFIEYLIEGGPSSGAPPPS

SEQ ID NO: 143 - protein, 39 aa, synthetic construct
  REGION 1..39: note = Synthetic Construct
  SITE 1: note = MISC_FEATURE - Xaa at position 1 is DesTyr
  SITE 2: note = MISC_FEATURE - Xaa at position 2 is Aib
  SITE 6: note = MISC_FEATURE - Xaa at position 6 is alpha-methyl-Phe(2F)
  SITE 13: note = MISC_FEATURE - Xaa at position 13 is alpha-methyl-Leu
  MOD_RES 17: note = Lys at position 17 is chemically modified by conjugation of the epsilon-amino group of the Lys side chain with (2-[2-(2-amino-ethoxy)-ethoxy]-acetyl)2-(gamma-Glu)-CO-(CH2)18-CO 2H
  SITE 20: note = MISC_FEATURE - Xaa at position 20 is Aib
  MOD_RES 39: note = Ser at position 39 is amidated
XXEGTXTSDYSIXLDEKAQXEFIEYLIEGGPSSGAPPPS

SEQ ID NO: 144 - protein, 39 aa, synthetic construct
  REGION 1..39: note = Synthetic Construct
  SITE 2: note = MISC_FEATURE - Xaa at position 2 is Aib
  MOD_RES 17: note = Lys at position 17 is chemically modified by conjugation of the epsilon-amino group of the Lys side chain with (2-[2-(2-amino-ethoxy)-ethoxy]-acetyl)2-(gamma-Glu)-CO-(CH2)18-CO 2H
  SITE 20: note = MISC_FEATURE - Xaa at position 20 is Aib
  MOD_RES 39: note = Ser at position 39 is amidated
HXNGTFTSDYSILLDKKAQXAFIEYLIEGGPSSGAPPPS

SEQ ID NO: 145 - protein, 39 aa, synthetic construct
  REGION 1..39: note = Synthetic Construct
  SITE 2: note = MISC_FEATURE - Xaa at position 2 is Aib
  MOD_RES 17: note = Lys at position 17 is chemically modified by conjugation of the epsilon-amino group of the Lys side chain with (2-[2-(2-amino-ethoxy)-ethoxy]-acetyl)2-(gamma-Glu)-CO-(CH2)18-CO 2H
  SITE 20: note = MISC_FEATURE - Xaa at position 20 is Aib
  MOD_RES 39: note = Ser at position 39 is amidated
YXEGTFTSDASILLDKKAQXAFIEYLIEAGPSSGAPPPS

SEQ ID NO: 146 - protein, 39 aa, synthetic construct
  REGION 1..39: note = Synthetic Construct
  SITE 2: note = MISC_FEATURE - Xaa at position 2 is Aib
  SITE 6: note = MISC_FEATURE - Xaa at position 6 is alpha-methyl-Phe
  SITE 13: note = MISC_FEATURE - Xaa at position 13 is alpha-methyl-Leu
  MOD_RES 17: note = Lys at position 17 is chemically modified by conjugation of the epsilon-amino group of the Lys side chain with (2-[2-(2-amino-ethoxy)-ethoxy]-acetyl)2-(gamma-Glu)-CO-(CH2)18-CO 2H
  SITE 20: note = MISC_FEATURE - Xaa at position 20 is Aib
  SITE 21: note = MISC_FEATURE - Xaa at position 21 is Aad
  MOD_RES 39: note = Ser at position 39 is amidated
YXEGTXTSDYSIXLDKKAQXXFIEYLIEGGPSSGAPPPS

SEQ ID NO: 147 - protein, 39 aa, synthetic construct
  REGION 1..39: note = Synthetic Construct
  SITE 2: note = MISC_FEATURE - Xaa at position 2 is Aib
  SITE 6: note = MISC_FEATURE - Xaa at position 6 is alpha-methyl-Phe
  SITE 13: note = MISC_FEATURE - Xaa at position 13 is alpha-methyl-Leu
  MOD_RES 17: note = Lys at position 17 is chemically modified by conjugation of the epsilon-amino group of the Lys side chain with (2-[2-(2-amino-ethoxy)-ethoxy]-acetyl)2-(gamma-Glu)-CO-(CH2)18-CO 2H
  SITE 20: note = MISC_FEATURE - Xaa at position 20 is Aib
  MOD_RES 39: note = Ser at position 39 is amidated
YXEGTXTSDYSIXLDKKAQXSFIEYLIEGGPSSGAPPPS

SEQ ID NO: 148 - protein, 39 aa, synthetic construct
  REGION 1..39: note = Synthetic Construct
  SITE 2: note = MISC_FEATURE - Xaa at position 2 is Aib
  SITE 6: note = MISC_FEATURE - Xaa at position 6 is alpha-methyl-Phe
  SITE 13: note = MISC_FEATURE - Xaa at position 13 is alpha-methyl-Leu
  MOD_RES 17: note = Lys at position 17 is chemically modified by conjugation of the epsilon-amino group of the Lys side chain with (2-[2-(2-amino-ethoxy)-ethoxy]-acetyl)2-(gamma-Glu)-CO-(CH2)18-CO 2H
  SITE 20: note = MISC_FEATURE - Xaa at position 20 is Aib
  MOD_RES 39: note = Ser at position 39 is amidated
YXEGTXTSDYSIXLDKKAQXTFIEYLIEGGPSSGAPPPS

SEQ ID NO: 149 - protein, 39 aa, synthetic construct
  REGION 1..39: note = Synthetic Construct
  SITE 2: note = MISC_FEATURE - Xaa at position 2 is Aib
  SITE 6: note = MISC_FEATURE - Xaa at position 6 is alpha-methyl-Phe
  SITE 13: note = MISC_FEATURE - Xaa at position 13 is alpha-methyl-Leu
  MOD_RES 17: note = Lys at position 17 is chemically modified by conjugation of the epsilon-amino group of the Lys side chain with (2-[2-(2-amino-ethoxy)-ethoxy]-acetyl)2-(gamma-Glu)-CO-(CH2)18-CO 2H
  SITE 20: note = MISC_FEATURE - Xaa at position 20 is Aib
  MOD_RES 39: note = Ser at position 39 is amidated
YXEGTXTSDYSIXLDKKAQXDFIEYLIEGGPSSGAPPPS

SEQ ID NO: 150 - protein, 39 aa, synthetic construct
  REGION 1..39: note = Synthetic Construct
  SITE 2: note = MISC_FEATURE - Xaa at position 2 is Aib
  SITE 6: note = MISC_FEATURE - Xaa at position 6 is alpha-methyl-Phe
  SITE 13: note = MISC_FEATURE - Xaa at position 13 is alpha-methyl-Leu
  MOD_RES 17: note = Lys at position 17 is chemically modified by conjugation of the epsilon-amino group of the Lys side chain with (2-[2-(2-amino-ethoxy)-ethoxy]-acetyl)2-(gamma-Glu)-CO-(CH2)18-CO 2H
  SITE 20: note = MISC_FEATURE - Xaa at position 20 is Aib
  MOD_RES 39: note = Ser at position 39 is amidated
YXEGTXTSDYSIXLDKKAQXIFIEYLIEGGPSSGAPPPS

SEQ ID NO: 151 - protein, 39 aa, synthetic construct
  REGION 1..39: note = Synthetic Construct
  SITE 2: note = MISC_FEATURE - Xaa at position 2 is Aib
  SITE 6: note = MISC_FEATURE - Xaa at position 6 is alpha-methyl-Phe
  SITE 13: note = MISC_FEATURE - Xaa at position 13 is alpha-methyl-Leu
  MOD_RES 17: note = Lys at position 17 is chemically modified by conjugation of the epsilon-amino group of the Lys side chain with (2-[2-(2-amino-ethoxy)-ethoxy]-acetyl)2-(gamma-Glu)-CO-(CH2)18-CO 2H
  SITE 20: note = MISC_FEATURE - Xaa at position 2 is Aib
  MOD_RES 39: note = Ser at position 39 is amidated
YXEGTXTSDYSIXLDKKAQXHFIEYLIEGGPSSGAPPPS

SEQ ID NO: 152 - protein, 39 aa, synthetic construct; identical to SEQ ID NO: 146
  REGION 1..39: note = Synthetic Construct
  SITE 2: note = MISC_FEATURE - Xaa at position 2 is Aib
  SITE 6: note = MISC_FEATURE - Xaa at position 6 is alpha-methyl-Phe
  SITE 13: note = MISC_FEATURE - Xaa at position 13 is alpha-methyl-Leu
  MOD_RES 17: note = Lys at position 17 is chemically modified by conjugation of the epsilon-amino group of the Lys side chain with (2-[2-(2-amino-ethoxy)-ethoxy]-acetyl)2-(gamma-Glu)-CO-(CH2)18-CO 2H
  SITE 20: note = MISC_FEATURE - Xaa at position 20 is Aib
  SITE 21: note = MISC_FEATURE - Xaa at position 21 is Aib
  MOD_RES 39: note = Ser at position 39 is amidated

SEQ ID NO: 153 - protein, 39 aa, synthetic construct
  REGION 1..39: note = Synthetic Construct
  SITE 2: note = MISC_FEATURE - Xaa at position 2 is Aib
  SITE 6: note = MISC_FEATURE - Xaa at position 6 is alpha-methyl-Phe
  SITE 13: note = MISC_FEATURE - Xaa at position 13 is alpha-methyl-Leu
  MOD_RES 17: note = Lys at position 17 is chemically modified by conjugation of the epsilon-amino group of the Lys side chain with (2-[2-(2-amino-ethoxy)-ethoxy]-acetyl)2-(gamma-Glu)-CO-(CH2)18-CO 2H
  SITE 21: note = MISC_FEATURE - Xaa at position 21 is Aib
  MOD_RES 39: note = Ser at position 39 is amidated
YXEGTXTSDYSIXLDKKAQHXFIEYLIEGGPSSGAPPPS

SEQ ID NO: 154 - protein, 39 aa, synthetic construct
  REGION 1..39: note = Synthetic Construct
  SITE 2: note = MISC_FEATURE - Xaa at position 2 is Aib
  SITE 6: note = MISC_FEATURE - Xaa at position 6 is alpha-methyl-Phe
  SITE 13: note = MISC_FEATURE - Xaa at position 13 is alpha-methyl-Leu
  MOD_RES 17: note = Lys at position 17 is chemically modified by conjugation of the epsilon-amino group of the Lys side chain with (2-[2-(2-amino-ethoxy)-ethoxy]-acetyl)2-(gamma-Glu)-CO-(CH2)18-CO 2H
  SITE 20: note = MISC_FEATURE - Xaa at position 20 is Aib
  MOD_RES 39: note = Ser at position 39 is amidated
YXEGTXTSDASIXLDKKAQXAFIEYLIEGGPSSGAPPPS

SEQ ID NO: 155 - protein, 39 aa, synthetic construct
  REGION 1..39: note = Synthetic Construct
  SITE 2: note = MISC_FEATURE - Xaa at position 2 is Aib
  SITE 6: note = MISC_FEATURE - Xaa at position 6 is alpha-methyl-Phe(2F)
  SITE 13: note = MISC_FEATURE - Xaa at position 13 is alpha-methyl-Leu
  MOD_RES 17: note = Lys at position 17 is chemically modified by conjugation of the epsilon-amino group of the Lys side chain with (2-[2-(2-amino-ethoxy)-ethoxy]-acetyl)2-(gamma-Glu)-CO-(CH2)18-CO 2H
  SITE 20: note = MISC_FEATURE - Xaa at position 20 is Aib
  MOD_RES 39: note = Ser at position 39 is amidated
YXEGTXTSDYSIXLDEKAQXEFIQYLIEGGPSSGAPPPS

SEQ ID NO: 156 - protein, 39 aa, synthetic construct; identical to SEQ ID NO: 10
  REGION 1..39: note = Synthetic Construct
  SITE 2: note = MISC_FEATURE - Xaa at position 2 is Aib
  SITE 6: note = MISC_FEATURE - Xaa at position 6 is alpha-methyl-Phe(2F)
  SITE 13: note = MISC_FEATURE - Xaa at position 13 is alpha-methyl-Leu
  MOD_RES 17: note = Lys at position 17 is chemically modified by conjugation of the epsilon-amino group of the Lys side chain with (2-[2-(2-amino-ethoxy)-ethoxy]-acetyl)2-(gamma-Glu)-CO-(CH2)18-CO 2H
  SITE 20: note = MISC_FEATURE - Xaa at position 20 is Aib
  SITE 24: note = MISC_FEATURE - Xaa at position 24 is Aad
  MOD_RES 39: note = Ser at position 39 is amidated

SEQ ID NO: 157 - protein, 39 aa, synthetic construct
  REGION 1..39: note = Synthetic Construct
  SITE 2: note = MISC_FEATURE - Xaa at position 2 is Aib
  SITE 6: note = MISC_FEATURE - Xaa at position 6 is alpha-methyl-Phe(2F)
  SITE 13: note = MISC_FEATURE - Xaa at position 13 is alpha-methyl-Leu
  MOD_RES 17: note = Lys at position 17 is chemically modified by conjugation of the epsilon-amino group of the Lys side chain with (2-[2-(2-amino-ethoxy)-ethoxy]-acetyl)2-(gamma-Glu)-CO-(CH2)18-CO 2H
  SITE 20: note = MISC_FEATURE - Xaa at position 20 is Aib
  MOD_RES 39: note = Ser at position 39 is amidated
YXEGTXTSDYSIXLDEKAQXEFIAYLIEGGPSSGAPPPS

SEQ ID NO: 158 - protein, 39 aa, synthetic construct
  REGION 1..39: note = Synthetic Construct
  SITE 2: note = MISC_FEATURE - Xaa at position 2 is Aib
  SITE 6: note = MISC_FEATURE - Xaa at position 6 is alpha-methyl-Phe(2F)
  SITE 13: note = MISC_FEATURE - Xaa at position 13 is alpha-methyl-Leu
  MOD_RES 17: note = Lys at position 17 is chemically modified by conjugation of the epsilon-amino group of the Lys side chain with (2-[2-(2-amino-ethoxy)-ethoxy]-acetyl)2-(gamma-Glu)-CO-(CH2)18-CO 2H
  SITE 20: note = MISC_FEATURE - Xaa at position 20 is Aib
  MOD_RES 39: note = Ser at position 39 is amidated
YXEGTXTSDYSIXLDEKAQXEFIVYLIEGGPSSGAPPPS

SEQ ID NO: 159 - protein, 39 aa, synthetic construct
  REGION 1..39: note = Synthetic Construct
  SITE 2: note = MISC_FEATURE - Xaa at position 2 is Aib
  SITE 6: note = MISC_FEATURE - Xaa at position 6 is alpha-methyl-Phe(2F)
  SITE 13: note = MISC_FEATURE - Xaa at position 13 is alpha-methyl-Leu
  MOD_RES 17: note = Lys at position 17 is chemically modified by conjugation of the epsilon-amino group of the Lys side chain with (2-[2-(2-amino-ethoxy)-ethoxy]-acetyl)2-(gamma-Glu)-CO-(CH2)18-CO 2H
  SITE 20: note = MISC_FEATURE - Xaa at position 20 is Aib
  MOD_RES 39: note = Ser at position 39 is amidated
YXEGTXTSDYSIXLDEKAQXEFISYLIEGGPSSGAPPPS

SEQ ID NO: 160 - protein, 39 aa, synthetic construct
  REGION 1..39: note = Synthetic Construct
  SITE 2: note = MISC_FEATURE - Xaa at position 2 is Aib
  SITE 6: note = MISC_FEATURE - Xaa at position 6 is alpha-methyl-Phe(2F)
  SITE 13: note = MISC_FEATURE - Xaa at position 13 is alpha-methyl-Leu
  MOD_RES 17: note = Lys at position 17 is chemically modified by conjugation of the epsilon-amino group of the Lys side chain with (2-[2-(2-amino-ethoxy)-ethoxy]-acetyl)2-(gamma-Glu)-CO-(CH2)18-CO 2H
  SITE 20: note = MISC_FEATURE - Xaa at position 20 is Aib
  MOD_RES 39: note = Ser at position 39 is amidated
YXEGTXTSDYSIXLDEKAQXEFIPYLIEGGPSSGAPPPS

SEQ ID NO: 161 - protein, 39 aa, synthetic construct; identical to SEQ ID NO: 10
  REGION 1..39: note = Synthetic Construct
  SITE 2: note = MISC_FEATURE - Xaa at position 2 is Aib
  SITE 6: note = MISC_FEATURE - Xaa at position 6 is alpha-methyl-Phe(2F)
  SITE 13: note = MISC_FEATURE - Xaa at position 13 is alpha-methyl-Leu
  MOD_RES 17: note = Lys at position 17 is chemically modified by conjugation of the epsilon-amino group of the Lys side chain with (2-[2-(2-amino-ethoxy)-ethoxy]-acetyl)2-(gamma-Glu)-CO-(CH2)18-CO 2H
  SITE 20: note = MISC_FEATURE - Xaa at position 20 is Aib
  SITE 24: note = MISC_FEATURE - Xaa at position 24 is Aib
  MOD_RES 39: note = Ser at position 39 is amidated

SEQ ID NO: 162 - protein, 39 aa, synthetic construct
  REGION 1..39: note = Synthetic Construct
  SITE 2: note = MISC_FEATURE - Xaa at position 2 is Aib
  SITE 6: note = MISC_FEATURE - Xaa at position 6 is alpha-methyl-Phe(2F)
  SITE 13: note = MISC_FEATURE - Xaa at position 13 is alpha-methyl-Leu
  MOD_RES 17: note = Lys at position 17 is chemically modified by conjugation of the epsilon-amino group of the Lys side chain with (2-[2-(2-amino-ethoxy)-ethoxy]-acetyl)2-(gamma-Glu)-CO-(CH2)18-CO 2H
  SITE 20: note = MISC_FEATURE - Xaa at position 20 is Aib
  MOD_RES 39: note = Ser at position 39 is amidated
YXEGTXTSDYSIXLDEKAQXEFIHYLIEGGPSSGAPPPS

SEQ ID NO: 163 - protein, 39 aa, synthetic construct
  REGION 1..39: note = Synthetic Construct
  SITE 2: note = MISC_FEATURE - Xaa at position 2 is Aib
  SITE 6: note = MISC_FEATURE - Xaa at position 6 is alpha-methyl-Phe(2F)
  SITE 13: note = MISC_FEATURE - Xaa at position 13 is alpha-methyl-Leu
  MOD_RES 17: note = Lys at position 17 is chemically modified by conjugation of the epsilon-amino group of the Lys side chain with (2-[2-(2-amino-ethoxy)-ethoxy]-acetyl)2-(gamma-Glu)-CO-(CH2)18-CO 2H
  SITE 20: note = MISC_FEATURE - Xaa at position 20 is Aib
  MOD_RES 39: note = Ser at position 39 is amidated
YXEGTXTSDHSIXLDEKAQXEFIEYLIEGGPSSGAPPPS

SEQ ID NO: 164 - protein, 39 aa, synthetic construct
  REGION 1..39: note = Synthetic Construct
  SITE 2: note = MISC_FEATURE - Xaa at position 2 is Aib
  SITE 6: note = MISC_FEATURE - Xaa at position 6 is alpha-methyl-Phe(2F)
  SITE 10: note = MISC_FEATURE - Xaa at position 10 is cTA
  SITE 13: note = MISC_FEATURE - Xaa at position 13 is alpha-methyl-Leu
  MOD_RES 17: note = Lys at position 17 is chemically modified by conjugation of the epsilon-amino group of the Lys side chain with (2-[2-(2-amino-ethoxy)-ethoxy]-acetyl)2-(gamma-Glu)-CO-(CH2)18-CO 2H
  SITE 20: note = MISC_FEATURE - Xaa at position 20 is Aib
  MOD_RES 39: note = Ser at position 39 is amidated
YXEGTXTSDXSIXLDEKAQXEFIEYLIEGGPSSGAPPPS

SEQ ID NO: 165 - protein, 39 aa, synthetic construct; identical to SEQ ID NO: 164
  REGION 1..39: note = Synthetic Construct
  SITE 2: note = MISC_FEATURE - Xaa at position 2 is Aib
  SITE 6: note = MISC_FEATURE - Xaa at position 6 is alpha-methyl-Phe(2F)
  SITE 10: note = MISC_FEATURE - Xaa at position 10 is 2Pal
  SITE 13: note = MISC_FEATURE - Xaa at position 13 is alpha-methyl-Leu
  MOD_RES 17: note = Lys at position 17 is chemically modified by conjugation of the epsilon-amino group of the Lys side chain with (2-[2-(2-amino-ethoxy)-ethoxy]-acetyl)2-(gamma-Glu)-CO-(CH2)18-CO 2H
  SITE 20: note = MISC_FEATURE - Xaa at position 20 is Aib
  MOD_RES 39: note = Ser at position 39 is amidated

SEQ ID NO: 166 - protein, 39 aa, synthetic construct; identical to SEQ ID NO: 164
  REGION 1..39: note = Synthetic Construct
  SITE 2: note = MISC_FEATURE - Xaa at position 2 is Aib
  SITE 6: note = MISC_FEATURE - Xaa at position 6 is alpha-methyl-Phe(2F)
  SITE 10: note = MISC_FEATURE - Xaa at position 10 is 3Pal
  SITE 13: note = MISC_FEATURE - Xaa at position 13 is alpha-methyl-Leu
  MOD_RES 17: note = Lys at position 17 is chemically modified by conjugation of the epsilon-amino group of the Lys side chain with (2-[2-(2-amino-ethoxy)-ethoxy]-acetyl)2-(gamma-Glu)-CO-(CH2)18-CO 2H
  SITE 20: note = MISC_FEATURE - Xaa at position 20 is Aib
  MOD_RES 39: note = Ser at position 39 is amidated

SEQ ID NO: 167 - protein, 39 aa, synthetic construct; identical to SEQ ID NO: 164
  REGION 1..39: note = Synthetic Construct
  SITE 2: note = MISC_FEATURE - Xaa at position 2 is Aib
  SITE 6: note = MISC_FEATURE - Xaa at position 6 is alpha-methyl-Phe(2F)
  SITE 10: note = MISC_FEATURE - Xaa at position 10 is 4Pal
  SITE 13: note = MISC_FEATURE - Xaa at position 13 is alpha-methyl-Leu
  MOD_RES 17: note = Lys at position 17 is chemically modified by conjugation of the epsilon-amino group of the Lys side chain with (2-[2-(2-amino-ethoxy)-ethoxy]-acetyl)2-(gamma-Glu)-CO-(CH2)18-CO 2H
  SITE 20: note = MISC_FEATURE - Xaa at position 20 is Aib
  MOD_RES 39: note = Ser at position 39 is amidated

SEQ ID NO: 168 - protein, 39 aa, synthetic construct; identical to SEQ ID NO: 164
  REGION 1..39: note = Synthetic Construct
  SITE 2: note = MISC_FEATURE - Xaa at position 2 is Aib
  SITE 6: note = MISC_FEATURE - Xaa at position 6 is alpha-methyl-Phe(2F)
  SITE 10: note = MISC_FEATURE - Xaa at position 10 is alpha-methyl-Phe
  SITE 13: note = MISC_FEATURE - Xaa at position 13 is alpha-methyl-Leu
  MOD_RES 17: note = Lys at position 17 is chemically modified by conjugation of the epsilon-amino group of the Lys side chain with (2-[2-(2-amino-ethoxy)-ethoxy]-acetyl)2-(gamma-Glu)-CO-(CH2)18-CO 2H
  SITE 20: note = MISC_FEATURE - Xaa at position 20 is Aib
  MOD_RES 39: note = Ser at position 39 is amidated

SEQ ID NO: 169 - protein, 39 aa, synthetic construct
  REGION 1..39: note = Synthetic Construct
  SITE 2: note = MISC_FEATURE - Xaa at position 2 is Aib
  SITE 6: note = MISC_FEATURE - Xaa at position 6 is alpha-methyl-Phe(2F)
  SITE 10: note = MISC_FEATURE - Xaa at position 10 is Aib
  SITE 13: note = MISC_FEATURE - Xaa at position 13 is alpha-methyl-Leu
  MOD_RES 17: note = Lys at position 17 is chemically modified by conjugation of the epsilon-amino group of the Lys side chain with (2-[2-(2-amino-ethoxy)-ethoxy]-acetyl)2-(gamma-Glu)-CO-(CH2)18-CO 2H
  SITE 20: note = MISC_FEATURE - Xaa at position 20 is Aib
  SITE 24: note = MISC_FEATURE - Xaa at position 24 is D-Glu
  MOD_RES 39: note = Ser at position 39 is amidated
YXEGTXTSDXSIXLDEKAQXTFIXYLIEGGPSSGAPPPS

SEQ ID NO: 170 - protein, 34 aa, synthetic construct
  REGION 1..34: note = Synthetic Construct
  SITE 2: note = MISC_FEATURE - Xaa at position 2 is Aib
  SITE 6: note = MISC_FEATURE - Xaa at position 6 is alpha-methyl-Phe(2F)
  SITE 13: note = MISC_FEATURE - Xaa at position 13 is alpha-methyl-Leu
  MOD_RES 17: note = Lys at position 17 is chemically modified by conjugation of the epsilon-amino group of the Lys side chain with (2-[2-(2-amino-ethoxy)-ethoxy]-acetyl)2-(gamma-Glu)2-CO-(CH2)18-C O2H
  SITE 20: note = MISC_FEATURE - Xaa at position 20 is Aib
  SITE 24: note = MISC_FEATURE - Xaa at position 24 is D-Glu
  MOD_RES 34: note = Gly at position 34 is amidated
YXEGTXTSDHSIXLDEKAQXTFIXYLIEGGPSSG

SEQ ID NO: 171 - protein, 34 aa, synthetic construct
  REGION 1..34: note = Synthetic Construct
  SITE 2: note = MISC_FEATURE - Xaa at position 2 is Aib
  SITE 6: note = MISC_FEATURE - Xaa at position 6 is alpha-methyl-Phe(2F)
  SITE 13: note = MISC_FEATURE - Xaa at position 13 is alpha-methyl-Leu
  MOD_RES 17: note = Lys at position 17 is chemically modified by conjugation of the epsilon-amino group of the Lys side chain with (2-[2-(2-amino-ethoxy)-ethoxy]-acetyl)2-(gamma-Glu)2-CO-(CH2)18-C O2H
  SITE 20: note = MISC_FEATURE - Xaa at position 20 is Aib
  SITE 24: note = MISC_FEATURE - Xaa at position 24 is D-Glu
  MOD_RES 34: note = Gly at position 34 is amidated
YXEGTXTSDHSIXLDEKAQXTFIXHLIEGGPSSG

SEQ ID NO: 172 - protein, 39 aa, synthetic construct
  REGION 1..39: note = Synthetic Construct
  SITE 2: note = MISC_FEATURE - Xaa at position 2 is Aib
  SITE 6: note = MISC_FEATURE - Xaa at position 6 is alpha-methyl-Phe(2F)
  SITE 13: note = MISC_FEATURE - Xaa at position 13 is alpha-methyl-Leu
  MOD_RES 17: note = Lys at position 17 is chemically modified by conjugation of the epsilon-amino group of the Lys side chain with (2-[2-(2-amino-ethoxy)-ethoxy]-acetyl)2-(gamma-Glu)-CO-(CH2)18-CO 2H
  SITE 20: note = MISC_FEATURE - Xaa at position 20 is Aib
  MOD_RES 39: note = Ser at position 39 is amidated
HXEGTXTSDYSIXLDEKAQXEFIEYLIEGGPSSGAPPPS

SEQ ID NO: 173 - protein, 39 aa, synthetic construct
  REGION 1..39: note = Synthetic Construct
  SITE 2: note = MISC_FEATURE - Xaa at position 2 is Aib
  SITE 6: note = MISC_FEATURE - Xaa at position 6 is alpha-methyl-Phe(2F)
  SITE 13: note = MISC_FEATURE - Xaa at position 13 is alpha-methyl-Leu
  MOD_RES 17: note = Lys at position 17 is chemically modified by conjugation of the epsilon-amino group of the Lys side chain with (2-[2-(2-amino-ethoxy)-ethoxy]-acetyl)2-(gamma-Glu)-CO-(CH2)18-CO 2H
  SITE 20: note = MISC_FEATURE - Xaa at position 20 is Aib
  SITE 24: note = MISC_FEATURE - Xaa at position 24 is D-Glu
  SITE 28: note = MISC_FEATURE - Xaa at position 28 is D-Glu
  MOD_RES 39: note = Ser at position 39 is amidated
YXEGTXTSDHSIXLDEKAQXTFIXYLIXGGPSSGAPPPS

SEQ ID NO: 174 - protein, 39 aa, synthetic construct
  REGION 1..39: note = Synthetic Construct
  SITE 2: note = MISC_FEATURE - Xaa at position 2 is Aib
  SITE 6: note = MISC_FEATURE - Xaa at position 6 is alpha-methyl-Phe(2F)
  SITE 13: note = MISC_FEATURE - Xaa at position 13 is alpha-methyl-Leu
  MOD_RES 17: note = Lys at position 17 is chemically modified by conjugation of the epsilon-amino group of the Lys side chain with (2-[2-(2-amino-ethoxy)-ethoxy]-acetyl)2-(gamma-Glu)-CO-(CH2)18-CO 2H
  SITE 20: note = MISC_FEATURE - Xaa at position 20 is Aib
  SITE 24: note = MISC_FEATURE - Xaa at position 24 is D-Glu
  SITE 25: note = MISC_FEATURE - Xaa at position 25 is alpha-methyl-Phe
  SITE 28: note = MISC_FEATURE - Xaa at position 28 is D-Glu
  MOD_RES 39: note = Ser at position 39 is amidated
YXEGTXTSDHSIXLDEKAQXTFIXXLIXGGPSSGAPPPS

SEQ ID NO: 175 - protein, 30 aa, synthetic construct
  REGION 1..30: note = Synthetic Construct
  SITE 2: note = MISC_FEATURE - Xaa at position 2 is Aib
  SITE 6: note = MISC_FEATURE - Xaa at position 6 is alpha-methyl-Phe(2F)
  SITE 13: note = MISC_FEATURE - Xaa at position 13 is alpha-methyl-Leu
  MOD_RES 17: note = Lys at position 17 is chemically modified by conjugation of the epsilon-amino group of the Lys side chain with (2-[2-(2-amino-ethoxy)-ethoxy]-acetyl)2-(gamma-Glu)-CO-(CH2)18-CO 2H
  SITE 20: note = MISC_FEATURE - Xaa at position 20 is Aib
  SITE 24: note = MISC_FEATURE - Xaa at position 24 is D-Glu
  MOD_RES 30: note = Gly at position 30 is amidated
YXEGTXTSDHSIXLDEKAQXTFIXYLIEGG

SEQ ID NO: 176 - protein, 34 aa, synthetic construct; identical to SEQ ID NO: 170
  REGION 1..34: note = Synthetic Construct
  SITE 2: note = MISC_FEATURE - Xaa at position 2 is Aib
  SITE 6: note = MISC_FEATURE - Xaa at position 6 is alpha-methyl-Phe(2F)
  SITE 13: note = MISC_FEATURE - Xaa at position 13 is alpha-methyl-Leu
  MOD_RES 17: note = Lys at position 17 is chemically modified by conjugation of the epsilon-amino group of the Lys side chain with (2-[2-(2-amino-ethoxy)-ethoxy]-acetyl)2-(gamma-Glu)-CO-(CH2)18-CO 2H
  SITE 20: note = MISC_FEATURE - Xaa at position 20 is Aib
  SITE 24: note = MISC_FEATURE - Xaa at position 24 is D-Glu
  MOD_RES 34: note = Gly at position 34 is amidated

SEQ ID NO: 177 - protein, 39 aa, synthetic construct
  REGION 1..39: note = Synthetic Construct
  SITE 2: note = MISC_FEATURE - Xaa at position 2 is Aib
  SITE 6: note = MISC_FEATURE - Xaa at position 6 is alpha-methyl-Phe(2F)
  SITE 13: note = MISC_FEATURE - Xaa at position 13 is alpha-methyl-Leu
  MOD_RES 17: note = Lys at position 17 is chemically modified by conjugation of the epsilon-amino group of the Lys side chain with (2-[2-(2-amino-ethoxy)-ethoxy]-acetyl)2-(gamma-Glu)-CO-(CH2)18-CO 2H
  SITE 20: note = MISC_FEATURE - Xaa at position 20 is Aib
  SITE 24: note = MISC_FEATURE - Xaa at position 24 is D-Glu
  MOD_RES 39: note = Ser at position 39 is amidated
YXEGTXTSDHSIXLDEKAQXTFIXYLIEGGPSSGAPPPS

SEQ ID NO: 178 - protein, 39 aa, synthetic construct; identical to SEQ ID NO: 177
  REGION 1..39: note = Synthetic Construct
  SITE 2: note = MISC_FEATURE - Xaa at position 2 is Aib
  SITE 6: note = MISC_FEATURE - Xaa at position 6 is alpha-methyl-Phe(2F)
  SITE 13: note = MISC_FEATURE - Xaa at position 13 is alpha-methyl-Leu
  MOD_RES 17: note = Lys at position 17 is chemically modified by conjugation of the epsilon-amino group of the Lys side chain with (2-[2-(2-amino-ethoxy)-ethoxy]-acetyl)2-(gamma-Glu)-CO-(CH2)16-CO 2H
  SITE 20: note = MISC_FEATURE - Xaa at position 20 is Aib
  SITE 24: note = MISC_FEATURE - Xaa at position 24 is D-Glu
  MOD_RES 39: note = Ser at position 39 is amidated

SEQ ID NO: 179 - protein, 39 aa, synthetic construct; identical to SEQ ID NO: 177
  REGION 1..39: note = Synthetic Construct
  SITE 2: note = MISC_FEATURE - Xaa at position 2 is Aib
  SITE 6: note = MISC_FEATURE - Xaa at position 6 is alpha-methyl-Phe(2F)
  SITE 13: note = MISC_FEATURE - Xaa at position 13 is alpha-methyl-Leu
  MOD_RES 17: note = Lys at position 17 is chemically modified by conjugation of the epsilon-amino group of the Lys side chain with (2-[2-(2-amino-ethoxy)-ethoxy]-acetyl)2-(gamma-Glu)-CO-(CH2)14-CO 2H
  SITE 20: note = MISC_FEATURE - Xaa at position 20 is Aib
  SITE 24: note = MISC_FEATURE - Xaa at position 24 is D-Glu
  MOD_RES 39: note = Ser at position 39 is amidated

SEQ ID NO: 180 - protein, 39 aa, synthetic construct
  REGION 1..39: note = Synthetic Construct
  SITE 2: note = MISC_FEATURE - Xaa at position 2 is Aib
  SITE 6: note = MISC_FEATURE - Xaa at position 6 is alpha-methyl-Phe(2F)
  SITE 13: note = MISC_FEATURE - Xaa at position 13 is alpha-methyl-Leu
  SITE 16: note = MISC_FEATURE - Xaa at position 16 is Orn
  MOD_RES 17: note = Lys at position 17 is chemically modified by conjugation of the epsilon-amino group of the Lys side chain with (2-[2-(2-amino-ethoxy)-ethoxy]-acetyl)2-(gamma-Glu)-CO-(CH2)18-CO 2H
  SITE 20: note = MISC_FEATURE - Xaa at position 20 is Aib
  SITE 24: note = MISC_FEATURE - Xaa at position 24 is D-Glu
  MOD_RES 39: note = Ser at position 39 is amidated
YXEGTXTSDHSIXLDXKAQXTFIXYLIEGGPSSGAPPPS

SEQ ID NO: 181 - protein, 39 aa, synthetic construct; identical to SEQ ID NO: 180
  REGION 1..39: note = Synthetic Construct
  SITE 2: note = MISC_FEATURE - Xaa at position 2 is Aib
  SITE 6: note = MISC_FEATURE - Xaa at position 6 is alpha-methyl-Phe(2F)
  SITE 13: note = MISC_FEATURE - Xaa at position 13 is alpha-methyl-Leu
  SITE 16: note = MISC_FEATURE - Xaa at position 16 is Dab
  MOD_RES 17: note = Lys at position 17 is chemically modified by conjugation of the epsilon-amino group of the Lys side chain with (2-[2-(2-amino-ethoxy)-ethoxy]-acetyl)2-(gamma-Glu)-CO-(CH2)18-CO 2H
  SITE 20: note = MISC_FEATURE - Xaa at position 20 is a Aib
  SITE 24: note = MISC_FEATURE - Xaa at position 24 is D-Glu
  MOD_RES 39: note = Ser at position 39 is amidated

SEQ ID NO: 182 - protein, 39 aa, synthetic construct; identical to SEQ ID NO: 180
  REGION 1..39: note = Synthetic Construct
  SITE 2: note = MISC_FEATURE - Xaa at position 2 is Aib
  SITE 6: note = MISC_FEATURE - Xaa at position 6 is alpha-methyl-Phe(2F)
  SITE 13: note = MISC_FEATURE - Xaa at position 13 is alpha-methyl-Leu
  SITE 16: note = MISC_FEATURE - Xaa at position 16 is Dap
  MOD_RES 17: note = Lys at position 17 is chemically modified by conjugation of the epsilon-amino group of the Lys side chain with (2-[2-(2-amino-ethoxy)-ethoxy]-acetyl)2-(gamma-Glu)-CO-(CH2)18-CO 2H
  SITE 20: note = MISC_FEATURE - Xaa at position 20 is Aib
  SITE 24: note = MISC_FEATURE - Xaa at position 24 is D-Glu
  MOD_RES 39: note = Ser at position 39 is amidated

SEQ ID NO: 183 - protein, 39 aa, synthetic construct; identical to SEQ ID NO: 177
  REGION 1..39: note = Synthetic Construct
  SITE 2: note = MISC_FEATURE - Xaa at position 2 is Aib
  SITE 6: note = MISC_FEATURE - Xaa at position 6 is alpha-methyl-Phe(2F)
  SITE 13: note = MISC_FEATURE - Xaa at position 13 is alpha-methyl-Leu
  MOD_RES 17: note = Lys at position 17 is chemically modified by conjugation of the epsilon-amino group of the Lys side chain with (2-[2-(2-amino-ethoxy)-ethoxy]-acetyl)2-CO-(CH2)18-CO2H
  SITE 20: note = MISC_FEATURE - Xaa at position 20 is Aib
  SITE 24: note = MISC_FEATURE - Xaa at position 24 is D-Glu
  MOD_RES 39: note = Ser at position 39 is amidated

SEQ ID NO: 184 - protein, 39 aa, synthetic construct; identical to SEQ ID NO: 177
  REGION 1..39: note = Synthetic Construct
  SITE 2: note = MISC_FEATURE - Xaa at position 2 is Aib
  SITE 6: note = MISC_FEATURE - Xaa at position 6 is alpha-methyl-Phe(2F)
  SITE 13: note = MISC_FEATURE - Xaa at position 13 is alpha-methyl-Leu
  MOD_RES 17: note = Lys at position 17 is chemically modified by conjugation of the epsilon-amino group of the Lys side chain with (2-[2-(2-amino-ethoxy)-ethoxy]-acetyl)2-(epsilon-Lys)-CO-(CH2)18- CO2H
  SITE 20: note = MISC_FEATURE - Xaa at position 20 is Aib
  SITE 24: note = MISC_FEATURE - Xaa at position 24 is D-Glu
  MOD_RES 39: note = Ser at position 39 is amidated

SEQ ID NO: 185 - protein, 39 aa, synthetic construct; identical to SEQ ID NO: 177
  REGION 1..39: note = Synthetic Construct
  SITE 2: note = MISC_FEATURE - Xaa at position 2 is Aib
  SITE 6: note = MISC_FEATURE - Xaa at position 6 is alpha-methyl-Phe(2F)
  SITE 13: note = MISC_FEATURE - Xaa at position 13 is alpha-methyl-Leu
  MOD_RES 17: note = Lys at position 17 is chemically modified by conjugation of the epsilon-amino group of the Lys side chain with (2-[2-(2-amino-ethoxy)-ethoxy]-acetyl)2-(epsilon-Lys)-CO-(CH2)16- CO2H
  SITE 20: note = MISC_FEATURE - Xaa at position 20 is Aib
  SITE 24: note = MISC_FEATURE - Xaa at position 24 is D-Glu
  MOD_RES 39: note = Ser at position 39 is amidated

SEQ ID NO: 186 - protein, 39 aa, synthetic construct
  REGION 1..39: note = Synthetic Construct
  SITE 2: note = MISC_FEATURE - Xaa at position 2 is Aib
  SITE 6: note = MISC_FEATURE - Xaa at position 6 is alpha-methyl-Phe(2F)
  SITE 13: note = MISC_FEATURE - Xaa at position 13 is alpha-methyl-Leu
  MOD_RES 17: note = Lys at position 17 is chemically modified by conjugation of the epsilon-amino group of the Lys side chain with (2-[2-(2-amino-ethoxy)-ethoxy]-acetyl)2-(gamma-Glu)-CO-(CH2)16-CO 2H
  SITE 20: note = MISC_FEATURE - Xaa at position 20 is Aib
  SITE 24: note = MISC_FEATURE - Xaa at position 24 is D-Glu
  MOD_RES 39: note = Ser at position 39 is amidated
YXEGTXTSDHSIXLDEKAQXHFIXYLIEGGPSSGAPPPS

SEQ ID NO: 187 - protein, 39 aa, synthetic construct; identical to SEQ ID NO: 186
  REGION 1..39: note = Synthetic Construct
  SITE 2: note = MISC_FEATURE - Xaa at position 2 is Aib
  SITE 6: note = MISC_FEATURE - Xaa at position 6 is alpha-methyl-Phe(2F)
  SITE 13: note = MISC_FEATURE - Xaa at position 13 is alpha-methyl-Leu
  MOD_RES 17: note = Lys at position 17 is chemically modified by conjugation of the epsilon-amino group of the Lys side chain with (2-[2-(2-amino-ethoxy)-ethoxy]-acetyl)2-(gamma-Glu)-CO-(CH2)14-CO 2H
  SITE 20: note = MISC_FEATURE - Xaa at position 20 is Aib
  SITE 24: note = MISC_FEATURE - Xaa at position 24 is D-Glu
  MOD_RES 39: note = Ser at position 39 is amidated

SEQ ID NO: 188 - protein, 34 aa, synthetic construct
  REGION 1..34: note = Synthetic Construct
  SITE 2: note = MISC_FEATURE - Xaa at position 2 is Aib
  SITE 6: note = MISC_FEATURE - Xaa at position 6 is alpha-methyl-Phe(2F)
  SITE 13: note = MISC_FEATURE - Xaa at position 13 is alpha-methyl-Leu
  MOD_RES 17: note = Lys at position 17 is chemically modified by conjugation of the epsilon-amino group of the Lys side chain with (2-[2-(2-amino-ethoxy)-ethoxy]-acetyl)2-(gamma-Glu)-CO-(CH2)16-CO 2H
  SITE 20: note = MISC_FEATURE - Xaa at position 20 is Aib
  SITE 24: note = MISC_FEATURE - Xaa at position 24 is D-Glu
  MOD_RES 34: note = Gly at position 34 is amidated
YXEGTXTSDHSIXLDEKAQXHFIXYLIEGGPSSG

SEQ ID NO: 189 - protein, 30 aa, synthetic construct
  REGION 1..30: note = Synthetic Construct
  SITE 2: note = MISC_FEATURE - Xaa at position 2 is Aib
  SITE 6: note = MISC_FEATURE - Xaa at position 6 is alpha-methyl-Phe(2F)
  SITE 13: note = MISC_FEATURE - Xaa at position 13 is alpha-methyl-Leu
  MOD_RES 17: note = Lys at position 17 is chemically modified by conjugation of the epsilon-amino group of the Lys side chain with (2-[2-(2-amino-ethoxy)-ethoxy]-acetyl)2-(gamma-Glu)-CO-(CH2)16-CO 2H
  SITE 20: note = MISC_FEATURE - Xaa at position 20 is Aib
  SITE 24: note = MISC_FEATURE - Xaa at position 24 is D-Glu
  MOD_RES 30: note = Gly at position 30 is amidated
YXEGTXTSDHSIXLDEKAQXHFIXYLIEGG

SEQ ID NO: 190 - protein, 39 aa, synthetic construct
  REGION 1..39: note = Synthetic Construct
  SITE 2: note = MISC_FEATURE - Xaa at position 2 is Aib
  SITE 6: note = MISC_FEATURE - Xaa at position 6 is alpha-methyl-Phe(2F)
  SITE 10: note = MISC_FEATURE - Xaa at position 10 is 3Pal
  SITE 13: note = MISC_FEATURE - Xaa at position 13 is alpha-methyl-Leu
  MOD_RES 17: note = Lys at position 17 is chemically modified by conjugation of the epsilon-amino group of the Lys side chain with (2-[2-(2-amino-ethoxy)-ethoxy]-acetyl)2-(gamma-Glu)-CO-(CH2)18-CO 2H
  SITE 20: note = MISC_FEATURE - Xaa at position 20 is Aib
  SITE 24: note = MISC_FEATURE - Xaa at position 24 is D-Glu
  MOD_RES 39: note = Ser at position 39 is amidated
YXEGTXTSDXSIXLDEKAQXEFIXYLIEGGPSSGAPPPS

SEQ ID NO: 191 - protein, 39 aa, synthetic construct; identical to SEQ ID NO: 190
  REGION 1..39: note = Synthetic Construct
  SITE 2: note = MISC_FEATURE - Xaa at position 2 is Aib
  SITE 6: note = MISC_FEATURE - Xaa at position 6 is alpha-methyl-Phe(2F)
  SITE 10: note = MISC_FEATURE - Xaa at position 10 is 4Pal
  SITE 13: note = MISC_FEATURE - Xaa at position 13 is alpha-methyl-Leu
  MOD_RES 17: note = Lys at position 17 is chemically modified by conjugation of the epsilon-amino group of the Lys side chain with (2-[2-(2-amino-ethoxy)-ethoxy]-acetyl)2-(gamma-Glu)-CO-(CH2)18-CO 2H
  SITE 20: note = MISC_FEATURE - Xaa at position 20 is Aib
  SITE 24: note = MISC_FEATURE - Xaa at position 24 is D-Glu
  MOD_RES 39: note = Ser at position 39 is amidated

SEQ ID NO: 192 - protein, 39 aa, synthetic construct
  REGION 1..39: note = Synthetic Construct
  SITE 2: note = MISC_FEATURE - Xaa at position 2 is Aib
  SITE 6: note = MISC_FEATURE - Xaa at position 6 is alpha-methyl-Phe(2F)
  SITE 13: note = MISC_FEATURE - Xaa at position 13 is alpha-methyl-Leu
  MOD_RES 17: note = Lys at position 17 is chemically modified by conjugation of the epsilon-amino group of the Lys side chain with (2-[2-(2-amino-ethoxy)-ethoxy]-acetyl)2-(gamma-Glu)-CO-(CH2)18-CO 2H
  SITE 20: note = MISC_FEATURE - Xaa at position 20 is Aib
  SITE 24: note = MISC_FEATURE - Xaa at position 24 is D-Glu
  MOD_RES 39: note = Ser at position 39 is amidated
YXEGTXTSDLSIXLDEKAQXEFIXYLIEGGPSSGAPPPS

SEQ ID NO: 193 - protein, 39 aa, synthetic construct; identical to SEQ ID NO: 190
  REGION 1..39: note = Synthetic Construct
  SITE 2: note = MISC_FEATURE - Xaa at position 2 is Aib
  SITE 6: note = MISC_FEATURE - Xaa at position 6 is alpha-methyl-Phe(2F)
  SITE 10: note = MISC_FEATURE - Xaa at position 10 is D-Tyr
  SITE 13: note = MISC_FEATURE - Xaa at position 13 is alpha-methyl-Leu
  MOD_RES 17: note = Lys at position 17 is chemically modified by conjugation of the epsilon-amino group of the Lys side chain with (2-[2-(2-amino-ethoxy)-ethoxy]-acetyl)2-(gamma-Glu)-CO-(CH2)18-CO 2H
  SITE 20: note = MISC_FEATURE - Xaa at position 20 is Aib
  SITE 24: note = MISC_FEATURE - Xaa at position 24 is D-Glu
  MOD_RES 39: note = Ser at position 39 is amidated

SEQ ID NO: 194 - protein, 39 aa, synthetic construct; identical to SEQ ID NO: 190
  REGION 1..39: note = Synthetic Construct
  SITE 2: note = MISC_FEATURE - Xaa at position 2 is Aib
  SITE 6: note = MISC_FEATURE - Xaa at position 6 is alpha-methyl-Phe(2F)
  SITE 10: note = MISC_FEATURE - Xaa at position 10 is D-His
  SITE 13: note = MISC_FEATURE - Xaa at position 13 is alpha-methyl-Leu
  MOD_RES 17: note = Lys at position 17 is chemically modified by conjugation of the epsilon-amino group of the Lys side chain with (2-[2-(2-amino-ethoxy)-ethoxy]-acetyl)2-(gamma-Glu)-CO-(CH2)18-CO 2H
  SITE 20: note = MISC_FEATURE - Xaa at position 20 is Aib
  SITE 24: note = MISC_FEATURE - Xaa at position 24 is D-Glu
  MOD_RES 39: note = Ser at position 39 is amidated

SEQ ID NO: 195 - protein, 39 aa, synthetic construct; identical to SEQ ID NO: 190
  REGION 1..39: note = Synthetic Construct
  SITE 2: note = MISC_FEATURE - Xaa at position 2 is Aib
  SITE 6: note = MISC_FEATURE - Xaa at position 6 is alpha-methyl-Phe(2F)
  SITE 10: note = MISC_FEATURE - Xaa at position 10 is alpha-methyl-Tyr
  SITE 13: note = MISC_FEATURE - Xaa at position 13 is alpha-methyl-Leu
  MOD_RES 17: note = Lys at position 17 is chemically modified by conjugation of the epsilon-amino group of the Lys side chain with (2-[2-(2-amino-ethoxy)-ethoxy]-acetyl)2-(gamma-Glu)-CO-(CH2)18-CO 2H
  SITE 20: note = MISC_FEATURE - Xaa at position 20 is Aib
  SITE 24: note = MISC_FEATURE - Xaa at position 24 is D-Glu
  MOD_RES 39: note = Ser at position 39 is amidated

SEQ ID NO: 196 - protein, 39 aa, synthetic construct
  REGION 1..39: note = Synthetic Construct
  SITE 2: note = MISC_FEATURE - Xaa at position 2 is Aib
  SITE 6: note = MISC_FEATURE - Xaa at position 6 is alpha-methyl-Phe(2F)
  SITE 13: note = MISC_FEATURE - Xaa at position 13 is alpha-methyl-Leu
  MOD_RES 17: note = Lys at position 17 is chemically modified by conjugation of the epsilon-amino group of the Lys side chain with (2-[2-(2-amino-ethoxy)-ethoxy]-acetyl)2-(gamma-Glu)-CO-(CH2)18-CO 2H
  SITE 20: note = MISC_FEATURE - Xaa at position 20 is Aib
  SITE 24: note = MISC_FEATURE - Xaa at position 24 is D-Glu
  MOD_RES 39: note = Ser at position 39 is amidated
YXEGTXTSDQSIXLDEKAQXEFIXYLIEGGPSSGAPPPS

SEQ ID NO: 197 - protein, 39 aa, synthetic construct; identical to SEQ ID NO: 190
  REGION 1..39: note = Synthetic Construct
  SITE 2: note = MISC_FEATURE - Xaa at position 2 is Aib
  SITE 6: note = MISC_FEATURE - Xaa at position 6 is alpha-methyl-Phe(2F)
  SITE 10: note = MISC_FEATURE - Xaa at position 10 is 3Pal
  SITE 13: note = MISC_FEATURE - Xaa at position 13 is alpha-methyl-Leu
  MOD_RES 17: note = Lys at position 17 is chemically modified by conjugation of the epsilon-amino group of the Lys side chain with (2-[2-(2-amino-ethoxy)-ethoxy]-acetyl)2-(gamma-Glu)-CO-(CH2)18-CO 2H
  SITE 20: note = MISC_FEATURE - Xaa at position 20 is Aib
  SITE 24: note = MISC_FEATURE - Xaa at position 24 is Aib
  MOD_RES 39: note = Ser at position 39 is amidated

SEQ ID NO: 198 - protein, 39 aa, synthetic construct; identical to SEQ ID NO: 190
  REGION 1..39: note = Synthetic Construct
  SITE 2: note = MISC_FEATURE - Xaa at position 2 is Aib
  SITE 6: note = MISC_FEATURE - Xaa at position 6 is alpha-methyl-Phe(2F)
  SITE 10: note = MISC_FEATURE - Xaa at position 10 is 4Pal
  SITE 13: note = MISC_FEATURE - Xaa at position 13 is alpha-methyl-Leu
  MOD_RES 17: note = Lys at position 17 is chemically modified by conjugation of the epsilon-amino group of the Lys side chain with (2-[2-(2-amino-ethoxy)-ethoxy]-acetyl)2-(gamma-Glu)-CO-(CH2)18-CO 2H
  SITE 20: note = MISC_FEATURE - Xaa at position 20 is Aib
  SITE 24: note = MISC_FEATURE - Xaa at position 24 is Aib
  MOD_RES 39: note = Ser at position 39 is amidated

SEQ ID NO: 199 - protein, 39 aa, synthetic construct
  REGION 1..39: note = Synthetic Construct
  SITE 2: note = MISC_FEATURE - Xaa at position 2 is Aib
  SITE 6: note = MISC_FEATURE - Xaa at position 6 is alpha-methyl-Phe(2F)
  SITE 10: note = MISC_FEATURE - Xaa at position 10 is 3Pal
  SITE 13: note = MISC_FEATURE - Xaa at position 13 is alpha-methyl-Leu
  MOD_RES 17: note = Lys at position 17 is chemically modified by conjugation of the epsilon-amino group of the Lys side chain with (2-[2-(2-amino-ethoxy)-ethoxy]-acetyl)2-(gamma-Glu)-CO-(CH2)18-CO 2H
  SITE 20: note = MISC_FEATURE - Xaa at position 20 is Aib
  SITE 24: note = MISC_FEATURE - Xaa at position 24 is D-Glu
  MOD_RES 39: note = Ser at position 39 is amidated
HXEGTXTSDXSIXLDEKAQXEFIXYLIEGGPSSGAPPPS

SEQ ID NO: 200 - protein, 39 aa, synthetic construct
  REGION 1..39: note = Synthetic Construct
  SITE 2: note = MISC_FEATURE - Xaa at position 2 is Aib
  SITE 6: note = MISC_FEATURE - Xaa at position 6 is alpha-methyl-Phe(2F)
  SITE 13: note = MISC_FEATURE - Xaa at position 13 is alpha-methyl-Leu
  MOD_RES 17: note = Lys at position 17 is chemically modified by conjugation of the epsilon-amino group of the Lys side chain with (2-[2-(2-amino-ethoxy)-ethoxy]-acetyl)2-(gamma-Glu)-CO-(CH2)18-CO 2H
  SITE 20: note = MISC_FEATURE - Xaa at position 20 is Aib
  SITE 24: note = MISC_FEATURE - Xaa at position 24 is D-Glu
  MOD_RES 39: note = Ser at position 39 is amidated
YXEGTXTSDVSIXLDEKAQXEFIXYLIEGGPSSGAPPPS

SEQ ID NO: 201 - protein, 39 aa, synthetic construct
  REGION 1..39: note = Synthetic Construct
  SITE 2: note = MISC_FEATURE - Xaa at position 2 is Aib
  SITE 6: note = MISC_FEATURE - Xaa at position 6 is alpha-methyl-Phe(2F)
  SITE 13: note = MISC_FEATURE - Xaa at position 13 is alpha-methyl-Leu
  MOD_RES 17: note = Lys at position 17 is chemically modified by conjugation of the epsilon-amino group of the Lys side chain with (2-[2-(2-amino-ethoxy)-ethoxy]-acetyl)2-(gamma-Glu)-CO-(CH2)18-CO 2H
  SITE 20: note = MISC_FEATURE - Xaa at position 20 is Aib
  SITE 24: note = MISC_FEATURE - Xaa at position 24 is D-Glu
  MOD_RES 39: note = Ser at position 39 is amidated
YXEGTXTSDASIXLDEKAQXEFIXYLIEGGPSSGAPPPS

SEQ ID NO: 202 - protein, 39 aa, synthetic construct
  REGION 1..39: note = Synthetic Construct
  SITE 2: note = MISC_FEATURE - Xaa at position 2 is alpha-methyl-Pro
  MOD_RES 17: note = Lys at position 17 is chemically modified by conjugation of the epsilon-amino group of the Lys side chain with (2-[2-(2-amino-ethoxy)-ethoxy]-acetyl)2-(gamma-Glu)-CO-(CH2)18-CO 2H
  MOD_RES 39: note = Ser at position 39 is amidated
YXEGTFTSDYSILLDEKAQQAFIEYLIEGGPSSGAPPPS

SEQ ID NO: 203 - protein, 39 aa, synthetic construct
  REGION 1..39: note = Synthetic Construct
  SITE 2: note = MISC_FEATURE - Xaa at position 2 is alpha-methyl-Pro
  MOD_RES 17: note = Lys at position 17 is chemically modified by conjugation of the epsilon-amino group of the Lys side chain with (2-[2-(2-amino-ethoxy)-ethoxy]-acetyl)2-(gamma-Glu)-CO-(CH2)18-CO 2H
  MOD_RES 39: note = Ser at position 39 is amidated
YXEGTFTSDYSILLDEKAQHAFIEYLIEGGPSSGAPPPS

SEQ ID NO: 204 - protein, 39 aa, synthetic construct
  REGION 1..39: note = Synthetic Construct
  SITE 2: note = MISC_FEATURE - Xaa at position 2 is alpha-methyl-Pro
  MOD_RES 17: note = Lys at position 17 is chemically modified by conjugation of the epsilon-amino group of the Lys side chain with (2-[2-(2-amino-ethoxy)-ethoxy]-acetyl)2-(gamma-Glu)-CO-(CH2)18-CO 2H
  MOD_RES 39: note = Ser at position 39 is amidated
YXEGTFTSDYSILLDRKAQQAFIEYLIEGGPSSGAPPPS

SEQ ID NO: 205 - protein, 39 aa, synthetic construct
  REGION 1..39: note = Synthetic Construct
  SITE 2: note = MISC_FEATURE - Xaa at position 2 is alpha-methyl-Pro
  MOD_RES 17: note = Lys at position 17 is chemically modified by conjugation of the epsilon-amino group of the Lys side chain with (2-[2-(2-amino-ethoxy)-ethoxy]-acetyl)2-(gamma-Glu)-CO-(CH2)18-CO 2H
  MOD_RES 39: note = Ser at position 39 is amidated
YXEGTFTSDYSILLDRKAQHAFIEYLIEGGPSSGAPPPS

SEQ ID NO: 206 - protein, 34 aa, synthetic construct
  REGION 1..34: note = Synthetic Construct
  SITE 2: note = MISC_FEATURE - Xaa at position 2 is alpha-methyl-Pro
  MOD_RES 17: note = Lys at position 17 is chemically modified by conjugation of the epsilon-amino group of the Lys side chain with (2-[2-(2-amino-ethoxy)-ethoxy]-acetyl)2-(gamma-Glu)-CO-(CH2)16-CO 2H
  MOD_RES 34: note = Gly at position 34 is amidated
YXEGTFTSDYSILLDEKAQQAFIEYLIEGGPSSG

SEQ ID NO: 207 - protein, 34 aa, synthetic construct
  REGION 1..34: note = Synthetic Construct
  SITE 1: note = MISC_FEATURE - Xaa at position 1 is D-Tyr
  SITE 2: note = MISC_FEATURE - Xaa at position 2 is alpha-methyl-Pro
  MOD_RES 17: note = Lys at position 17 is chemically modified by conjugation of the epsilon-amino group of the Lys side chain with (2-[2-(2-amino-ethoxy)-ethoxy]-acetyl)2-(gamma-Glu)-CO-(CH2)16-CO 2H
  MOD_RES 34: note = Gly at position 34 is amidated
XXEGTFTSDYSILLDEKAQQAFIEYLIEGGPSSG

SEQ ID NO: 208 - protein, 39 aa, synthetic construct
  REGION 1..39: note = Synthetic Construct
  SITE 1: note = MISC_FEATURE - Xaa at position 1 is DesTyr
  SITE 2: note = MISC_FEATURE - Xaa at position 2 is Aib
  MOD_RES 17: note = Lys at position 17 is chemically modified by conjugation of the epsilon-amino group of the Lys side chain with (2-[2-(2-amino-ethoxy)-ethoxy]-acetyl)2-(gamma-Glu)-CO-(CH2)18-CO 2H
  MOD_RES 39: note = Ser at position 39 is amidated
XXEGTFTSDYSILLDEKAQQAFIEYLIEGGPSSGAPPPS

SEQ ID NO: 209 - protein, 39 aa, synthetic construct
  REGION 1..39: note = Synthetic Construct
  SITE 1: note = MISC_FEATURE - Xaa at position 1 is DesTyr
  MOD_RES 17: note = Lys at position 17 is chemically modified by conjugation of the epsilon-amino group of the Lys side chain with (2-[2-(2-amino-ethoxy)-ethoxy]-acetyl)2-(gamma-Glu)-CO-(CH2)18-CO 2H
  MOD_RES 39: note = Ser at position 39 is amidated
XAEGTFTSDYSILLDEKAQQAFIEYLIEGGPSSGAPPPS

SEQ ID NO: 210 - protein, 39 aa, synthetic construct; identical to SEQ ID NO: 208
  REGION 1..39: note = Synthetic Construct
  SITE 1: note = MISC_FEATURE - Xaa at position 1 is DesHis
  SITE 2: note = MISC_FEATURE - Xaa at position 2 is alpha-methyl-Pro
  MOD_RES 17: note = Lys at position 17 is chemically modified by conjugation of the epsilon-amino group of the Lys side chain with (2-[2-(2-amino-ethoxy)-ethoxy]-acetyl)2-(gamma-Glu)-CO-(CH2)18-CO 2H
  MOD_RES 39: note = Ser at position 39 is amidated

SEQ ID NO: 211 - protein, 39 aa, synthetic construct
  REGION 1..39: note = Synthetic Construct
  SITE 2: note = MISC_FEATURE - Xaa at position 2 is Aib
  SITE 6: note = MISC_FEATURE - Xaa at position 6 is alpha-methyl-Phe(2F)
  SITE 10: note = MISC_FEATURE - Xaa at position 10 is 4Pal
  SITE 13: note = MISC_FEATURE - Xaa at position 13 is alpha-methyl-Leu
  MOD_RES 17: note = Lys at position 17 is chemically modified by conjugation of the epsilon-amino group of the Lys side chain with (2-[2-(2-Amino-ethoxy)-ethoxy]-acetyl)-(gamma-Glu)-(2-[2-(2-Amino -ethoxy)-ethoxy]-acetyl)-CO-(CH2)18-CO2H
  SITE 20: note = MISC_FEATURE - Xaa at position 20 is Aib
  SITE 24: note = MISC_FEATURE - Xaa at position 24 is D-Glu
  MOD_RES 39: note = Ser at position 39 is amidated
YXEGTXTSDXSIXLDKKAQXEFIXYLIEGGPSSGAPPPS

SEQ ID NO: 212 - protein, 39 aa, synthetic construct; identical to SEQ ID NO: 211
  REGION 1..39: note = Synthetic Construct
  SITE 2: note = MISC_FEATURE - Xaa at position 2 is Aib
  SITE 6: note = MISC_FEATURE - Xaa at position 6 is alpha-methyl-Phe(2F)
  SITE 10: note = MISC_FEATURE - Xaa at position 10 is 4Pal
  SITE 13: note = MISC_FEATURE - Xaa at position 13 is alpha-methyl-Leu
  MOD_RES 17: note = Lys at position 17 is chemically modified by conjugation of the epsilon-amino group of the Lys side chain with (2-[2-(2-amino-ethoxy)-ethoxy]-acetyl)2-(gamma-Glu)-CO-(CH2)18-CO 2H
  SITE 20: note = MISC_FEATURE - Xaa at position 20 is Aib
  SITE 24: note = MISC_FEATURE - Xaa at position 24 is D-Glu
  MOD_RES 39: note = Ser at position 39 is amidated

SEQ ID NO: 213 - protein, 39 aa, synthetic construct; identical to SEQ ID NO: 190
  REGION 1..39: note = Synthetic Construct
  SITE 2: note = MISC_FEATURE - Xaa at position 2 is Aib
  SITE 6: note = MISC_FEATURE - Xaa at position 6 is alpha-methyl-Phe(2F)
  SITE 10: note = MISC_FEATURE - Xaa at position 10 is 4Pal
  SITE 13: note = MISC_FEATURE - Xaa at position 13 is alpha-methyl-Leu
  MOD_RES 17: note = Lys at position 17 is chemically modified by conjugation of the epsilon-amino group of the Lys side chain with (2-[2-(2-amino-ethoxy)-ethoxy]-acetyl)2-(gamma-Glu)-CO-(CH2)16-CO 2H
  SITE 20: note = MISC_FEATURE - Xaa at position 20 is Aib
  SITE 24: note = MISC_FEATURE - Xaa at position 24 is D-Glu
  MOD_RES 39: note = Ser at position 39 is amidated

SEQ ID NO: 214 - protein, 39 aa, synthetic construct; identical to SEQ ID NO: 190
  REGION 1..39: note = Synthetic Construct
  SITE 2: note = MISC_FEATURE - Xaa at position 2 is Aib
  SITE 6: note = MISC_FEATURE - Xaa at position 6 is alpha-methyl-Phe(2F)
  SITE 10: note = MISC_FEATURE - Xaa at position 10 is 4Pal
  SITE 13: note = MISC_FEATURE - Xaa at position 13 is alpha-methyl-Leu
  MOD_RES 17: note = Lys at position 17 is chemically modified by conjugation of the epsilon-amino group of the Lys side chain with (2-[2-(2-amino-ethoxy)-ethoxy]-acetyl)2-CO-(CH2)16-CO2H
  SITE 20: note = MISC_FEATURE - Xaa at position 20 is Aib
  SITE 24: note = MISC_FEATURE - Xaa at position 24 is D-Glu
  MOD_RES 39: note = Ser at position 39 is amidated

SEQ ID NO: 215 - protein, 39 aa, synthetic construct; identical to SEQ ID NO: 190
  REGION 1..39: note = Synthetic Construct
  SITE 2: note = MISC_FEATURE - Xaa at position 2 is Aib
  SITE 6: note = MISC_FEATURE - Xaa at position 6 is alpha-methyl-Phe(2F)
  SITE 10: note = MISC_FEATURE - Xaa at position 10 is 4Pal
  SITE 13: note = MISC_FEATURE - Xaa at position 13 is alpha-methyl-Leu
  MOD_RES 17: note = Lys at position 17 is chemically modified by conjugation of the epsilon-amino group of the Lys side chain with (2-[2-(2-amino-ethoxy)-ethoxy]-acetyl)2-CO-(CH2)18-CO2H
  SITE 20: note = MISC_FEATURE - Xaa at position 20 is Aib
  SITE 24: note = MISC_FEATURE - Xaa at position 24 is D-Glu
  MOD_RES 39: note = Ser at position 39 is amidated

SEQ ID NO: 216 - protein, 39 aa, synthetic construct; identical to SEQ ID NO: 190
  REGION 1..39: note = Synthetic Construct
  SITE 2: note = MISC_FEATURE - Xaa at position 2 is Aib
  SITE 6: note = MISC_FEATURE - Xaa at position 6 is alpha-methyl-Phe(2F)
  SITE 10: note = MISC_FEATURE - Xaa at position 10 is 4Pal
  SITE 13: note = MISC_FEATURE - Xaa at position 13 is alpha-methyl-Leu
  MOD_RES 17: note = Lys at position 17 is chemically modified by conjugation of the epsilon-amino group of the Lys side chain with (2-[2-(2-Amino-ethoxy)-ethoxy]-acetyl)2-(epsilon-Lys)-CO-(CH2)18- CO2H
  SITE 20: note = MISC_FEATURE - Xaa at position 20 is Aib
  SITE 24: note = MISC_FEATURE - Xaa at position 24 is D-Glu
  MOD_RES 39: note = Ser at position 39 is amidated

SEQ ID NO: 217 - protein, 39 aa, synthetic construct; identical to SEQ ID NO: 10
  REGION 1..39: note = Synthetic Construct
  SITE 2: note = MISC_FEATURE - Xaa at position 2 is Aib
  SITE 6: note = MISC_FEATURE - Xaa at position 6 is alpha-methyl-Phe(2F)
  SITE 13: note = MISC_FEATURE - Xaa at position 13 is alpha-methyl-Leu
  MOD_RES 17: note = Lys at position 17 is chemically modified by conjugation of the epsilon-amino group of the Lys side chain with (2-[2-(2-amino-ethoxy)-ethoxy]-acetyl)2-(gamma-Glu)-CO-(CH2)14-CO 2H
  SITE 20: note = MISC_FEATURE - Xaa at position 20 is Aib
  SITE 24: note = MISC_FEATURE - Xaa at position 24 is D-Glu
  MOD_RES 39: note = Ser at position 39 is amidated

SEQ ID NO: 218 - protein, 39 aa, synthetic construct; identical to SEQ ID NO: 11
  REGION 1..39: note = Synthetic Construct
  SITE 2: note = MISC_FEATURE - Xaa at position 2 is Aib
  SITE 6: note = MISC_FEATURE - Xaa at position 6 is alpha-methyl-Phe(2F)
  SITE 13: note = MISC_FEATURE - Xaa at position 13 is alpha-methyl-Leu
  SITE 16: note = MISC_FEATURE - Xaa at position 16 is Dab
  MOD_RES 17: note = Lys at position 17 is chemically modified by conjugation of the epsilon-amino group of the Lys side chain with (2-[2-(2-amino-ethoxy)-ethoxy]-acetyl)2-(gamma-Glu)-CO-(CH2)16-CO 2H
  SITE 20: note = MISC_FEATURE - Xaa at position 20 is Aib
  SITE 24: note = MISC_FEATURE - Xaa at position 24 is D-Glu
  MOD_RES 39: note = Ser at position 39 is amidated

SEQ ID NO: 219 - protein, 39 aa, synthetic construct; identical to SEQ ID NO: 11
  REGION 1..39: note = Synthetic Construct
  SITE 2: note = MISC_FEATURE - Xaa at position 2 is Aib
  SITE 6: note = MISC_FEATURE - Xaa at position 6 is alpha-methyl-Phe(2F)
  SITE 13: note = MISC_FEATURE - Xaa at position 13 is alpha-methyl-Leu
  SITE 16: note = MISC_FEATURE - Xaa at position 16 is Dap
  MOD_RES 17: note = Lys at position 17 is chemically modified by conjugation of the epsilon-amino group of the Lys side chain with (2-[2-(2-amino-ethoxy)-ethoxy]-acetyl)2-(gamma-Glu)-CO-(CH2)16-CO 2H
  SITE 20: note = MISC_FEATURE - Xaa at position 20 is Aib
  SITE 24: note = MISC_FEATURE - Xaa at position 24 is D-Glu
  MOD_RES 39: note = Ser at position 39 is amidated

SEQ ID NO: 220 - protein, 39 aa, synthetic construct
  REGION 1..39: note = Synthetic Construct
  SITE 2: note = MISC_FEATURE - Xaa at position 2 is Aib
  SITE 6: note = MISC_FEATURE - Xaa at position 6 is alpha-methyl-Phe(2F)
  SITE 13: note = MISC_FEATURE - Xaa at position 13 is alpha-methyl-Leu
  MOD_RES 17: note = Lys at position 17 is chemically modified by conjugation of the epsilon-amino group of the Lys side chain with (2-[2-(2-Amino-ethoxy)-ethoxy]-acetyl)-(gamma-Glu)-(2-[2-(2-Amino -ethoxy)-ethoxy]-acetyl)-CO-(CH2)18-CO2H
  SITE 20: note = MISC_FEATURE - Xaa at position 20 is Aib
  SITE 24: note = MISC_FEATURE - Xaa at position 24 is D-Glu
  MOD_RES 39: note = Ser at position 39 is amidated
YXEGTXTSDYSIXLDKKAQXEFIXYLIEGGPSSGAPPPS

SEQ ID NO: 221 - protein, 39 aa, synthetic construct; identical to SEQ ID NO: 220
  REGION 1..39: note = Synthetic Construct
  SITE 2: note = MISC_FEATURE - Xaa at position 2 is Aib
  SITE 6: note = MISC_FEATURE - Xaa at position 6 is alpha-methyl-Phe(2F)
  SITE 13: note = MISC_FEATURE - Xaa at position 13 is alpha-methyl-Leu
  MOD_RES 17: note = Lys at position 17 is chemically modified by conjugation of the epsilon-amino group of the Lys side chain with (2-[2-(2-amino-ethoxy)-ethoxy]-acetyl)2-(gamma-Glu)-CO-(CH2)18-CO 2H
  SITE 20: note = MISC_FEATURE - Xaa at position 20 is Aib
  SITE 24: note = MISC_FEATURE - Xaa at position 24 is D-Glu
  MOD_RES 39: note = Ser at position 39 is amidated

SEQ ID NO: 222 - protein, 39 aa, synthetic construct; identical to SEQ ID NO: 10
  REGION 1..39: note = Synthetic Construct
  SITE 2: note = MISC_FEATURE - Xaa at position 2 is Aib
  SITE 6: note = MISC_FEATURE - Xaa at position 6 is alpha-methyl-Phe
  SITE 13: note = MISC_FEATURE - Xaa at position 13 is alpha-methyl-Leu
  MOD_RES 17: note = Lys at position 17 is chemically modified by conjugation of the epsilon-amino group of the Lys side chain with (2-[2-(2-amino-ethoxy)-ethoxy]-acetyl)2-(gamma-Glu)-CO-(CH2)16-CO 2H
  SITE 20: note = MISC_FEATURE - Xaa at position 20 is Aib
  SITE 24: note = MISC_FEATURE - Xaa at position 24 is D-Glu
  MOD_RES 39: note = Ser at position 39 is amidated

SEQ ID NO: 223 - protein, 39 aa, synthetic construct; identical to SEQ ID NO: 10
  REGION 1..39: note = Synthetic Construct
  SITE 2: note = MISC_FEATURE - Xaa at position 2 is Aib
  SITE 6: note = MISC_FEATURE - Xaa at position 6 is alpha-methyl-Phe(2F)
  SITE 13: note = MISC_FEATURE - Xaa at position 13 is alpha-methyl-Leu
  MOD_RES 17: note = Lys at position 17 is chemically modified by conjugation of the epsilon-amino group of the Lys side chain with (2-[2-(2-amino-ethoxy)-ethoxy]-acetyl)2-CO-(CH2)16-CO2H
  SITE 20: note = MISC_FEATURE - Xaa at position 20 is Aib
  SITE 24: note = MISC_FEATURE - Xaa at position 24 is D-Glu
  MOD_RES 39: note = Ser at position 39 is amidated

SEQ ID NO: 224 - protein, 39 aa, synthetic construct; identical to SEQ ID NO: 10
  REGION 1..39: note = Synthetic Construct
  SITE 2: note = MISC_FEATURE - Xaa at position 2 is Aib
  SITE 6: note = MISC_FEATURE - Xaa at position 6 is alpha-methyl-Phe(2F)
  SITE 13: note = MISC_FEATURE - Xaa at position 13 is alpha-methyl-Leu
  MOD_RES 17: note = Lys at position 17 is chemically modified by conjugation of the epsilon-amino group of the Lys side chain with (2-[2-(2-amino-ethoxy)-ethoxy]-acetyl)2-CO-(CH2)18-CO2H
  SITE 20: note = MISC_FEATURE - Xaa at position 20 is Aib
  SITE 24: note = MISC_FEATURE - Xaa at position 24 is D-Glu
  MOD_RES 39: note = Ser at position 39 is amidated

SEQ ID NO: 225 - protein, 39 aa, synthetic construct; identical to SEQ ID NO: 10
  REGION 1..39: note = Synthetic Construct
  SITE 2: note = MISC_FEATURE - Xaa at position 2 is Aib
  SITE 6: note = MISC_FEATURE - Xaa at position 6 is alpha-methyl-Phe(2F)
  SITE 13: note = MISC_FEATURE - Xaa at position 13 is alpha-methyl-Leu
  MOD_RES 17: note = Lys at position 17 is chemically modified by conjugation of the epsilon-amino group of the Lys side chain with (2-[2-(2-amino-ethoxy)-ethoxy]-acetyl)2-(epsilon-Lys)-CO-(CH2)18- CO2H
  SITE 20: note = MISC_FEATURE - Xaa at position 20 is Aib
  SITE 24: note = MISC_FEATURE - Xaa at position 24 is D-Glu
  MOD_RES 39: note = Ser at position 39 is amidated

SEQ ID NO: 226 - protein, 39 aa, synthetic construct; identical to SEQ ID NO: 11
  REGION 1..39: note = Synthetic Construct
  SITE 2: note = MISC_FEATURE - Xaa at position 2 is Aib
  SITE 6: note = MISC_FEATURE - Xaa at position 6 is alpha-methyl-Phe(2F)
  SITE 13: note = MISC_FEATURE - Xaa at position 13 is alpha-methyl-Leu
  SITE 16: note = MISC_FEATURE - Xaa at position 16 is Dab
  MOD_RES 17: note = Lys at position 17 is chemically modified by conjugation of the epsilon-amino group of the Lys side chain with (2-[2-(2-amino-ethoxy)-ethoxy]-acetyl)2-(gamma-Glu)-CO-(CH2)18-CO 2H
  SITE 20: note = MISC_FEATURE - Xaa at position 20 is Aib
  SITE 24: note = MISC_FEATURE - Xaa at position 24 is D-Glu
  MOD_RES 39: note = Ser at position 39 is amidated

SEQ ID NO: 227 - protein, 39 aa, synthetic construct; identical to SEQ ID NO: 11
  REGION 1..39: note = Synthetic Construct
  SITE 2: note = MISC_FEATURE - Xaa at position 2 is Aib
  SITE 6: note = MISC_FEATURE - Xaa at position 6 is alpha-methyl-Phe(2F)
  SITE 13: note = MISC_FEATURE - Xaa at position 13 is alpha-methyl-Leu
  SITE 16: note = MISC_FEATURE - Xaa at position 16 is Dap
  MOD_RES 17: note = Lys at position 17 is chemically modified by conjugation of the epsilon-amino group of the Lys side chain with (2-[2-(2-amino-ethoxy)-ethoxy]-acetyl)2-(gamma-Glu)-CO-(CH2)18-CO 2H
  SITE 20: note = MISC_FEATURE - Xaa at position 20 is Aib
  SITE 24: note = MISC_FEATURE - Xaa at position 24 is D-Glu
  MOD_RES 39: note = Ser at position 39 is amidated

SEQ ID NO: 228 - protein, 34 aa, synthetic construct
  REGION 1..34: note = Synthetic Construct
  SITE 2: note = MISC_FEATURE - Xaa at position 2 is Aib
  SITE 6: note = MISC_FEATURE - Xaa at position 6 is alpha-methyl-Phe(2F)
  SITE 13: note = MISC_FEATURE - Xaa at position 13 is alpha-methyl-Leu
  MOD_RES 17: note = Lys at position 17 is chemically modified by conjugation of the epsilon-amino group of the Lys side chain with (2-[2-(2-amino-ethoxy)-ethoxy]-acetyl)2-(gamma-Glu)-CO-(CH2)16-CO 2H
  SITE 20: note = MISC_FEATURE - Xaa at position 20 is Aib
  SITE 24: note = MISC_FEATURE - Xaa at position 24 is D-Glu
  MOD_RES 34: note = Gly at position 34 is amidated
YXEGTXTSDYSIXLDEKAQXEFIXYLIEGGPSSG

SEQ ID NO: 229 - protein, 30 aa, synthetic construct
  REGION 1..30: note = Synthetic Construct
  SITE 2: note = MISC_FEATURE - Xaa at position 2 is Aib
  SITE 6: note = MISC_FEATURE - Xaa at position 6 is alpha-methyl-Phe(2F)
  SITE 13: note = MISC_FEATURE - Xaa at position 13 is alpha-methyl-Leu
  MOD_RES 17: note = Lys at position 17 is chemically modified by conjugation of the epsilon-amino group of the Lys side chain with (2-[2-(2-amino-ethoxy)-ethoxy]-acetyl)2-(gamma-Glu)-CO-(CH2)16-CO 2H
  SITE 20: note = MISC_FEATURE - Xaa at position 20 is Aib
  SITE 24: note = MISC_FEATURE - Xaa at position 24 is D-Glu
  MOD_RES 30: note = Gly at position 30 is amidated
YXEGTXTSDYSIXLDEKAQXEFIXYLIEGG

SEQ ID NO: 230 - protein, 39 aa, synthetic construct; identical to SEQ ID NO: 10
  REGION 1..39: note = Synthetic Construct
  SITE 2: note = MISC_FEATURE - Xaa at position 2 is Aib
  SITE 6: note = MISC_FEATURE - Xaa at position 6 is alpha-methyl-Phe(2F)
  SITE 13: note = MISC_FEATURE - Xaa at position 13 is alpha-methyl-Leu
  MOD_RES 17: note = Lys at position 17 is chemically modified by conjugation of the epsilon-amino group of the Lys side chain with (2-[2-(2-amino-ethoxy)-ethoxy]-acetyl)2-(gamma-Glu)-CO-(CH2)16-CO 2H
  SITE 20: note = MISC_FEATURE - Xaa at position 20 is Aib
  SITE 24: note = MISC_FEATURE - Xaa at position 24 is D-Glu
  MOD_RES 39: note = Ser at position 39 is amidated

SEQ ID NO: 231 - protein, 39 aa, synthetic construct
  REGION 1..39: note = Synthetic Construct
  SITE 2: note = MISC_FEATURE - Xaa at position 2 is Aib
  SITE 6: note = MISC_FEATURE - Xaa at position 6 is alpha-methyl-Phe(2F)
  SITE 13: note = MISC_FEATURE - Xaa at position 13 is alpha-methyl-Leu
  MOD_RES 17: note = Lys at position 17 is chemically modified by conjugation of the epsilon-amino group of the Lys side chain with (2-[2-(2-amino-ethoxy)-ethoxy]-acetyl)2-(gamma-Glu)-CO-(CH2)18-CO 2H
  SITE 20: note = MISC_FEATURE - Xaa at position 20 is Aib
  SITE 24: note = MISC_FEATURE - Xaa at position 24 is D-Glu
  SITE 25: note = MISC_FEATURE - Xaa at position 25 alpha-methyl-Tyr
  MOD_RES 39: note = Ser at position 39 is amidated
YXEGTXTSDYSIXLDEKAQXEFIXXLIEGGPSSGAPPPS

SEQ ID NO: 232 - protein, 39 aa, synthetic construct
  REGION 1..39: note = Synthetic Construct
  SITE 2: note = MISC_FEATURE - Xaa at position 2 is Aib
  SITE 6: note = MISC_FEATURE - Xaa at position 6 is alpha-methyl-Phe(2F)
  SITE 13: note = MISC_FEATURE - Xaa at position 13 is alpha-methyl-Leu
  MOD_RES 17: note = Lys at position 17 is chemically modified by conjugation of the epsilon-amino group of the Lys side chain with (2-[2-(2-amino-ethoxy)-ethoxy]-acetyl)2-(gamma-Glu)-CO-(CH2)18-CO 2H
  SITE 20: note = MISC_FEATURE - Xaa at position 20 is Aib
  SITE 25: note = MISC_FEATURE - Xaa at position 25 is alpha-methyl-Tyr
  MOD_RES 39: note = Ser at position 39 is amidated
YXEGTXTSDYSIXLDEKAQXEFIEXLIEGGPSSGAPPPS

SEQ ID NO: 233 - protein, 39 aa, synthetic construct; identical to SEQ ID NO: 10
  REGION 1..39: note = Synthetic Construct
  SITE 2: note = MISC_FEATURE - Xaa at position 2 is Aib
  SITE 6: note = MISC_FEATURE - Xaa at position 6 is alpha-methyl-Phe(2F)
  SITE 13: note = MISC_FEATURE - Xaa at position 13 is Aib
  MOD_RES 17: note = Lys at position 17 is chemically modified by conjugation of the epsilon-amino group of the Lys side chain with (2-[2-(2-amino-ethoxy)-ethoxy]-acetyl)2-(gamma-Glu)-CO-(CH2)18-CO 2H
  SITE 20: note = MISC_FEATURE - Xaa at position 20 is Aib
  SITE 24: note = MISC_FEATURE - Xaa at position 24 is D-Glu
  MOD_RES 39: note = Ser at position 39 is amidated

SEQ ID NO: 234 - protein, 39 aa, synthetic construct; identical to SEQ ID NO: 10
  REGION 1..39: note = Synthetic Construct
  SITE 2: note = MISC_FEATURE - Xaa at position 2 is Aib
  SITE 6: note = MISC_FEATURE - Xaa at position 6 is alpha-methyl-Phe
  SITE 13: note = MISC_FEATURE - Xaa at position 13 is Aib
  MOD_RES 17: note = Lys at position 17 is chemically modified by conjugation of the epsilon-amino group of the Lys side chain with (2-[2-(2-amino-ethoxy)-ethoxy]-acetyl)2-(gamma-Glu)-CO-(CH2)18-CO 2H
  SITE 20: note = MISC_FEATURE - Xaa at position 20 is Aib
  SITE 24: note = MISC_FEATURE - Xaa at position 24 is D-Glu
  MOD_RES 39: note = Ser at position 39 is amidated

SEQ ID NO: 235 - protein, 39 aa, synthetic construct
  REGION 1..39: note = Synthetic Construct
  SITE 2: note = MISC_FEATURE - Xaa at position 2 is Aib
  SITE 6: note = MISC_FEATURE - Xaa at position 6 is alpha-methyl-Phe(2F)
  MOD_RES 17: note = Lys at position 17 is chemically modified by conjugation of the epsilon-amino group of the Lys side chain with (2-[2-(2-amino-ethoxy)-ethoxy]-acetyl)2-(gamma-Glu)-CO-(CH2)18-CO 2H
  SITE 20: note = MISC_FEATURE - Xaa at position 20 is Aib
  SITE 24: note = MISC_FEATURE - Xaa at position 24 is D-Glu
  MOD_RES 39: note = Ser at position 39 is amidated
YXEGTXTSDYSILLDEKAQXEFIXYLIEGGPSSGAPPPS

SEQ ID NO: 236 - protein, 39 aa, synthetic construct; identical to SEQ ID NO: 10
  REGION 1..39: note = Synthetic Construct
  SITE 2: note = MISC_FEATURE - Xaa at position 2 is Aib
  SITE 6: note = MISC_FEATURE - Xaa at position 6 is alpha-methyl-Phe
  SITE 13: note = MISC_FEATURE - Xaa at position 13 is alpha-methyl-Leu
  MOD_RES 17: note = Lys at position 17 is chemically modified by conjugation of the epsilon-amino group of the Lys side chain with (2-[2-(2-amino-ethoxy)-ethoxy]-acetyl)2-(gamma-Glu)-CO-(CH2)18-CO 2H
  SITE 20: note = MISC_FEATURE - Xaa at position 20 is Aib
  SITE 24: note = MISC_FEATURE - Xaa at position 24 is D-Glu
  MOD_RES 39: note = Ser at position 39 is amidated

SEQ ID NO: 237 - protein, 34 aa, synthetic construct
  REGION 1..34: note = Synthetic Construct
  SITE 2: note = MISC_FEATURE - Xaa at position 2 is Aib
  SITE 6: note = MISC_FEATURE - Xaa at position 6 is alpha-methyl-Phe
  SITE 13: note = MISC_FEATURE - Xaa at position 13 is alpha-methyl-Leu
  MOD_RES 17: note = Lys at position 17 is chemically modified by conjugation of the epsilon-amino group of the Lys side chain with (2-[2-(2-amino-ethoxy)-ethoxy]-acetyl)2-(gamma-Glu)-CO-(CH2)18-CO 2H
  SITE 20: note = MISC_FEATURE - Xaa at position 20 is Aib
  SITE 24: note = MISC_FEATURE - Xaa at position 24 is D-Glu
  MOD_RES 34: note = Gly at position 34 is amidated
YXEGTXTSDYSIXLDKKAQXEFIXYLIEGGPSSG

SEQ ID NO: 238 - protein, 38 aa, synthetic construct
  REGION 1..38: note = Synthetic Construct
  SITE 2: note = MISC_FEATURE - Xaa at position 2 is Aib
  SITE 6: note = MISC_FEATURE - Xaa at position 6 is alpha-methyl-Phe(2F)
  SITE 12: note = MISC_FEATURE - Xaa at position 12 is alpha-methyl-Leu
  MOD_RES 16: note = Lys at position 16 is chemically modified by conjugation of the epsilon-amino group of the Lys side chain with (2-[2-(2-amino-ethoxy)-ethoxy]-acetyl)2-(gamma-Glu)-CO-(CH2)18-CO 2H
  SITE 19: note = MISC_FEATURE - Xaa at position 19 is Aib
  SITE 23: note = MISC_FEATURE - Xaa at position 23 is D-Glu
  MOD_RES 38: note = Ser at position 39 is amidated
YXEGTXTSDYSXLDEKAQXEFIXYLIEGGPSSGAPPPS

SEQ ID NO: 239 - protein, 39 aa, synthetic construct
  REGION 1..39: note = Synthetic Construct
  SITE 2: note = MISC_FEATURE - Xaa at position 2 is Aib
  SITE 6: note = MISC_FEATURE - Xaa at position 6 is alpha-methyl-Phe(2F)
  SITE 13: note = MISC_FEATURE - Xaa at position 13 is alpha-methyl-Leu
  MOD_RES 17: note = Lys at position 17 is chemically modified by conjugation of the epsilon-amino group of the Lys side chain with (2-[2-(2-amino-ethoxy)-ethoxy]-acetyl)2-(gamma-Glu)-CO-(CH2)18-CO 2H
  SITE 20: note = MISC_FEATURE - Xaa at position 20 is Aib
  SITE 24: note = MISC_FEATURE - Xaa at position 24 is D-Glu
  MOD_RES 39: note = Ser at position 39 is amidated
YXEGTXTSDYSIXLDHKAQXEFIXYLIEGGPSSGAPPPS

SEQ ID NO: 240 - protein, 39 aa, synthetic construct; identical to SEQ ID NO: 220
  REGION 1..39: note = Synthetic Construct
  SITE 2: note = MISC_FEATURE - Xaa at position 2 is Aib
  SITE 6: note = MISC_FEATURE - Xaa at position 6 is alpha-methyl-Phe(2F)
  SITE 13: note = MISC_FEATURE - Xaa at position 13 is alpha-methyl-Leu
  MOD_RES 17: note = Lys at position 17 is chemically modified by conjugation of the epsilon-amino group of the Lys side chain with (2-[2-(2-amino-ethoxy)-ethoxy]-acetyl)2-(gamma-Glu)-CO-(CH2)16-CO 2H
  SITE 20: note = MISC_FEATURE - Xaa at position 20 is Aib
  SITE 24: note = MISC_FEATURE - Xaa at position 24 is D-Glu
  MOD_RES 39: note = Ser at position 39 is amidated

SEQ ID NO: 241 - protein, 39 aa, synthetic construct
  REGION 1..39: note = Synthetic Construct
  SITE 2: note = MISC_FEATURE - Xaa at position 2 is Aib
  SITE 6: note = MISC_FEATURE - Xaa at position 6 is alpha-methyl-Phe(2F)
  SITE 10: note = MISC_FEATURE - Xaa at position 10 is 4Pal
  SITE 13: note = MISC_FEATURE - Xaa at position 13 is alpha-methyl-Leu
  SITE 16: note = MISC_FEATURE - Xaa at position 16 is Orn
  MOD_RES 17: note = Lys at position 17 is chemically modified by conjugation of the epsilon-amino group of the Lys side chain with (2-[2-(2-amino-ethoxy)-ethoxy]-acetyl)2-(gamma-Glu)-CO-(CH2)16-CO 2H
  SITE 20: note = MISC_FEATURE - Xaa at position 20 is Aib
  SITE 24: note = MISC_FEATURE - Xaa at position 24 is D-Glu
  MOD_RES 39: note = Ser at position 39 is amidated
YXEGTXTSDXSIXLDXKAQXEFIXYLIEGGPSSGAPPPS

SEQ ID NO: 242 - protein, 39 aa, synthetic construct; identical to SEQ ID NO: 241
  REGION 1..39: note = Synthetic Construct
  SITE 2: note = MISC_FEATURE - Xaa at position 2 is Aib
  SITE 6: note = MISC_FEATURE - Xaa at position 6 is alpha-methyl-Phe(2F)
  SITE 10: note = MISC_FEATURE - Xaa at position 10 is 4Pal
  SITE 13: note = MISC_FEATURE - Xaa at position 13 is alpha-methyl-Leu
  SITE 16: note = MISC_FEATURE - Xaa at position 16 is Dab
  MOD_RES 17: note = Lys at position 17 is chemically modified by conjugation of the epsilon-amino group of the Lys side chain with (2-[2-(2-amino-ethoxy)-ethoxy]-acetyl)2-(gamma-Glu)-CO-(CH2)16-CO 2H
  SITE 20: note = MISC_FEATURE - Xaa at position 20 is Aib
  SITE 24: note = MISC_FEATURE - Xaa at position 24 is D-Glu
  MOD_RES 39: note = Ser at position 39 is amidated

SEQ ID NO: 243 - protein, 39 aa, synthetic construct
  REGION 1..39: note = Synthetic Construct
  SITE 2: note = MISC_FEATURE - Xaa at position 2 is Aib
  SITE 6: note = MISC_FEATURE - Xaa at position 6 is alpha-methyl-Phe(2F)
  SITE 10: note = MISC_FEATURE - Xaa at position 10 is 4Pal
  SITE 16: note = MISC_FEATURE - Xaa at position 16 is Dab
  MOD_RES 17: note = Lys at position 17 is chemically modified by conjugation of the epsilon-amino group of the Lys side chain with (2-[2-(2-amino-ethoxy)-ethoxy]-acetyl)2-(gamma-Glu)-CO-(CH2)16-CO 2H
  SITE 20: note = MISC_FEATURE - Xaa at position 20 is Aib
  SITE 24: note = MISC_FEATURE - Xaa at position 24 is D-Glu
  MOD_RES 39: note = Ser at position 39 is amidated
YXEGTXTSDXSILLDXKAQXEFIXYLIEGGPSSGAPPPS

SEQ ID NO: 244 - protein, 39 aa, synthetic construct; identical to SEQ ID NO: 241
  REGION 1..39: note = Synthetic Construct
  SITE 2: note = MISC_FEATURE - Xaa at position 2 is Aib
  SITE 6: note = MISC_FEATURE - Xaa at position 6 is alpha-methyl-Phe
  SITE 10: note = MISC_FEATURE - Xaa at position 10 is 4Pal
  SITE 13: note = MISC_FEATURE - Xaa at position 13 is alpha-methyl-Leu
  SITE 16: note = MISC_FEATURE - Xaa at position 16 is Dab
  MOD_RES 17: note = Lys at position 17 is chemically modified by conjugation of the epsilon-amino group of the Lys side chain with (2-[2-(2-amino-ethoxy)-ethoxy]-acetyl)2-(gamma-Glu)-CO-(CH2)16-CO 2H
  SITE 20: note = MISC_FEATURE - Xaa at position 20 is Aib
  SITE 24: note = MISC_FEATURE - Xaa at position 24 is D-Glu
  MOD_RES 39: note = Ser at position 39 is amidated

SEQ ID NO: 245 - protein, 39 aa, synthetic construct
  REGION 1..39: note = Synthetic Construct
  SITE 2: note = MISC_FEATURE - Xaa at position 2 is Aib
  SITE 6: note = MISC_FEATURE - Xaa at position 6 is alpha-methyl-Phe(2F)
  SITE 13: note = MISC_FEATURE - Xaa at position 13 is alpha-methyl-Leu
  SITE 16: note = MISC_FEATURE - Xaa at position 16 is Orn
  MOD_RES 17: note = Lys at position 17 is chemically modified by conjugation of the epsilon-amino group of the Lys side chain with (2-[2-(2-amino-ethoxy)-ethoxy]-acetyl)2-(gamma-Glu)-CO-(CH2)16-CO 2H
  SITE 20: note = MISC_FEATURE - Xaa at position 20 is Aib
  SITE 24: note = MISC_FEATURE - Xaa at position 24 is D-Glu
  SITE 25: note = MISC_FEATURE - Xaa at position 25 is alpha-methyl-Tyr
  MOD_RES 39: note = Ser at position 39 is amidated
YXEGTXTSDYSIXLDXKAQXEFIXXLIEGGPSSGAPPPS

SEQ ID NO: 246 - protein, 39 aa, synthetic construct
  REGION 1..39: note = Synthetic Construct
  SITE 2: note = MISC_FEATURE - Xaa at position 2 is Aib
  SITE 6: note = MISC_FEATURE - Xaa at position 6 is alpha-methyl-Phe(2F)
  SITE 13: note = MISC_FEATURE - Xaa at position 13 is alpha-methyl-Leu
  SITE 16: note = MISC_FEATURE - Xaa at position 16 is Orn
  MOD_RES 17: note = Lys at position 17 is chemically modified by conjugation of the epsilon-amino group of the Lys side chain with (2-[2-(2-amino-ethoxy)-ethoxy]-acetyl)2-(gamma-Glu)-CO-(CH2)16-CO 2H
  SITE 20: note = MISC_FEATURE - Xaa at position 20 is Aib
  SITE 24: note = MISC_FEATURE - Xaa at position 24 is D-Glu
  SITE 25: note = MISC_FEATURE - Xaa at position 25 alpha-methyl-Tyr
  MOD_RES 39: note = Ser at position 39 is amidated
YXEGTXTSDASIXLDXKAQXEFIXXLIEGGPSSGAPPPS

SEQ ID NO: 247 - protein, 39 aa, synthetic construct
  REGION 1..39: note = Synthetic Construct
  SITE 2: note = MISC_FEATURE - Xaa at position 2 is Aib
  SITE 6: note = MISC_FEATURE - Xaa at position 6 is alpha-methyl-Phe(2F)
  SITE 13: note = MISC_FEATURE - Xaa at position 13 is alpha-methyl-Leu
  SITE 16: note = MISC_FEATURE - Xaa at position 16 is Orn
  MOD_RES 17: note = Lys at position 17 is chemically modified by conjugation of the epsilon-amino group of the Lys side chain with (2-[2-(2-amino-ethoxy)-ethoxy]-acetyl)2-(gamma-Glu)-CO-(CH2)16-CO 2H
  SITE 20: note = MISC_FEATURE - Xaa at position 20 is Aib
  SITE 24: note = MISC_FEATURE - Xaa at position 24 is D-Glu
  SITE 25: note = MISC_FEATURE - Xaa at position 25 is alpha-methyl-Tyr
  MOD_RES 39: note = Ser at position 39 is amidated
YXEGTXTSDLSIXLDXKAQXEFIXXLIEGGPSSGAPPPS

SEQ ID NO: 248 - protein, 39 aa, synthetic construct
  REGION 1..39: note = Synthetic Construct
  SITE 2: note = MISC_FEATURE - Xaa at position 2 is Aib
  SITE 6: note = MISC_FEATURE - Xaa at position 6 is alpha-methyl-Phe(2F)
  SITE 10: note = MISC_FEATURE - Xaa at position 10 is 4Pal
  SITE 13: note = MISC_FEATURE - Xaa at position 13 is alpha-methyl-Leu
  SITE 16: note = MISC_FEATURE - Xaa at position 16 is Orn
  MOD_RES 17: note = Lys at position 17 is chemically modified by conjugation of the epsilon-amino group of the Lys side chain with (2-[2-(2-amino-ethoxy)-ethoxy]-acetyl)2-(gamma-Glu)-CO-(CH2)16-CO 2H
  SITE 20: note = MISC_FEATURE - Xaa at position 20 is Aib
  SITE 24: note = MISC_FEATURE - Xaa at position 24 is D-Glu
  SITE 25: note = MISC_FEATURE - Xaa at position 25 is alpha-methyl-Tyr
  MOD_RES 39: note = Ser at position 39 is amidated
YXEGTXTSDXSIXLDXKAQXTFIXXLIEGGPSSGAPPPS

SEQ ID NO: 249 - protein, 39 aa, synthetic construct
  REGION 1..39: note = Synthetic Construct
  SITE 2: note = MISC_FEATURE - Xaa at position 2 is Aib
  SITE 6: note = MISC_FEATURE - Xaa at position 6 is alpha-methyl-Phe(2F)
  SITE 10: note = MISC_FEATURE - Xaa at position 10 is 4Pal
  SITE 13: note = MISC_FEATURE - Xaa at position 13 is alpha-methyl-Leu
  SITE 16: note = MISC_FEATURE - Xaa at position 16 is Orn
  MOD_RES 17: note = Lys at position 17 is chemically modified by conjugation of the epsilon-amino group of the Lys side chain with (2-[2-(2-amino-ethoxy)-ethoxy]-acetyl)2-(gamma-Glu)-CO-(CH2)16-CO 2H
  SITE 20: note = MISC_FEATURE - Xaa at position 20 is Aib
  SITE 24: note = MISC_FEATURE - Xaa at position 24 is D-Glu
  SITE 25: note = MISC_FEATURE - Xaa at position 25 is alpha-methyl-Tyr
  MOD_RES 39: note = Ser at position 39 is amidated
YXEGTXTSDXSIXLDXKAQXAFIXXLIEGGPSSGAPPPS

SEQ ID NO: 250 - protein, 39 aa, synthetic construct
  REGION 1..39: note = Synthetic Construct
  SITE 2: note = MISC_FEATURE - Xaa at position 2 is Aib
  SITE 6: note = MISC_FEATURE - Xaa at position 6 is alpha-methyl-Phe(2F)
  SITE 13: note = MISC_FEATURE - Xaa at position 13 is alpha-methyl-Leu
  SITE 16: note = MISC_FEATURE - Xaa at position 16 is Orn
  MOD_RES 17: note = Lys at position 17 is chemically modified by conjugation of the epsilon-amino group of the Lys side chain with (2-[2-(2-amino-ethoxy)-ethoxy]-acetyl)2-(gamma-Glu)-CO-(CH2)16-CO 2H
  SITE 20: note = MISC_FEATURE - Xaa at position 20 is Aib
  SITE 24: note = MISC_FEATURE - Xaa at position 24 is D-Glu
  SITE 25: note = MISC_FEATURE - Xaa at position 25 is alpha-methyl-Tyr
  MOD_RES 39: note = Ser at position 39 is amidated
YXEGTXTSDVSIXLDXKAQXTFIXXLIEGGPSSGAPPPS

SEQ ID NO: 251 - protein, 39 aa, synthetic construct
  REGION 1..39: note = Synthetic Construct
  SITE 2: note = MISC_FEATURE - Xaa at position 2 is Aib
  SITE 6: note = MISC_FEATURE - Xaa at position 6 is alpha-methyl-Phe(2F)
  SITE 13: note = MISC_FEATURE - Xaa at position 13 is alpha-methyl-Leu
  SITE 16: note = MISC_FEATURE - Xaa at position 16 is Orn
  MOD_RES 17: note = Lys at position 17 is chemically modified by conjugation of the epsilon-amino group of the Lys side chain with (2-[2-(2-amino-ethoxy)-ethoxy]-acetyl)2-(gamma-Glu)-CO-(CH2)16-CO 2H
  SITE 20: note = MISC_FEATURE - Xaa at position 20 is Aib
  SITE 24: note = MISC_FEATURE - Xaa at position 24 is D-Glu
  SITE 25: note = MISC_FEATURE - Xaa at position 25 is alpha-methyl-Tyr
  MOD_RES 39: note = Ser at position 39 is amidated
YXEGTXTSDVSIXLDXKAQXAFIXXLIEGGPSSGAPPPS

SEQ ID NO: 252 - protein, 39 aa, synthetic construct
  REGION 1..39: note = Synthetic Construct
  SITE 2: note = MISC_FEATURE - Xaa at position 2 is Aib
  SITE 6: note = MISC_FEATURE - Xaa at position 6 is alpha-methyl-Phe(2F)
  SITE 13: note = MISC_FEATURE - Xaa at position 13 is alpha-methyl-Leu
  SITE 16: note = MISC_FEATURE - Xaa at position 16 is Orn
  MOD_RES 17: note = Lys at position 17 is chemically modified by conjugation of the epsilon-amino group of the Lys side chain with (2-[2-(2-amino-ethoxy)-ethoxy]-acetyl)2-(gamma-Glu)-CO-(CH2)16-CO 2H
  SITE 20: note = MISC_FEATURE - Xaa at position 20 is Aib
  SITE 24: note = MISC_FEATURE - Xaa at position 24 is D-Glu
  SITE 25: note = MISC_FEATURE - Xaa at position 25 is alpha-methyl-Tyr
  MOD_RES 39: note = Ser at position 39 is amidated
YXEGTXTSDLSIXLDXKAQXTFIXXLIEGGPSSGAPPPS

SEQ ID NO: 253 - protein, 39 aa, synthetic construct
  REGION 1..39: note = Synthetic Construct
  SITE 2: note = MISC_FEATURE - Xaa at position 2 is Aib
  SITE 6: note = MISC_FEATURE - Xaa at position 6 is alpha-methyl-Phe(2F)
  SITE 13: note = MISC_FEATURE - Xaa at position 13 is alpha-methyl-Leu
  SITE 16: note = MISC_FEATURE - Xaa at position 16 is Orn
  MOD_RES 17: note = Lys at position 17 is chemically modified by conjugation of the epsilon-amino group of the Lys side chain with (2-[2-(2-amino-ethoxy)-ethoxy]-acetyl)2-(gamma-Glu)-CO-(CH2)16-CO 2H
  SITE 20: note = MISC_FEATURE - Xaa at position 20 is Aib
  SITE 24: note = MISC_FEATURE - Xaa at position 24 is D-Glu
  SITE 25: note = MISC_FEATURE - Xaa at position 25 is alpha-methyl-Tyr
  MOD_RES 39: note = Ser at position 39 is amidated
YXEGTXTSDLSIXLDXKAQXAFIXXLIEGGPSSGAPPPS

SEQ ID NO: 254 - protein, 39 aa, synthetic construct
  REGION 1..39: note = Synthetic Construct
  SITE 2: note = MISC_FEATURE - Xaa at position 2 is Aib
  SITE 6: note = MISC_FEATURE - Xaa at position 6 is alpha-methyl-Phe(2F)
  SITE 13: note = MISC_FEATURE - Xaa at position 13 is alpha-methyl-Leu
  SITE 16: note = MISC_FEATURE - Xaa at position 16 is Orn
  MOD_RES 17: note = Lys at position 17 is chemically modified by conjugation of the epsilon-amino group of the Lys side chain with (2-[2-(2-amino-ethoxy)-ethoxy]-acetyl)2-(gamma-Glu)-CO-(CH2)16-CO 2H
  SITE 20: note = MISC_FEATURE - Xaa at position 20 is Aib
  SITE 24: note = MISC_FEATURE - Xaa at position 24 is D-Glu
  SITE 25: note = MISC_FEATURE - Xaa at position 25 is alpha-methyl-Tyr
  MOD_RES 39: note = Ser at position 39 is amidated
YXEGTXTSDASIXLDXKAQXTFIXXLIEGGPSSGAPPPS

SEQ ID NO: 255 - protein, 39 aa, synthetic construct
  REGION 1..39: note = Synthetic Construct
  SITE 2: note = MISC_FEATURE - Xaa at position 2 is Aib
  SITE 6: note = MISC_FEATURE - Xaa at position 6 is alpha-methyl-Phe(2F)
  SITE 13: note = MISC_FEATURE - Xaa at position 13 is alpha-methyl-Leu
  SITE 16: note = MISC_FEATURE - Xaa at position 16 is Orn
  MOD_RES 17: note = Lys at position 17 is chemically modified by conjugation of the epsilon-amino group of the Lys side chain with (2-[2-(2-amino-ethoxy)-ethoxy]-acetyl)2-(gamma-Glu)-CO-(CH2)16-CO 2H
  SITE 20: note = MISC_FEATURE - Xaa at position 20 is Aib
  SITE 24: note = MISC_FEATURE - Xaa at position 24 is D-Glu
  SITE 25: note = MISC_FEATURE - Xaa at position 25 is alpha-methyl-Tyr
  MOD_RES 39: note = Ser at position 39 is amidated
YXEGTXTSDASIXLDXKAQXAFIXXLIEGGPSSGAPPPS

SEQ ID NO: 256 - protein, 39 aa, synthetic construct; identical to SEQ ID NO: 11
  REGION 1..39: note = Synthetic Construct
  SITE 2: note = MISC_FEATURE - Xaa at position 2 is Aib
  SITE 6: note = MISC_FEATURE - Xaa at position 6 is alpha-methyl-Phe(2F)
  SITE 13: note = MISC_FEATURE - Xaa at position 13 is Aib
  SITE 16: note = MISC_FEATURE - Xaa at position 16 is Orn
  MOD_RES 17: note = Lys at position 17 is chemically modified by conjugation of the epsilon-amino group of the Lys side chain with (2-[2-(2-amino-ethoxy)-ethoxy]-acetyl)2-(gamma-Glu)-CO-(CH2)16-CO 2H
  SITE 20: note = MISC_FEATURE - Xaa at position 20 is Aib
  SITE 24: note = MISC_FEATURE - Xaa at position 24 is D-Glu
  MOD_RES 39: note = Ser at position 39 is amidated

SEQ ID NO: 257 - protein, 39 aa, synthetic construct
  REGION 1..39: note = Synthetic Construct
  SITE 2: note = MISC_FEATURE - Xaa at position 2 is Aib
  SITE 6: note = MISC_FEATURE - Xaa at position 6 is alpha-methyl-Phe(2F)
  SITE 16: note = MISC_FEATURE - Xaa at position 16 is Orn
  MOD_RES 17: note = Lys at position 17 is chemically modified by conjugation of the epsilon-amino group of the Lys side chain with (2-[2-(2-amino-ethoxy)-ethoxy]-acetyl)2-(gamma-Glu)-CO-(CH2)16-CO 2H
  SITE 20: note = MISC_FEATURE - Xaa at position 20 is Aib
  SITE 24: note = MISC_FEATURE - Xaa at position 24 is D-Glu
  MOD_RES 39: note = Ser at position 39 is amidated
YXEGTXTSDYSILLDXKAQXEFIXYLIEGGPSSGAPPPS

SEQ ID NO: 258 - protein, 39 aa, synthetic construct; identical to SEQ ID NO: 11
  REGION 1..39: note = Synthetic Construct
  SITE 2: note = MISC_FEATURE - Xaa at position 2 is Aib
  SITE 6: note = MISC_FEATURE - Xaa at position 6 is alpha-methyl-Phe(2F)
  SITE 13: note = MISC_FEATURE - Xaa at position 13 is Nle
  SITE 16: note = MISC_FEATURE - Xaa at position 16 is Orn
  MOD_RES 17: note = Lys at position 17 is chemically modified by conjugation of the epsilon-amino group of the Lys side chain with (2-[2-(2-amino-ethoxy)-ethoxy]-acetyl)2-(gamma-Glu)-CO-(CH2)16-CO 2H
  SITE 20: note = MISC_FEATURE - Xaa at position 20 is Aib
  SITE 24: note = MISC_FEATURE - Xaa at position 24 is D-Glu
  MOD_RES 39: note = Ser at position 39 is amidated

SEQ ID NO: 259 - protein, 39 aa, synthetic construct; identical to SEQ ID NO: 11
  REGION 1..39: note = Synthetic Construct
  SITE 2: note = MISC_FEATURE - Xaa at position 2 is Aib
  SITE 6: note = MISC_FEATURE - Xaa at position 6 is alpha-methyl-Phe(2F)
  SITE 13: note = MISC_FEATURE - Xaa at position 13 is Aib
  SITE 16: note = MISC_FEATURE - Xaa at position 16 is Orn
  MOD_RES 17: note = Lys at position 17 is chemically modified by conjugation of the epsilon-amino group of the Lys side chain with (2-[2-(2-amino-ethoxy)-ethoxy]-acetyl)2-(gamma-Glu)-CO-(CH2)18-CO 2H
  SITE 20: note = MISC_FEATURE - Xaa at position 20 is Aib
  SITE 24: note = MISC_FEATURE - Xaa at position 24 is D-Glu
  MOD_RES 39: note = Ser at position 39 is amidated

SEQ ID NO: 260 - protein, 39 aa, synthetic construct; identical to SEQ ID NO: 249
  REGION 1..39: note = Synthetic Construct
  SITE 2: note = MISC_FEATURE - Xaa at position 2 is Aib
  SITE 6: note = MISC_FEATURE - Xaa at position 6 is alpha-methyl-Phe(2F)
  SITE 10: note = MISC_FEATURE - Xaa at position 10 is 4Pal
  SITE 13: note = MISC_FEATURE - Xaa at position 13 is alpha-methyl-Leu
  SITE 16: note = MISC_FEATURE - Xaa at position 16 is Orn
  MOD_RES 17: note = Lys at position 17 is chemically modified by conjugation of the epsilon-amino group of the Lys side chain with (2-[2-(2-amino-ethoxy)-ethoxy]-acetyl)2-(epsilon-Lys)-CO-(CH2)18- CO2H
  SITE 20: note = MISC_FEATURE - Xaa at position 20 is Aib
  SITE 24: note = MISC_FEATURE - Xaa at position 24 is D-Glu
  SITE 25: note = MISC_FEATURE - Xaa at position 25 is alpha-methyl-Tyr
  MOD_RES 39: note = Ser at position 39 is amidated

SEQ ID NO: 261 - protein, 39 aa, synthetic construct
  REGION 1..39: note = Synthetic Construct
  SITE 2: note = MISC_FEATURE - Xaa at position 2 is Aib
  SITE 6: note = MISC_FEATURE - Xaa at position 6 is alpha-methyl-Phe(2F)
  SITE 10: note = MISC_FEATURE - Xaa at position 10 is 4Pal
  SITE 13: note = MISC_FEATURE - Xaa at position 13 is alpha-methyl-Leu
  SITE 16: note = MISC_FEATURE - Xaa at position 16 is Orn
  MOD_RES 17: note = Lys at position 17 is chemically modified by conjugation of the epsilon-amino group of the Lys side chain with (2-[2-(2-amino-ethoxy)-ethoxy]-acetyl)2-(epsilon-Lys)-CO-(CH2)18- CO2H
  SITE 20: note = MISC_FEATURE - Xaa at position 20 is Aib
  SITE 24: note = MISC_FEATURE - Xaa at position 24 is D-Glu
  SITE 25: note = MISC_FEATURE - Xaa at position 25 is alpha-methyl-Tyr
  MOD_RES 39: note = Ser at position 39 is amidated
YXEGTXTSDXSIXLDXKAQXAFIXXLIAGGPSSGAPPPS

SEQ ID NO: 262 - protein, 39 aa, synthetic construct
  REGION 1..39: note = Synthetic Construct
  SITE 2: note = MISC_FEATURE - Xaa at position 2 is Aib
  MOD_RES 17: note = Lys at position 17 is chemically modified by conjugation of the epsilon-amino group of the Lys side chain with (2-[2-(2-amino-ethoxy)-ethoxy]-acetyl)2-(gamma-Glu)-CO-(CH2)18-CO 2H
  MOD_RES 39: note = Ser at position 39 is amidated
YXEGTFTSDYSILLDKKAQAAFIEYLIEGGPSSGAPPPS

SEQ ID NO: 263 - protein, 39 aa, synthetic construct
  REGION 1..39: note = Synthetic Construct
  SITE 2: note = MISC_FEATURE - Xaa at position 2 is Aib
  MOD_RES 17: note = Lys at position 17 is chemically modified by conjugation of the epsilon-amino group of the Lys side chain with (2-[2-(2-amino-ethoxy)-ethoxy]-acetyl)2-(gamma-Glu)-CO-(CH2)18-CO 2H
  MOD_RES 39: note = Ser at position 39 is amidated
YXEGTFTSDYSILLDKKAQQAFIEYLIEGGPSSGAPPPS

SEQ ID NO: 264 - protein, 39 aa, synthetic construct
  REGION 1..39: note = Synthetic Construct
  SITE 2: note = MISC_FEATURE - Xaa at position 2 is Aib
  MOD_RES 17: note = Lys at position 17 is chemically modified by conjugation of the epsilon-amino group of the Lys side chain with (2-[2-(2-amino-ethoxy)-ethoxy]-acetyl)2-(gamma-Glu)-CO-(CH2)18-CO 2H
  MOD_RES 39: note = Ser at position 39 is amidated
YXEGTFTSDYSILLDKKAQHAFIEYLIEGGPSSGAPPPS

SEQ ID NO: 265 - protein, 39 aa, synthetic construct
  REGION 1..39: note = Synthetic Construct
  SITE 2: note = MISC_FEATURE - Xaa at position 2 is Aib
  MOD_RES 17: note = Lys at position 17 is chemically modified by conjugation of the epsilon-amino group of the Lys side chain with (2-[2-(2-amino-ethoxy)-ethoxy]-acetyl)2-(gamma-Glu)-CO-(CH2)18-CO 2H
  MOD_RES 39: note = Ser at position 39 is amidated
YXEGTFTSDYSILLDKKAQKAFIEYLIEGGPSSGAPPPS

SEQ ID NO: 266 - protein, 39 aa, synthetic construct
  REGION 1..39: note = Synthetic Construct
  SITE 2: note = MISC_FEATURE - Xaa at position 2 is Aib
  MOD_RES 17: note = Lys at position 17 is chemically modified by conjugation of the epsilon-amino group of the Lys side chain with (2-[2-(2-amino-ethoxy)-ethoxy]-acetyl)2-(gamma-Glu)-CO-(CH2)18-CO 2H
  MOD_RES 39: note = Ser at position 39 is amidated
YXEGTFTSDYSILLDKKAQRAFIEYLIEGGPSSGAPPPS

SEQ ID NO: 267 - protein, 39 aa, synthetic construct
  REGION 1..39: note = Synthetic Construct
  SITE 2: note = MISC_FEATURE - Xaa at position 2 is Aib
  MOD_RES 17: note = Lys at position 17 is chemically modified by conjugation of the epsilon-amino group of the Lys side chain with (2-[2-(2-amino-ethoxy)-ethoxy]-acetyl)2-(gamma-Glu)-CO-(CH2)18-CO 2H
  MOD_RES 39: note = Ser at position 39 is amidated
YXEGTFTSDYSILLDEKAQKAFIEYLIEGGPSSGAPPPS

SEQ ID NO: 268 - protein, 39 aa, synthetic construct
  REGION 1..39: note = Synthetic Construct
  SITE 2: note = MISC_FEATURE - Xaa at position 2 is Aib
  MOD_RES 17: note = Lys at position 17 is chemically modified by conjugation of the epsilon-amino group of the Lys side chain with (2-[2-(2-amino-ethoxy)-ethoxy]-acetyl)2-(gamma-Glu)-CO-(CH2)18-CO 2H
  SITE 20: note = MISC_FEATURE - Xaa at position 20 is Aib
  MOD_RES 39: note = Ser at position 39 is amidated
YXEGTFTSDYSILLDEKAQXAFIEYLIEGGPSSGAPPPS

SEQ ID NO: 269 - protein, 39 aa, synthetic construct
  REGION 1..39: note = Synthetic Construct
  SITE 2: note = MISC_FEATURE - Xaa at position 2 is Aib
  MOD_RES 17: note = Lys at position 17 is chemically modified by conjugation of the epsilon-amino group of the Lys side chain with (2-[2-(2-amino-ethoxy)-ethoxy]-acetyl)2-(gamma-Glu)-CO-(CH2)18-CO 2H
  SITE 20: note = MISC_FEATURE - Xaa at position 20 is Aib
  SITE 39: note = MISC_FEATURE - Ser at position 39 is amidated
YXEGTFTSDHSILLDKKAQXAFIEYLIEGGPSSGAPPPS

SEQ ID NO: 270 - protein, 39 aa, synthetic construct
  REGION 1..39: note = Synthetic Construct
  SITE 2: note = MISC_FEATURE - Xaa at position 2 is Aib
  MOD_RES 17: note = Lys at position 17 is chemically modified by conjugation of the epsilon-amino group of the Lys side chain with (2-[2-(2-amino-ethoxy)-ethoxy]-acetyl)2-(gamma-Glu)-CO-(CH2)18-CO 2H
  MOD_RES 39: note = Ser at position 39 is amidated
YXEGTFTSDYSILLDKKAQEAFIEYLIEGGPSSGAPPPS

SEQ ID NO: 271 - protein, 39 aa, synthetic construct
  REGION 1..39: note = Synthetic Construct
  SITE 2: note = MISC_FEATURE - Xaa at position 2 is Aib
  MOD_RES 17: note = Lys at position 17 is chemically modified by conjugation of the epsilon-amino group of the Lys side chain with (2-[2-(2-amino-ethoxy)-ethoxy]-acetyl)2-(gamma-Glu)-CO-(CH2)18-CO 2H
  MOD_RES 39: note = Ser at position 39 is amidated
YXEGTFTSDYSILLDKKAQTAFIEYLIEGGPSSGAPPPS

SEQ ID NO: 272 - protein, 39 aa, synthetic construct
  REGION 1..39: note = Synthetic Construct
  SITE 2: note = MISC_FEATURE - Xaa at position 2 is Aib
  MOD_RES 17: note = Lys at position 17 is chemically modified by conjugation of the epsilon-amino group of the Lys side chain with (2-[2-(2-amino-ethoxy)-ethoxy]-acetyl)2-(gamma-Glu)-CO-(CH2)18-CO 2H
  MOD_RES 39: note = Ser at position 39 is amidated
YXEGTFTSDYSILLDKKAQSAFIEYLIEGGPSSGAPPPS

SEQ ID NO: 273 - protein, 34 aa, synthetic construct
  REGION 1..34: note = Synthetic Construct
  SITE 2: note = MISC_FEATURE - Xaa at position 2 is Aib
  SITE 6: note = MISC_FEATURE - Xaa at position 6 is alpha-methyl-Phe(2F)
  SITE 10: note = MISC_FEATURE - Xaa at position 10 is 4Pal
  SITE 13: note = MISC_FEATURE - Xaa at position 13 is alpha-methyl-Leu
  SITE 16: note = MISC_FEATURE - Xaa at position 16 is Orn
  MOD_RES 17: note = Lys at position 17 is chemically modified by conjugation of the epsilon-amino group of the Lys side chain with (2-[2-(2-amino-ethoxy)-ethoxy]-acetyl)2-(gamma-Glu)-CO-(CH2)16-CO 2H
  SITE 20: note = MISC_FEATURE - Xaa at position 20 is Aib
  SITE 24: note = MISC_FEATURE - Xaa at position 24 is D-Glu
  SITE 25: note = MISC_FEATURE - Xaa at position 25 is alpha-methyl-Tyr
  MOD_RES 34: note = Gly at position 34 is amidated
YXEGTXTSDXSIXLDXKAQXEFIXXLIEGGPSSG

SEQ ID NO: 274 - protein, 30 aa, synthetic construct
  REGION 1..30: note = Synthetic Construct
  SITE 2: note = MISC_FEATURE - Xaa at position 2 is Aib
  SITE 6: note = MISC_FEATURE - Xaa at position 6 is alpha-methyl-Phe(2F)
  SITE 10: note = MISC_FEATURE - Xaa at position 10 is 4Pal
  SITE 13: note = MISC_FEATURE - Xaa at position 13 is alpha-methyl-Leu
  SITE 16: note = MISC_FEATURE - Xaa at position 13 is Orn
  MOD_RES 17: note = Lys at position 17 is chemically modified by conjugation of the epsilon-amino group of the Lys side chain with (2-[2-(2-amino-ethoxy)-ethoxy]-acetyl)2-(gamma-Glu)-CO-(CH2)16-CO 2H
  SITE 20: note = MISC_FEATURE - Xaa at position 20 is Aib
  SITE 24: note = MISC_FEATURE - Xaa at position 24 is D-Glu
  SITE 25: note = MISC_FEATURE - Xaa at position 25 is alpha-methyl-Tyr
  MOD_RES 30: note = Gly at position 30 is amidated
YXEGTXTSDXSIXLDXKAQXEFIXXLIEGG

SEQ ID NO: 275 - protein, 34 aa, synthetic construct; identical to SEQ ID NO: 59
  REGION 1..34: note = Synthetic Construct
  SITE 2: note = MISC_FEATURE - Xaa at position 2 is Aib
  MOD_RES 17: note = Lys at position 17 is chemically modified by conjugation of the epsilon-amino group of the Lys side chain with (2-[2-(2-amino-ethoxy)-ethoxy]-acetyl)2-(gamma-Glu)-CO-(CH2)16-CO 2H
  SITE 20: note = MISC_FEATURE - Xaa at position 20 is Aib
  MOD_RES 34: note = Gly at position 34 is amidated

SEQ ID NO: 276 - protein, 30 aa, synthetic construct; identical to SEQ ID NO: 60
  REGION 1..30: note = Synthetic Construct
  SITE 2: note = MISC_FEATURE - Xaa at position 2 is Aib
  MOD_RES 17: note = Lys at position 17 is chemically modified by conjugation of the epsilon-amino group of the Lys side chain with (2-[2-(2-amino-ethoxy)-ethoxy]-acetyl)2-(gamma-Glu)-CO-(CH2)16-CO 2H
  SITE 20: note = MISC_FEATURE - Xaa at position 20 is Aib
  MOD_RES 30: note = Gly at position 30 is amidated

SEQ ID NO: 277 - protein, 34 aa, synthetic construct
  REGION 1..34: note = Synthetic Construct
  SITE 2: note = MISC_FEATURE - Xaa at position 2 is Aib
  MOD_RES 17: note = Lys at position 17 is chemically modified by conjugation of the epsilon-amino group of the Lys side chain with (2-[2-(2-amino-ethoxy)-ethoxy]-acetyl)2-(gamma-Glu)-CO-(CH2)16-CO 2H
  SITE 20: note = MISC_FEATURE - Xaa at position 20 is Aib
  MOD_RES 34: note = Gly at position 34 is amidated
YXEGTFTSDYSILLDEKAQXAFIEYLIEGGPSSG

SEQ ID NO: 278 - protein, 30 aa, synthetic construct
  REGION 1..30: note = Synthetic Construct
  SITE 2: note = MISC_FEATURE - Xaa at position 2 is Aib
  MOD_RES 17: note = Lys at position 17 is chemically modified by conjugation of the epsilon-amino group of the Lys side chain with (2-[2-(2-amino-ethoxy)-ethoxy]-acetyl)2-(gamma-Glu)-CO-(CH2)16-CO 2H
  SITE 20: note = MISC_FEATURE - Xaa at position 20 is Aib
  SITE 30: note = MISC_FEATURE - Gly at position 30 is amidated
YXEGTFTSDYSILLDEKAQXAFIEYLIEGG

SEQ ID NO: 279 - protein, 34 aa, synthetic construct
  REGION 1..34: note = Synthetic Construct
  SITE 2: note = MISC_FEATURE - Xaa at position 2 is Aib
  MOD_RES 17: note = Lys at position 17 is chemically modified by conjugation of the epsilon-amino group of the Lys side chain with (2-[2-(2-amino-ethoxy)-ethoxy]-acetyl)2-(gamma-Glu)-CO-(CH2)16-CO 2H
  SITE 20: note = MISC_FEATURE - Xaa at position 20 is Aib
  MOD_RES 34: note = Gly at position 34 is amidated
YXEGTFTSDYSILLDKKAQXEFIEYLIEGGPSSG

SEQ ID NO: 280 - protein, 30 aa, synthetic construct
  REGION 1..30: note = Synthetic Construct
  SITE 2: note = MISC_FEATURE - Xaa at position 2 is Aib
  MOD_RES 17: note = Lys at position 17 is chemically modified by conjugation of the epsilon-amino group of the Lys side chain with (2-[2-(2-amino-ethoxy)-ethoxy]-acetyl)2-(gamma-Glu)-CO-(CH2)16-CO 2H
  SITE 20: note = MISC_FEATURE - Xaa at position 20 is Aib
  MOD_RES 30: note = Gly at position 30 is amidated
YXEGTFTSDYSILLDKKAQXEFIEYLIEGG

SEQ ID NO: 281 - protein, 34 aa, synthetic construct
  REGION 1..34: note = Synthetic Construct
  SITE 2: note = MISC_FEATURE - Xaa at position 2 is Aib
  MOD_RES 17: note = Lys at position 17 is chemically modified by conjugation of the epsilon-amino group of the Lys side chain with (2-[2-(2-amino-ethoxy)-ethoxy]-acetyl)2-(gamma-Glu)-CO-(CH2)16-CO 2H
  SITE 20: note = MISC_FEATURE - Xaa at position 20 is Aib
  MOD_RES 34: note = Gly at position 34 is amidated
YXEGTFTSDYSILLDKKAQXAFIEYLIAGGPSSG

SEQ ID NO: 282 - protein, 30 aa, synthetic construct
  REGION 1..30: note = Synthetic Construct
  SITE 2: note = MISC_FEATURE - Xaa at position 2 is Aib
  MOD_RES 17: note = Lys at position 17 is chemically modified by conjugation of the epsilon-amino group of the Lys side chain with (2-[2-(2-amino-ethoxy)-ethoxy]-acetyl)2-(gamma-Glu)-CO-(CH2)16-CO 2H
  SITE 20: note = MISC_FEATURE - Xaa at position 20 is Aib
  MOD_RES 30: note = Gly at position 30 is amidated
YXEGTFTSDYSILLDKKAQXAFIEYLIAGG

SEQ ID NO: 283 - protein, 34 aa, synthetic construct
  REGION 1..34: note = Synthetic Construct
  SITE 2: note = MISC_FEATURE - Xaa at position 2 is Aib
  MOD_RES 17: note = Lys at position 17 is chemically modified by conjugation of the epsilon-amino group of the Lys side chain with (2-[2-(2-amino-ethoxy)-ethoxy]-acetyl)2-(gamma-Glu)-CO-(CH2)16-CO 2H
  MOD_RES 34: note = Gly at position 34 is amidated
YXEGTFTSDYSILLDKKAQPAFIEYLIEGGPSSG

SEQ ID NO: 284 - protein, 30 aa, synthetic construct
  REGION 1..30: note = Synthetic Construct
  SITE 2: note = MISC_FEATURE - Xaa at position 2 is Aib
  MOD_RES 17: note = Lys at position 17 is chemically modified by conjugation of the epsilon-amino group of the Lys side chain with (2-[2-(2-amino-ethoxy)-ethoxy]-acetyl)2-(gamma-Glu)-CO-(CH2)16-CO 2H
  MOD_RES 30: note = Gly at position 30 is amidated
YXEGTFTSDYSILLDKKAQPAFIEYLIEGG

SEQ ID NO: 285 - protein, 39 aa, synthetic construct; identical to SEQ ID NO: 10
  REGION 1..39: note = Synthetic Construct
  SITE 2: note = MISC_FEATURE - Xaa at position 2 is Aib
  SITE 6: note = MISC_FEATURE - Xaa at position 6 is alpha-methyl-Phe(2F)
  SITE 13: note = MISC_FEATURE - Xaa at position 13 is alpha-methyl-Leu
  SITE 20: note = MISC_FEATURE - Xaa at position 20 is Aib
  SITE 24: note = MISC_FEATURE - Xaa at position 24 is D-Glu
  MOD_RES 39: note = Ser at position 39 is amidated

SEQ ID NO: 286 - protein, 39 aa, synthetic construct
  REGION 1..39: note = Synthetic Construct
  SITE 2: note = MISC_FEATURE - Xaa at position 2 is Aib
  SITE 6: note = MISC_FEATURE - Xaa at position 6 is alpha-methyl-Phe(2F)
  SITE 13: note = MISC_FEATURE - Xaa at position 13 is alpha-methyl-Leu
  SITE 20: note = MISC_FEATURE - Xaa at position 20 is Aib
  SITE 24: note = MISC_FEATURE - Xaa at position 24 is D-Glu
  MOD_RES 39: note = Ser at position 39 is amidated
YXEGTXTSDYSIXLDEQAQXEFIXYLIEGGPSSGAPPPS

SEQ ID NO: 287 - protein, 40 aa, synthetic construct
  REGION 1..40: note = Synthetic Construct
  SITE 2: note = MISC_FEATURE - Xaa at position 2 is Aib
  SITE 6: note = MISC_FEATURE - Xaa at position 6 is alpha-methyl-Phe(2F)
  SITE 13: note = MISC_FEATURE - Xaa at position 13 is alpha-methyl-Leu
  SITE 20: note = MISC_FEATURE - Xaa at position 20 is Aib
  SITE 24: note = MISC_FEATURE - Xaa at position 24 is D-Glu
  MOD_RES 40: note = Cys at position 40 is amidated
YXEGTXTSDYSIXLDEKAQXEFIXYLIEGGPSSGAPPPSC

SEQ ID NO: 288 - protein, 40 aa, synthetic construct
  REGION 1..40: note = Synthetic Construct
  SITE 2: note = MISC_FEATURE - Xaa at position 2 is Aib
  SITE 6: note = MISC_FEATURE - Xaa at position 6 is alpha-methyl-Phe(2F)
  SITE 13: note = MISC_FEATURE - Xaa at position 13 is alpha-methyl-Leu
  SITE 20: note = MISC_FEATURE - Xaa at position 20 is Aib
  SITE 24: note = MISC_FEATURE - Xaa at position 24 is D-Glu
  MOD_RES 40: note = Cys at position 40 is amidated
YXEGTXTSDYSIXLDEQAQXEFIXYLIEGGPSSGAPPPSC

SEQ ID NO: 289 - protein, 39 aa, synthetic construct; identical to SEQ ID NO: 11
  REGION 1..39: note = Synthetic Construct
  SITE 2: note = MISC_FEATURE - Xaa at position 2 is Aib
  SITE 6: note = MISC_FEATURE - Xaa at position 6 is alpha-methyl-Phe(2F)
  SITE 13: note = MISC_FEATURE - Xaa at position 13 is alpha-methyl-Leu
  SITE 16: note = MISC_FEATURE - Xaa at position 16 is Orn
  SITE 20: note = MISC_FEATURE - Xaa at position 20 is Aib
  SITE 24: note = MISC_FEATURE - Xaa at position 24 is D-Glu
  MOD_RES 39: note = Ser at position 39 is amidated

SEQ ID NO: 290 - protein, 39 aa, synthetic construct
  REGION 1..39: note = Synthetic Construct
  SITE 2: note = MISC_FEATURE - Xaa at position 2 is Aib
  SITE 6: note = MISC_FEATURE - Xaa at position 6 is alpha-methyl-Phe(2F)
  SITE 13: note = MISC_FEATURE - Xaa at position 13 is alpha-methyl-Leu
  SITE 16: note = MISC_FEATURE - Xaa at position 16 is Orn
  SITE 20: note = MISC_FEATURE - Xaa at position 20 is Aib
  SITE 24: note = MISC_FEATURE - Xaa at position 24 is D-Glu
  MOD_RES 39: note = Ser at position 39 is amidated
YXEGTXTSDYSIXLDXQAQXEFIXYLIEGGPSSGAPPPS

SEQ ID NO: 291 - protein, 40 aa, synthetic construct
  REGION 1..40: note = Synthetic Construct
  SITE 2: note = MISC_FEATURE - Xaa at position 2 is Aib
  SITE 6: note = MISC_FEATURE - Xaa at position 6 is alpha-methyl-Phe(2F)
  SITE 13: note = MISC_FEATURE - Xaa at position 13 is alpha-methyl-Leu
  SITE 16: note = MISC_FEATURE - Xaa at position 16 is Orn
  SITE 20: note = MISC_FEATURE - Xaa at position 20 is Aib
  SITE 24: note = MISC_FEATURE - Xaa at position 24 is D-Glu
  MOD_RES 40: note = Cys at position 40 is amidated
YXEGTXTSDYSIXLDXKAQXEFIXYLIEGGPSSGAPPPSC

SEQ ID NO: 292 - protein, 40 aa, synthetic construct
  REGION 1..40: note = Synthetic Construct
  SITE 2: note = MISC_FEATURE - Xaa at position 2 is Aib
  SITE 6: note = MISC_FEATURE - Xaa at position 6 is alpha-methyl-Phe(2F)
  SITE 13: note = MISC_FEATURE - Xaa at position 13 is alpha-methyl-Leu
  SITE 16: note = MISC_FEATURE - Xaa at position 16 is Orn
  SITE 20: note = MISC_FEATURE - Xaa at position 20 is Aib
  SITE 24: note = MISC_FEATURE - Xaa at position 24 is D-Glu
  MOD_RES 40: note = Cys at position 40 is amidated
YXEGTXTSDYSIXLDXQAQXEFIXYLIEGGPSSGAPPPSC

SEQ ID NO: 293 - protein, 39 aa, synthetic construct; identical to SEQ ID NO: 13
  REGION 1..39: note = Synthetic Construct
  SITE 2: note = MISC_FEATURE - Xaa at position 2 is Aib
  SITE 6: note = MISC_FEATURE - Xaa at position 6 is alpha-methyl-Phe(2F)
  SITE 10: note = MISC_FEATURE - Xaa at position 10 is 4Pal
  SITE 13: note = MISC_FEATURE - Xaa at position 13 is alpha-methyl-Leu
  SITE 16: note = MISC_FEATURE - Xaa at position 16 is Orn
  SITE 20: note = MISC_FEATURE - Xaa at position 20 is Aib
  SITE 24: note = MISC_FEATURE - Xaa at position 24 is D-Glu
  SITE 25: note = MISC_FEATURE - Xaa at position 25 is alpha-methyl-Tyr
  MOD_RES 39: note = Ser at position 39 is amidated

SEQ ID NO: 294 - protein, 39 aa, synthetic construct
  REGION 1..39: note = Synthetic Construct
  SITE 2: note = MISC_FEATURE - Xaa at position 2 is Aib
  SITE 6: note = MISC_FEATURE - Xaa at position 6 is alpha-methyl-Phe(2F)
  SITE 10: note = MISC_FEATURE - Xaa at position 10 is 4Pal
  SITE 13: note = MISC_FEATURE - Xaa at position 13 is alpha-methyl-Leu
  SITE 16: note = MISC_FEATURE - Xaa at position 16 is Orn
  SITE 20: note = MISC_FEATURE - Xaa at position 20 is Aib
  SITE 24: note = MISC_FEATURE - Xaa at position 24 is D-Glu
  SITE 25: note = MISC_FEATURE - Xaa at position 25 is alpha-methyl-Tyr
  SITE 39: note = mod - Ser at position 39 is amidated
YXEGTXTSDXSIXLDXQAQXEFIXXLIEGGPSSGAPPPS

SEQ ID NO: 295 - protein, 40 aa, synthetic construct
  REGION 1..40: note = Synthetic Construct
  SITE 2: note = MISC_FEATURE - Xaa at position 2 is Aib
  SITE 6: note = MISC_FEATURE - Xaa at position 6 is alpha-methyl-Phe(2F)
  SITE 10: note = MISC_FEATURE - Xaa at position 10 is 4Pal
  SITE 13: note = MISC_FEATURE - Xaa at position 13 is alpha-methyl-Leu
  SITE 16: note = MISC_FEATURE - Xaa at position 16 is Orn
  SITE 20: note = MISC_FEATURE - Xaa at position 20 is Aib
  SITE 24: note = MISC_FEATURE - Xaa at position 24 is D-Glu
  SITE 25: note = MISC_FEATURE - Xaa at position 25 is alpha-methyl-Tyr
  MOD_RES 40: note = Cys at position 40 is amidated
YXEGTXTSDXSIXLDXKAQXEFIXXLIEGGPSSGAPPPSC

SEQ ID NO: 296 - protein, 40 aa, synthetic construct
  REGION 1..40: note = Synthetic Construct
  SITE 2: note = MISC_FEATURE - Xaa at position 2 is Aib
  SITE 6: note = MISC_FEATURE - Xaa at position 6 is alpha-methyl-Phe(2F)
  SITE 10: note = MISC_FEATURE - Xaa at position 10 is 4Pal
  SITE 13: note = MISC_FEATURE - Xaa at position 13 is alpha-methyl-Leu
  SITE 16: note = MISC_FEATURE - Xaa at position 16 is Orn
  SITE 20: note = MISC_FEATURE - Xaa at position 20 is Aib
  SITE 24: note = MISC_FEATURE - Xaa at position 24 is D-Glu
  SITE 25: note = MISC_FEATURE - Xaa at position 25 is alpha-methyl-Tyr
  MOD_RES 40: note = Cys at position 40 is amidated
YXEGTXTSDXSIXLDXQAQXEFIXXLIEGGPSSGAPPPSC

SEQ ID NO: 297 - protein, 4 aa, synthetic construct
  REGION 1..4: note = Synthetic Construct
  MOD_RES 4: note = The C-terminal Gly is modified with R2 to provide PSSG-R2, wherein the modification is NH2 or absent.
PSSG

SEQ ID NO: 298 - protein, 9 aa, synthetic construct
  REGION 1..9: note = Synthetic Construct
  MOD_RES 9: note = The C-terminal Ser is modified with R2 to provide PSSGAPPPS-R2, wherein the modification is NH2 or absent.
PSSGAPPPS

SEQ ID NO: 299 - protein, 4 aa, synthetic construct
  REGION 1..4: note = Synthetic Construct
PSSG

SEQ ID NO: 300 - protein, 4 aa, synthetic construct
  REGION 1..4: note = Synthetic Construct
  MOD_RES 4: note = Gly at position 4 is amidated
PSSG

SEQ ID NO: 301 - protein, 9 aa, synthetic construct
  REGION 1..9: note = Synthetic Construct
PSSGAPPPS

SEQ ID NO: 302 - protein, 9 aa, synthetic construct
  REGION 1..9: note = Synthetic Construct
  MOD_RES 9: note = Ser at position 9 is amidated
PSSGAPPPS

SEQ ID NO: 303 - protein, 39 aa, synthetic construct
  REGION 1..39: note = Synthetic Construct
  SITE 2: note = MISC_FEATURE - Xaa at position 2 is Aib
  MOD_RES 17: note = Lys at position 17 is chemically modified by conjugation of the epsilon-amino group of the Lys side chain with (2-[2-(2-amino-ethoxy)-ethoxy]-acetyl)2-(gamma-Glu)-CO-(CH2)18-CO 2H
  SITE 20: note = MISC_FEATURE - Xaa at position 20 is Aib
  MOD_RES 39: note = Ser at position 39 is amidated
YXEGTFTSDYSILLDKKAQXAFIEYLIAGGPSSGAPPPS

SEQ ID NO: 304 - protein, 39 aa, synthetic construct
  REGION 1..39: note = Synthetic Construct
  SITE 2: note = MISC_FEATURE - Xaa at position 2 is Aib
  SITE 13: note = MISC_FEATURE - Xaa at position 13 is alpha-methyl-Leu
  MOD_RES 17: note = Lys at position 17 is chemically modified by conjugation of the epsilon-amino group of the Lys side chain with (2-[2-(2-amino-ethoxy)-ethoxy]-acetyl)2-(gamma-Glu)-CO-(CH2)18-CO 2H
  SITE 20: note = MISC_FEATURE - Xaa at position 20 is Aib
  MOD_RES 39: note = Ser at position 39 is amidated
YXEGTFTSDYSIXLDKKAQXEFIEYLIAGGPSSGAPPPS

SEQ ID NO: 305 - protein, 39 aa, synthetic construct
  REGION 1..39: note = Synthetic Construct
  SITE 1: note = MISC_FEATURE - Xaa at position 1 is D-Tyr
  SITE 2: note = MISC_FEATURE - Xaa at position 2 is Aib
  SITE 13: note = MISC_FEATURE - Xaa at position 13 is alpha-methyl-Leu
  MOD_RES 17: note = Lys at position 17 is chemically modified by conjugation of the epsilon-amino group of the Lys side chain with (2-[2-(2-amino-ethoxy)-ethoxy]-acetyl)2-(gamma-Glu)-CO-(CH2)18-CO 2H
  SITE 20: note = MISC_FEATURE - Xaa at position 20 is Aib
  MOD_RES 39: note = Ser at position 39 is amidated
XXEGTFTSDYSIXLDKKAQXEFIEYLIAGGPSSGAPPPS

SEQ ID NO: 306 - protein, 39 aa, synthetic construct
  REGION 1..39: note = Synthetic Construct
  SITE 1: note = MISC_FEATURE - Xaa at position 1 is D-Tyr
  SITE 2: note = MISC_FEATURE - Xaa at position 2 is Aib
  SITE 13: note = MISC_FEATURE - Xaa at position 13 is alpha-methyl-Leu
  SITE 16: note = MISC_FEATURE - Xaa at position 16 is Orn
  MOD_RES 17: note = Lys at position 17 is chemically modified by conjugation of the epsilon-amino group of the Lys side chain with (2-[2-(2-amino-ethoxy)-ethoxy]-acetyl)2-(gamma-Glu)-CO-(CH2)18-CO 2H
  SITE 20: note = MISC_FEATURE - Xaa at position 20 is Aib
  SITE 24: note = MISC_FEATURE - Xaa at position 24 is D-Glu
  MOD_RES 39: note = Ser at position 39 is amidated
XXEGTFTSDYSIXLDXKAQXAFIXYLIAGGPSSGAPPPS

SEQ ID NO: 307 - protein, 39 aa, synthetic construct
  REGION 1..39: note = Synthetic Construct
  SITE 1: note = MISC_FEATURE - Xaa at position 1 is D-Tyr
  SITE 2: note = MISC_FEATURE - Xaa at position 2 is Aib
  SITE 13: note = MISC_FEATURE - Xaa at position 13 is alpha-methyl-Leu
  MOD_RES 17: note = Lys at position 17 is chemically modified by conjugation of the epsilon-amino group of the Lys side chain with (2-[2-(2-amino-ethoxy)-ethoxy]-acetyl)2-(gamma-Glu)-CO-(CH2)18-CO 2H
  SITE 20: note = MISC_FEATURE - Xaa at position 20 is Aib
  SITE 25: note = MISC_FEATURE - Xaa at position 25 is alpha-methyl-Tyr
  MOD_RES 39: note = Ser at position 39 is amidated
XXEGTFTSDYSIXLDKKAQXEFIEXLIAGGPSSGAPPPS

SEQ ID NO: 308 - protein, 39 aa, synthetic construct
  REGION 1..39: note = Synthetic Construct
  SITE 1: note = MISC_FEATURE - Xaa at position 1 is D-Tyr
  SITE 2: note = MISC_FEATURE - Xaa at position 2 is Aib
  SITE 13: note = MISC_FEATURE - Xaa at position 13 is alpha-methyl-Leu
  SITE 16: note = MISC_FEATURE - Xaa at position 16 is Orn
  MOD_RES 17: note = Lys at position 17 is chemically modified by conjugation of the epsilon-amino group of the Lys side chain with (2-[2-(2-amino-ethoxy)-ethoxy]-acetyl)2-(gamma-Glu)-CO-(CH2)18-CO 2H
  SITE 20: note = MISC_FEATURE - Xaa at position 20 is Aib
  SITE 25: note = MISC_FEATURE - Xaa at position 25 is alpha-methyl-Tyr
  MOD_RES 39: note = Ser at position 39 is amidated
XXEGTFTSDYSIXLDXKAQXEFIEXLIAGGPSSGAPPPS

SEQ ID NO: 309 - protein, 30 aa, synthetic construct
  REGION 1..30: note = Synthetic Construct
  SITE 2: note = MISC_FEATURE - Xaa at position 2 is Aib
  MOD_RES 17: note = Lys at position 17 is chemically modified by conjugation of the epsilon-amino group of the Lys side chain with (2-[2-(2-amino-ethoxy)-ethoxy]-acetyl)2-(gamma-Glu)-CO-(CH2)16-CO 2H
  MOD_RES 30: note = Gly at position 30 is amidated
YXEGTFTSDYSILLDKKAQQAFIEYLIEGG

SEQ ID NO: 310 - protein, 30 aa, synthetic construct
  REGION 1..30: note = Synthetic Construct
  SITE 2: note = MISC_FEATURE - Xaa at position 2 is Aib
  MOD_RES 17: note = Lys at position 17 is chemically modified by conjugation of the epsilon-amino group of the Lys side chain with (2-[2-(2-amino-ethoxy)-ethoxy]-acetyl)2-(gamma-Glu)-CO-(CH2)16-CO 2H
  MOD_RES 30: note = Gly at position 30 is amidated
YXEGTFTSDYSILLDKKAQHAFIEYLIEGG

SEQ ID NO: 311 - protein, 34 aa, synthetic construct
  REGION 1..34: note = Synthetic Construct
  SITE 2: note = MISC_FEATURE - Xaa at position 2 is Aib
  MOD_RES 17: note = Lys at position 17 is chemically modified by conjugation of the epsilon-amino group of the Lys side chain with (2-[2-(2-amino-ethoxy)-ethoxy]-acetyl)2-(gamma-Glu)-CO-(CH2)16-CO 2H
  MOD_RES 34: note = Gly at position 34 is amidated
YXEGTFTSDYSILLDKKAQKAFIEYLIEGGPSSG

SEQ ID NO: 312 - protein, 30 aa, synthetic construct
  REGION 1..30: note = Synthetic Construct
  SITE 2: note = MISC_FEATURE - Xaa at position 2 is Aib
  MOD_RES 17: note = Lys at position 17 is chemically modified by conjugation of the epsilon-amino group of the Lys side chain with (2-[2-(2-amino-ethoxy)-ethoxy]-acetyl)2-(gamma-Glu)-CO-(CH2)16-CO 2H
  SITE 20: note = MISC_FEATURE - Xaa at position 20 is Aib
  MOD_RES 30: note = Gly at position 30 is amidated
YXEGTFTSDYSILLDKKAQXEFIEYLIAGG

SEQ ID NO: 313 - protein, 34 aa, synthetic construct
  REGION 1..34: note = Synthetic Construct
  SITE 2: note = MISC_FEATURE - Xaa at position 2 is Aib
  MOD_RES 17: note = Lys at position 17 is chemically modified by conjugation of the epsilon-amino group of the Lys side chain with (2-[2-(2-amino-ethoxy)-ethoxy]-acetyl)2-(gamma-Glu)-CO-(CH2)16-CO 2H
  SITE 20: note = MISC_FEATURE - Xaa at position 20 is Aib
  MOD_RES 34: note = Gly at position 34 is amidated
YXEGTFTSDYSILLDKKAQXAFVEYLIEGGPSSG

SEQ ID NO: 314 - protein, 34 aa, synthetic construct
  REGION 1..34: note = Synthetic Construct
  SITE 2: note = MISC_FEATURE - Xaa at position 2 is Aib
  MOD_RES 17: note = Lys at position 17 is chemically modified by conjugation of the epsilon-amino group of the Lys side chain with (2-[2-(2-amino-ethoxy)-ethoxy]-acetyl)2-(gamma-Glu)-CO-(CH2)16-CO 2H
  SITE 20: note = MISC_FEATURE - Xaa at position 20 is Aib
  MOD_RES 34: note = Gly at position 34 is amidated
YXEGTFTSDYSILLDKKAQXAFLEYLIEGGPSSG

SEQ ID NO: 315 - protein, 34 aa, synthetic construct
  REGION 1..34: note = Synthetic Construct
  SITE 2: note = MISC_FEATURE - Xaa at position 2 is Aib
  SITE 13: note = MISC_FEATURE - Xaa at position 13 is alpha-methyl-Leu
  MOD_RES 17: note = Lys at position 17 is chemically modified by conjugation of the epsilon-amino group of the Lys side chain with (2-[2-(2-amino-ethoxy)-ethoxy]-acetyl)2-(gamma-Glu)-CO-(CH2)16-CO 2H
  SITE 20: note = MISC_FEATURE - Xaa at position 20 is Aib
  MOD_RES 34: note = Gly at position 34 is amidated
YXEGTFTSDYSIXLDKKAQXAFIEYLIEGGPSSG

SEQ ID NO: 316 - protein, 34 aa, synthetic construct
  REGION 1..34: note = Synthetic Construct
  SITE 2: note = MISC_FEATURE - Xaa at position 2 is Aib
  SITE 6: note = MISC_FEATURE - Xaa at position 6 is alpha-methyl-Phe
  MOD_RES 17: note = Lys at position 17 is chemically modified by conjugation of the epsilon-amino group of the Lys side chain with (2-[2-(2-amino-ethoxy)-ethoxy]-acetyl)2-(gamma-Glu)-CO-(CH2)16-CO 2H
  SITE 20: note = MISC_FEATURE - Xaa at position 20 is Aib
  MOD_RES 34: note = Gly at position 34 is amidated
YXEGTXTSDYSILLDKKAQXAFIEYLIEGGPSSG

SEQ ID NO: 317 - protein, 34 aa, synthetic construct; identical to SEQ ID NO: 316
  REGION 1..34: note = Synthetic Construct
  SITE 2: note = MISC_FEATURE - Xaa at position 2 is Aib
  SITE 6: note = MISC_FEATURE - Xaa at position 6 is alpha-methyl-Phe(2F)
  MOD_RES 17: note = Lys at position 17 is chemically modified by conjugation of the epsilon-amino group of the Lys side chain with (2-[2-(2-amino-ethoxy)-ethoxy]-acetyl)2-(gamma-Glu)-CO-(CH2)16-CO 2H
  SITE 20: note = MISC_FEATURE - Xaa at position 20 is Aib
  MOD_RES 34: note = Gly at position 34 is amidated

SEQ ID NO: 318 - protein, 34 aa, synthetic construct
  REGION 1..34: note = Synthetic Construct
  SITE 2: note = MISC_FEATURE - Xaa at position 2 is Aib
  SITE 13: note = MISC_FEATURE - Xaa at position 13 is alpha-methyl-Leu
  MOD_RES 17: note = Lys at position 17 is chemically modified by conjugation of the epsilon-amino group of the Lys side chain with (2-[2-(2-amino-ethoxy)-ethoxy]-acetyl)2-(gamma-Glu)-CO-(CH2)16-CO 2H
  SITE 20: note = MISC_FEATURE - Xaa at position 20 is Aib
  MOD_RES 34: note = Gly at position 34 is amidated
YXEGTFTSDYSIXLDEKAQXAFIEYLIEGGPSSG

SEQ ID NO: 319 - protein, 34 aa, synthetic construct
  REGION 1..34: note = Synthetic Construct
  SITE 2: note = MISC_FEATURE - Xaa at position 2 is Aib
  SITE 13: note = MISC_FEATURE - Xaa at position 13 is alpha-methyl-Leu
  MOD_RES 17: note = Lys at position 17 is chemically modified by conjugation of the epsilon-amino group of the Lys side chain with (2-[2-(2-amino-ethoxy)-ethoxy]-acetyl)2-(gamma-Glu)-CO-(CH2)16-CO 2H
  SITE 20: note = MISC_FEATURE - Xaa at position 20 is Aib
  MOD_RES 34: note = Gly at position 34 is amidated
YXEGTFTSDYSIXLDKKAQXEFIEYLIEGGPSSG

SEQ ID NO: 320 - protein, 34 aa, synthetic construct
  REGION 1..34: note = Synthetic Construct
  SITE 2: note = MISC_FEATURE - Xaa at position 2 is Aib
  SITE 13: note = MISC_FEATURE - Xaa at position 13 is alpha-methyl-Leu
  MOD_RES 17: note = Lys at position 17 is chemically modified by conjugation of the epsilon-amino group of the Lys side chain with (2-[2-(2-amino-ethoxy)-ethoxy]-acetyl)2-(gamma-Glu)-CO-(CH2)16-CO 2H
  SITE 20: note = MISC_FEATURE - Xaa at position 20 is Aib
  MOD_RES 34: note = Gly at position 34 is amidated
YXEGTFTSDYSIXLDKKAQXAFIEYLIAGGPSSG

SEQ ID NO: 321 - protein, 34 aa, synthetic construct
  REGION 1..34: note = Synthetic Construct
  SITE 2: note = MISC_FEATURE - Xaa at position 2 is Aib
  SITE 13: note = MISC_FEATURE - Xaa at position 13 is alpha-methyl-Leu
  MOD_RES 17: note = Lys at position 17 is chemically modified by conjugation of the epsilon-amino group of the Lys side chain with (2-[2-(2-amino-ethoxy)-ethoxy]-acetyl)2-(gamma-Glu)-CO-(CH2)16-CO 2H
  SITE 20: note = MISC_FEATURE - Xaa at position 20 is Aib
  MOD_RES 34: note = Gly at position 34 is amidated
YXEGTFTSDYSIXLDKKAQXEFIEYLIAGGPSSG

SEQ ID NO: 322 - protein, 34 aa, synthetic construct
  REGION 1..34: note = Synthetic Construct
  SITE 2: note = MISC_FEATURE - Xaa at position 2 is Aib
  SITE 6: note = MISC_FEATURE - Xaa at position 6 is alpha-methyl-Phe
  MOD_RES 17: note = Lys at position 17 is chemically modified by conjugation of the epsilon-amino group of the Lys side chain with (2-[2-(2-amino-ethoxy)-ethoxy]-acetyl)2-(gamma-Glu)-CO-(CH2)16-CO 2H
  SITE 20: note = MISC_FEATURE - Xaa at position 20 is Aib
  MOD_RES 34: note = Gly at position 34 is amidated
YXEGTXTSDYSILLDEKAQXAFIEYLIEGGPSSG

SEQ ID NO: 323 - protein, 34 aa, synthetic construct
  REGION 1..34: note = Synthetic Construct
  SITE 2: note = MISC_FEATURE - Xaa at position 2 is Aib
  SITE 6: note = MISC_FEATURE - Xaa at position 6 is alpha-methyl-Phe
  MOD_RES 17: note = Lys at position 17 is chemically modified by conjugation of the epsilon-amino group of the Lys side chain with (2-[2-(2-amino-ethoxy)-ethoxy]-acetyl)2-(gamma-Glu)-CO-(CH2)16-CO 2H
  SITE 20: note = MISC_FEATURE - Xaa at position 20 is Aib
  MOD_RES 34: note = Gly at position 34 is amidated
YXEGTXTSDYSILLDKKAQXEFIEYLIEGGPSSG

SEQ ID NO: 324 - protein, 34 aa, synthetic construct
  REGION 1..34: note = Synthetic Construct
  SITE 2: note = MISC_FEATURE - Xaa at position 2 is Aib
  SITE 6: note = MISC_FEATURE - Xaa at position 6 is alpha-methyl-Phe
  MOD_RES 17: note = Lys at position 17 is chemically modified by conjugation of the epsilon-amino group of the Lys side chain with (2-[2-(2-amino-ethoxy)-ethoxy]-acetyl)2-(gamma-Glu)-CO-(CH2)16-CO 2H
  SITE 20: note = MISC_FEATURE - Xaa at position 20 is Aib
  MOD_RES 34: note = Gly at position 34 is amidated
YXEGTXTSDYSILLDKKAQXAFIEYLIAGGPSSG

SEQ ID NO: 325 - protein, 34 aa, synthetic construct
  REGION 1..34: note = Synthetic Construct
  SITE 2: note = MISC_FEATURE - Xaa at position 2 is Aib
  SITE 6: note = MISC_FEATURE - Xaa at position 6 is alpha-methyl-Phe
  MOD_RES 17: note = Lys at position 17 is chemically modified by conjugation of the epsilon-amino group of the Lys side chain with (2-[2-(2-amino-ethoxy)-ethoxy]-acetyl)2-(gamma-Glu)-CO-(CH2)16-CO 2H
  SITE 20: note = MISC_FEATURE - Xaa at position 20 is Aib
  MOD_RES 34: note = Gly at position 34 is amidated
YXEGTXTSDYSILLDKKAQXEFIEYLIAGGPSSG

SEQ ID NO: 326 - protein, 34 aa, synthetic construct; identical to SEQ ID NO: 322
  REGION 1..34: note = Synthetic Construct
  SITE 2: note = MISC_FEATURE - Xaa at position 2 is Aib
  SITE 6: note = MISC_FEATURE - Xaa at position 6 is alpha-methyl-Phe(2F)
  MOD_RES 17: note = Lys at position 17 is chemically modified by conjugation of the epsilon-amino group of the Lys side chain with (2-[2-(2-amino-ethoxy)-ethoxy]-acetyl)2-(gamma-Glu)-CO-(CH2)16-CO 2H
  SITE 20: note = MISC_FEATURE - Xaa at position 20 is Aib
  MOD_RES 34: note = Gly at position 34 is amidated

SEQ ID NO: 327 - protein, 34 aa, synthetic construct; identical to SEQ ID NO: 323
  REGION 1..34: note = Synthetic Construct
  SITE 2: note = MISC_FEATURE - Xaa at position 2 is Aib
  SITE 6: note = MISC_FEATURE - Xaa at position 6 is alpha-methyl-Phe(2F)
  MOD_RES 17: note = Lys at position 17 is chemically modified by conjugation of the epsilon-amino group of the Lys side chain with (2-[2-(2-amino-ethoxy)-ethoxy]-acetyl)2-(gamma-Glu)-CO-(CH2)16-CO 2H
  SITE 20: note = MISC_FEATURE - Xaa at position 20 is Aib
  MOD_RES 34: note = Gly at position 34 is amidated

SEQ ID NO: 328 - protein, 34 aa, synthetic construct; identical to SEQ ID NO: 324
  REGION 1..34: note = Synthetic Construct
  SITE 2: note = MISC_FEATURE - Xaa at position 2 is Aib
  SITE 6: note = MISC_FEATURE - Xaa at position 6 is alpha-methyl-Phe(2F)
  MOD_RES 17: note = Lys at position 17 is chemically modified by conjugation of the epsilon-amino group of the Lys side chain with (2-[2-(2-amino-ethoxy)-ethoxy]-acetyl)2-(gamma-Glu)-CO-(CH2)16-CO 2H
  SITE 20: note = MISC_FEATURE - Xaa at position 20 is Aib
  MOD_RES 34: note = Gly at position 34 is amidated

SEQ ID NO: 329 - protein, 34 aa, synthetic construct; identical to SEQ ID NO: 325
  REGION 1..34: note = Synthetic Construct
  SITE 2: note = MISC_FEATURE - Xaa at position 2 is Aib
  SITE 6: note = MISC_FEATURE - Xaa at position 6 is alpha-methyl-Phe(2F)
  MOD_RES 17: note = Lys at position 17 is chemically modified by conjugation of the epsilon-amino group of the Lys side chain with (2-[2-(2-amino-ethoxy)-ethoxy]-acetyl)2-(gamma-Glu)-CO-(CH2)16-CO 2H
  SITE 20: note = MISC_FEATURE - Xaa at position 20 is Aib
  MOD_RES 34: note = Gly at position 34 is amidated

SEQ ID NO: 330 - protein, 39 aa, synthetic construct; identical to SEQ ID NO: 17
  REGION 1..39: note = Synthetic Construct
  SITE 2: note = MISC_FEATURE - Xaa at position 2 is Aib
  MOD_RES 17: note = Lys at position 17 is chemically modified by conjugation of the epsilon-amino group of the Lys side chain with (2-[2-(2-amino-ethoxy)-ethoxy]-acetyl)2-(gamma-Glu)-CO-(CH2)16-CO 2H
  SITE 20: note = MISC_FEATURE - Xaa at position 20 is Aib
  MOD_RES 39: note = Ser at position 39 is amidated

SEQ ID NO: 331 - protein, 39 aa, synthetic construct; identical to SEQ ID NO: 303
  REGION 1..39: note = Synthetic Construct
  SITE 2: note = MISC_FEATURE - Xaa at position 2 is Aib
  MOD_RES 17: note = Lys at position 17 is chemically modified by conjugation of the epsilon-amino group of the Lys side chain with (2-[2-(2-amino-ethoxy)-ethoxy]-acetyl)2-(gamma-Glu)-CO-(CH2)16-CO 2H
  SITE 20: note = MISC_FEATURE - Xaa at position 20 is Aib
  MOD_RES 39: note = Ser at position 39 is amidated

SEQ ID NO: 332 - protein, 34 aa, synthetic construct; identical to SEQ ID NO: 281
  REGION 1..34: note = Synthetic Construct
  SITE 2: note = MISC_FEATURE - Xaa at position 2 is Aib
  MOD_RES 17: note = Lys at position 17 is chemically modified by conjugation of the epsilon-amino group of the Lys side chain with (2-[2-(2-amino-ethoxy)-ethoxy]-acetyl)2-(gamma-Glu)-CO-(CH2)18-CO 2H
  SITE 20: note = MISC_FEATURE - Xaa at position 20 is Aib
  MOD_RES 34: note = Gly at position 34 is amidated

SEQ ID NO: 333 - protein, 34 aa, synthetic construct
  REGION 1..34: note = Synthetic Construct
  SITE 2: note = MISC_FEATURE - Xaa at position 2 is Aib
  MOD_RES 17: note = Lys at position 17 is chemically modified by conjugation of the epsilon-amino group of the Lys side chain with (2-[2-(2-amino-ethoxy)-ethoxy]-acetyl)2-(gamma-Glu)-CO-(CH2)18-CO 2H
  SITE 20: note = MISC_FEATURE - Xaa at position 20 is Aib
  MOD_RES 34: note = Gly at position 34 is amidated
YXEGTFTSDYSILLDKKAQXEFIEYLIAGGPSSG

SEQ ID NO: 334 - protein, 39 aa, synthetic construct
  REGION 1..39: note = Synthetic Construct
  SITE 2: note = MISC_FEATURE - Xaa at position 2 is Aib
  MOD_RES 17: note = Lys at position 17 is chemically modified by conjugation of the epsilon-amino group of the Lys side chain with (2-[2-(2-amino-ethoxy)-ethoxy]-acetyl)2-(gamma-Glu)-CO-(CH2)18-CO 2H
  SITE 20: note = MISC_FEATURE - Xaa at position 20 is Aib
  MOD_RES 39: note = Ser at position 39 is amidated
YXEGTFTSDYSILLDKKAQXEFIEYLIAGGPSSGAPPPS

SEQ ID NO: 335 - protein, 34 aa, synthetic construct
  REGION 1..34: note = Synthetic Construct
  SITE 2: note = MISC_FEATURE - Xaa at position 2 is Aib
  MOD_RES 17: note = Lys at position 17 is chemically modified by conjugation of the epsilon-amino group of the Lys side chain with (2-[2-(2-amino-ethoxy)-ethoxy]-acetyl)2-(gamma-Glu)-CO-(CH2)16-CO 2H
  SITE 20: note = MISC_FEATURE - Xaa at position 20 is Aib
  MOD_RES 34: note = Gly at position 34 is amidated
YXEGTFTSDYSILLDKKAQXDFIEYLIEGGPSSG

SEQ ID NO: 336 - protein, 34 aa, synthetic construct
  REGION 1..34: note = Synthetic Construct
  SITE 2: note = MISC_FEATURE - Xaa at position 2 is Aib
  MOD_RES 17: note = Lys at position 17 is chemically modified by conjugation of the epsilon-amino group of the Lys side chain with (2-[2-(2-amino-ethoxy)-ethoxy]-acetyl)2-(gamma-Glu)-CO-(CH2)16-CO 2H
  SITE 20: note = MISC_FEATURE - Xaa at position 20 is Aib
  MOD_RES 34: note = Gly at position 34 is amidated
YXEGTFTSDYSILLDKKAQXTFIEYLIEGGPSSG

SEQ ID NO: 337 - protein, 34 aa, synthetic construct
  REGION 1..34: note = Synthetic Construct
  SITE 2: note = MISC_FEATURE - Xaa at position 2 is Aib
  MOD_RES 17: note = Lys at position 17 is chemically modified by conjugation of the epsilon-amino group of the Lys side chain with (2-[2-(2-amino-ethoxy)-ethoxy]-acetyl)2-(gamma-Glu)-CO-(CH2)16-CO 2H
  SITE 20: note = MISC_FEATURE - Xaa at position 20 is Aib
  MOD_RES 34: note = Gly at position 34 is amidated
YXEGTFTSDYSILLDKKAQXHFIEYLIEGGPSSG

SEQ ID NO: 338 - protein, 39 aa, synthetic construct; identical to SEQ ID NO: 68
  REGION 1..39: note = Synthetic Construct
  SITE 2: note = MISC_FEATURE - Xaa at position 2 is Aib
  SITE 13: note = MISC_FEATURE - Xaa at position 13 is alpha-methyl-Leu
  MOD_RES 17: note = Lys at position 17 is chemically modified by conjugation of the epsilon-amino group of the Lys side chain with (2-[2-(2-amino-ethoxy)-ethoxy]-acetyl)2-(gamma-Glu)-CO-(CH2)16-CO 2H
  SITE 20: note = MISC_FEATURE - Xaa at position 20 is Aib
  MOD_RES 39: note = Ser at position 39 is amidated

SEQ ID NO: 339 - protein, 39 aa, synthetic construct
  REGION 1..39: note = Synthetic Construct
  SITE 2: note = MISC_FEATURE - Xaa at position 2 is Aib
  SITE 13: note = MISC_FEATURE - Xaa at position 13 is alpha-methyl-Leu
  MOD_RES 17: note = Lys at position 17 is chemically modified by conjugation of the epsilon-amino group of the Lys side chain with (2-[2-(2-amino-ethoxy)-ethoxy]-acetyl)2-(gamma-Glu)-CO-(CH2)18-CO 2H
  SITE 20: note = MISC_FEATURE - Xaa at position 20 is Aib
  MOD_RES 39: note = Ser at position 39 is amidated
YXEGTFTSDYSIXLDKKAQXAFIEYLIAGGPSSGAPPPS

SEQ ID NO: 340 - protein, 39 aa, synthetic construct; identical to SEQ ID NO: 66
  REGION 1..39: note = Synthetic Construct
  SITE 2: note = MISC_FEATURE - Xaa at position 2 is Aib
  SITE 6: note = MISC_FEATURE - Xaa at position 6 is alpha-methyl-Phe(2F)
  MOD_RES 17: note = Lys at position 17 is chemically modified by conjugation of the epsilon-amino group of the Lys side chain with (2-[2-(2-amino-ethoxy)-ethoxy]-acetyl)2-(gamma-Glu)-CO-(CH2)18-CO 2H
  SITE 20: note = MISC_FEATURE - Xaa at position 20 is Aib
  MOD_RES 39: note = Ser at position 39 is amidated

SEQ ID NO: 341 - protein, 39 aa, synthetic construct
  REGION 1..39: note = Synthetic Construct
  SITE 2: note = MISC_FEATURE - Xaa at position 2 is Aib
  MOD_RES 17: note = Lys at position 17 is chemically modified by conjugation of the epsilon-amino group of the Lys side chain with (2-[2-(2-amino-ethoxy)-ethoxy]-acetyl)2-(gamma-Glu)-CO-(CH2)18-CO 2H
  SITE 20: note = MISC_FEATURE - Xaa at position 20 is Aib
  MOD_RES 39: note = Ser at position 39 is amidated
FXEGTFTSDYSILLDKKAQXAFIEYLIEGGPSSGAPPPS

SEQ ID NO: 342 - protein, 39 aa, synthetic construct
  REGION 1..39: note = Synthetic Construct
  SITE 2: note = MISC_FEATURE - Xaa at position 2 is Aib
  SITE 13: note = MISC_FEATURE - Xaa at position 13 is alpha-methyl-Leu
  MOD_RES 17: note = Lys at position 17 is chemically modified by conjugation of the epsilon-amino group of the Lys side chain with (2-[2-(2-amino-ethoxy)-ethoxy]-acetyl)2-(gamma-Glu)-CO-(CH2)18-CO 2H
  SITE 20: note = MISC_FEATURE - Xaa at position 20 is Aib
  MOD_RES 39: note = Ser at position 39 is amidated
FXEGTFTSDYSIXLDKKAQXAFIEYLIEGGPSSGAPPPS

SEQ ID NO: 343 - protein, 39 aa, synthetic construct
  REGION 1..39: note = Synthetic Construct
  SITE 2: note = MISC_FEATURE - Xaa at position 2 is Aib
  SITE 13: note = MISC_FEATURE - Xaa at position 13 is alpha-methyl-Leu
  MOD_RES 17: note = Lys at position 17 is chemically modified by conjugation of the epsilon-amino group of the Lys side chain with (2-[2-(2-amino-ethoxy)-ethoxy]-acetyl)2-(gamma-Glu)-CO-(CH2)16-CO 2H
  SITE 20: note = MISC_FEATURE - Xaa at position 20 is Aib
  MOD_RES 39: note = Ser at position 39 is amidated
FXEGTFTSDYSIXLDKKAQXAFIEYLIEAGPSSGAPPPS

SEQ ID NO: 344 - protein, 39 aa, synthetic construct
  REGION 1..39: note = Synthetic Construct
  SITE 1: note = MISC_FEATURE - Xaa at position 1 is D-Tyr
  SITE 2: note = MISC_FEATURE - Xaa at position 2 is Aib
  SITE 6: note = MISC_FEATURE - Xaa at position 6 is alpha-methyl-Phe
  MOD_RES 17: note = Lys at position 17 is chemically modified by conjugation of the epsilon-amino group of the Lys side chain with (2-[2-(2-amino-ethoxy)-ethoxy]-acetyl)2-(gamma-Glu)-CO-(CH2)18-CO 2H
  SITE 20: note = MISC_FEATURE - Xaa at position 20 is Aib
  MOD_RES 39: note = Ser at position 39 is amidated
XXEGTXTSDYSILLDKKAQXAFIEYLIEGGPSSGAPPPS

SEQ ID NO: 345 - protein, 39 aa, synthetic construct
  REGION 1..39: note = Synthetic Construct
  SITE 2: note = MISC_FEATURE - Xaa at position 2 is Aib
  MOD_RES 17: note = Lys at position 17 is chemically modified by conjugation of the epsilon-amino group of the Lys side chain with (2-[2-(2-amino-ethoxy)-ethoxy]-acetyl)2-(gamma-Glu)-CO-(CH2)18-CO 2H
  SITE 20: note = MISC_FEATURE - Xaa at position 20 is Aib
  MOD_RES 39: note = Ser at position 39 is amidated
YXEGTFTSDYSILLDEKAQXAFIEYLIAGGPSSGAPPPS

SEQ ID NO: 346 - protein, 39 aa, synthetic construct
  REGION 1..39: note = Synthetic Construct
  SITE 2: note = MISC_FEATURE - Xaa at position 2 is Aib
  SITE 13: note = MISC_FEATURE - Xaa at position 13 is alpha-methyl-Leu
  MOD_RES 17: note = Lys at position 17 is chemically modified by conjugation of the epsilon-amino group of the Lys side chain with (2-[2-(2-amino-ethoxy)-ethoxy]-acetyl)2-(gamma-Glu)-CO-(CH2)18-CO 2H
  SITE 20: note = MISC_FEATURE - Xaa at position 20 is Aib
  MOD_RES 39: note = Ser at position 39 is amidated
YXEGTFTSDYSIXLDEKAQXEFIEYLIAGGPSSGAPPPS

SEQ ID NO: 347 - protein, 39 aa, synthetic construct
  REGION 1..39: note = Synthetic Construct
  SITE 2: note = MISC_FEATURE - Xaa at position 2 is Aib
  SITE 13: note = MISC_FEATURE - Xaa at position 13 is alpha-methyl-Leu
  MOD_RES 17: note = Lys at position 17 is chemically modified by conjugation of the epsilon-amino group of the Lys side chain with (2-[2-(2-amino-ethoxy)-ethoxy]-acetyl)2-(gamma-Glu)-CO-(CH2)18-CO 2H
  SITE 20: note = MISC_FEATURE - Xaa at position 2 is Aib
  MOD_RES 39: note = Ser at position 39 is amidated
YXEGTFTSDYSIXLDEKAQXAFIEYLIAGGPSSGAPPPS

SEQ ID NO: 348 - protein, 39 aa, synthetic construct
  REGION 1..39: note = Synthetic Construct
  SITE 2: note = MISC_FEATURE - Xaa at position 2 is Aib
  SITE 13: note = MISC_FEATURE - Xaa at position 13 is alpha-methyl-Leu
  MOD_RES 17: note = Lys at position 17 is chemically modified by conjugation of the epsilon-amino group of the Lys side chain with (2-[2-(2-amino-ethoxy)-ethoxy]-acetyl)2-(gamma-Glu)-CO-(CH2)18-CO 2H
  SITE 20: note = MISC_FEATURE - Xaa at position 20 is Aib
  MOD_RES 39: note = Ser at position 39 is amidated
YXEGTFTSDYSIXLDKKAQXEFIEYLIEGGPSSGAPPPS

SEQ ID NO: 349 - protein, 39 aa, synthetic construct
  REGION 1..39: note = Synthetic Construct
  SITE 1: note = MISC_FEATURE - Xaa at position 1 is D-Tyr
  SITE 2: note = MISC_FEATURE - Xaa at position 2 is Aib
  SITE 13: note = MISC_FEATURE - Xaa at position 13 is alpha-methyl-Leu
  MOD_RES 17: note = Lys at position 17 is chemically modified by conjugation of the epsilon-amino group of the Lys side chain with (2-[2-(2-amino-ethoxy)-ethoxy]-acetyl)2-(gamma-Glu)-CO-(CH2)18-CO 2H
  SITE 20: note = MISC_FEATURE - Xaa at position 20 is Aib
  MOD_RES 39: note = Ser at position 39 is amidated
XXEGTFTSDYSIXLDKKAQXAFIEYLIEGGPSSGAPPPS

SEQ ID NO: 350 - protein, 39 aa, synthetic construct
  REGION 1..39: note = Synthetic Construct
  SITE 1: note = MISC_FEATURE - Xaa at position 1 is D-Tyr
  SITE 2: note = MISC_FEATURE - Xaa at position 2 is Aib
  SITE 6: note = MISC_FEATURE - Xaa at position 6 is alpha-methyl-Phe
  SITE 13: note = MISC_FEATURE - Xaa at position 13 is alpha-methyl-Leu
  MOD_RES 17: note = Lys at position 17 is chemically modified by conjugation of the epsilon-amino group of the Lys side chain with (2-[2-(2-amino-ethoxy)-ethoxy]-acetyl)2-(gamma-Glu)-CO-(CH2)18-CO 2H
  SITE 20: note = MISC_FEATURE - Xaa at position 20 is Aib
  MOD_RES 39: note = Ser at position 39 is amidated
XXEGTXTSDYSIXLDKKAQXAFIEYLIEGGPSSGAPPPS

SEQ ID NO: 351 - protein, 39 aa, synthetic construct; identical to SEQ ID NO: 350
  REGION 1..39: note = Synthetic Construct
  SITE 1: note = MISC_FEATURE - Xaa at position 1 is D-Tyr
  SITE 2: note = MISC_FEATURE - Xaa at position 2 is Aib
  SITE 6: note = MISC_FEATURE - Xaa at position 6 is alpha-methyl-Phe(2F)
  SITE 13: note = MISC_FEATURE - Xaa at position 13 is alpha-methyl-Leu
  MOD_RES 17: note = Lys at position 17 is chemically modified by conjugation of the epsilon-amino group of the Lys side chain with (2-[2-(2-amino-ethoxy)-ethoxy]-acetyl)2-(gamma-Glu)-CO-(CH2)18-CO 2H
  SITE 20: note = MISC_FEATURE - Xaa at position 20 is Aib
  MOD_RES 39: note = Ser at position 39 is amidated

SEQ ID NO: 352 - protein, 39 aa, synthetic construct
  REGION 1..39: note = Synthetic Construct
  SITE 2: note = MISC_FEATURE - Xaa at position 2 is Aib
  SITE 13: note = MISC_FEATURE - Xaa at position 13 is alpha-methyl-Leu
  MOD_RES 17: note = Lys at position 17 is chemically modified by conjugation of the epsilon-amino group of the Lys side chain with (2-[2-(2-amino-ethoxy)-ethoxy]-acetyl)2-(gamma-Glu)-CO-(CH2)18-CO 2H
  SITE 20: note = MISC_FEATURE - Xaa at position 20 is Aib
  MOD_RES 39: note = Ser at position 39 is amidated
FXEGTFTSDYSIXLDKKAQXAFIEYLIAGGPSSGAPPPS

SEQ ID NO: 353 - protein, 39 aa, synthetic construct
  REGION 1..39: note = Synthetic Construct
  SITE 2: note = MISC_FEATURE - Xaa at position 2 is Aib
  SITE 13: note = MISC_FEATURE - Xaa at position 13 is alpha-methyl-Leu
  MOD_RES 17: note = Lys at position 17 is chemically modified by conjugation of the epsilon-amino group of the Lys side chain with (2-[2-(2-amino-ethoxy)-ethoxy]-acetyl)2-(gamma-Glu)-CO-(CH2)18-CO 2H
  SITE 20: note = MISC_FEATURE - Xaa at position 20 is Aib
  MOD_RES 39: note = Ser at position 39 is amidated
FXEGTFTSDYSIXLDKKAQXEFIEYLIAGGPSSGAPPPS

SEQ ID NO: 354 - protein, 39 aa, synthetic construct; identical to SEQ ID NO: 304
  REGION 1..39: note = Synthetic Construct
  SITE 2: note = MISC_FEATURE - Xaa at position 2 is Aib
  SITE 13: note = MISC_FEATURE - Xaa at position 13 is alpha-methyl-Leu
  MOD_RES 17: note = Lys at position 17 is chemically modified by conjugation of the epsilon-amino group of the Lys side chain with (2-[2-(2-amino-ethoxy)-ethoxy]-acetyl)-(gamma-Glu)-CO-(CH2)18-CO2 H
  SITE 20: note = MISC_FEATURE - Xaa at position 20 is Aib
  MOD_RES 39: note = Ser at position 39 is amidated

SEQ ID NO: 355 - protein, 39 aa, synthetic construct
  REGION 1..39: note = Synthetic Construct
  SITE 1: note = MISC_FEATURE - Xaa at position 1 is D-Tyr
  SITE 2: note = MISC_FEATURE - Xaa at position 2 is Aib
  SITE 13: note = MISC_FEATURE - Xaa at position 13 is alpha-methyl-Leu
  MOD_RES 17: note = Lys at position 17 is chemically modified by conjugation of the epsilon-amino group of the Lys side chain with (2-[2-(2-amino-ethoxy)-ethoxy]-acetyl)2-(gamma-Glu)-CO-(CH2)18-CO 2H
  SITE 20: note = MISC_FEATURE - Xaa at position 20 is Aib
  MOD_RES 39: note = Ser at position 39 is amidated
XXEGTFTSDYSIXLDKKAQXAFIEYLIAGGPSSGAPPPS

SEQ ID NO: 356 - protein, 39 aa, synthetic construct
  REGION 1..39: note = Synthetic Construct
  SITE 1: note = MISC_FEATURE - Xaa at position 1 is D-Tyr
  SITE 2: note = MISC_FEATURE - Xaa at position 2 is Aib
  SITE 13: note = MISC_FEATURE - Xaa at position 13 is alpha-methyl-Leu
  MOD_RES 17: note = Lys at position 17 is chemically modified by conjugation of the epsilon-amino group of the Lys side chain with (2-[2-(2-amino-ethoxy)-ethoxy]-acetyl)2-(gamma-Glu)-CO-(CH2)18-CO 2H
  SITE 20: note = MISC_FEATURE - Xaa at position 20 is Aib
  MOD_RES 39: note = Ser at position 39 is amidated
XXEGTFTSDYSIXLDEKAQXAFIEYLIAGGPSSGAPPPS

SEQ ID NO: 357 - protein, 39 aa, synthetic construct
  REGION 1..39: note = Synthetic Construct
  SITE 1: note = MISC_FEATURE - Xaa at position 1 is D-Tyr
  SITE 2: note = MISC_FEATURE - Xaa at position 2 is Aib
  SITE 13: note = MISC_FEATURE - Xaa at position 13 is alpha-methyl-Leu
  MOD_RES 17: note = Lys at position 17 is chemically modified by conjugation of the epsilon-amino group of the Lys side chain with (2-[2-(2-amino-ethoxy)-ethoxy]-acetyl)2-(gamma-Glu)-CO-(CH2)18-CO 2H
  SITE 20: note = MISC_FEATURE - Xaa at position 20 is Aib
  MOD_RES 39: note = Ser at position 39 is amidated
XXEGTFTSDYSIXLDEKAQXEFIEYLIAGGPSSGAPPPS

SEQ ID NO: 358 - protein, 39 aa, synthetic construct
  REGION 1..39: note = Synthetic Construct
  SITE 2: note = MISC_FEATURE - Xaa at position 2 is Aib
  SITE 13: note = MISC_FEATURE - Xaa at position 13 is alpha-methyl-Leu
  MOD_RES 17: note = Lys at position 17 is chemically modified by conjugation of the epsilon-amino group of the Lys side chain with (2-[2-(2-amino-ethoxy)-ethoxy]-acetyl)2-(gamma-Glu)-CO-(CH2)18-CO 2H
  SITE 20: note = MISC_FEATURE - Xaa at position 20 is Aib
  SITE 24: note = MISC_FEATURE - Xaa at position 24 is D-Glu
  MOD_RES 39: note = Ser at position 39 is amidated
YXEGTFTSDYSIXLDEKAQXAFIXYLIAGGPSSGAPPPS

SEQ ID NO: 359 - protein, 39 aa, synthetic construct
  REGION 1..39: note = Synthetic Construct
  SITE 2: note = MISC_FEATURE - Xaa at position 2 is Aib
  SITE 13: note = MISC_FEATURE - Xaa at position 13 is alpha-methyl-Leu
  MOD_RES 17: note = Lys at position 17 is chemically modified by conjugation of the epsilon-amino group of the Lys side chain with (2-[2-(2-amino-ethoxy)-ethoxy]-acetyl)2-(gamma-Glu)-CO-(CH2)18-CO 2H
  SITE 20: note = MISC_FEATURE - Xaa at position 20 is Aib
  MOD_RES 39: note = Ser at position 39 is amidated
YXEGTFTSDYSIXLDEKAQXDFIEYLIAGGPSSGAPPPS

SEQ ID NO: 360 - protein, 39 aa, synthetic construct
  REGION 1..39: note = Synthetic Construct
  SITE 1: note = MISC_FEATURE - Xaa at position 1 is D-Tyr
  SITE 2: note = MISC_FEATURE - Xaa at position 2 is Aib
  SITE 6: note = MISC_FEATURE - Xaa at position 6 is alpha-methyl-Phe
  SITE 13: note = MISC_FEATURE - Xaa at position 13 is alpha-methyl-Leu
  MOD_RES 17: note = Lys at position 17 is chemically modified by conjugation of the epsilon-amino group of the Lys side chain with (2-[2-(2-amino-ethoxy)-ethoxy]-acetyl)2-(gamma-Glu)-CO-(CH2)18-CO 2H
  SITE 20: note = MISC_FEATURE - Xaa at position 20 is Aib
  MOD_RES 39: note = Ser at position 39 is amidated
XXEGTXTSDYSIXLDKKAQXEFIEYLIAGGPSSGAPPPS

SEQ ID NO: 361 - protein, 39 aa, synthetic construct
  REGION 1..39: note = Synthetic Construct
  SITE 1: note = MISC_FEATURE - Xaa at position 1 is D-Tyr
  SITE 2: note = MISC_FEATURE - Xaa at position 2 is Aib
  SITE 13: note = MISC_FEATURE - Xaa at position 13 is alpha-methyl-Leu
  SITE 16: note = MISC_FEATURE - Xaa at position 16 is Orn
  MOD_RES 17: note = Lys at position 17 is chemically modified by conjugation of the epsilon-amino group of the Lys side chain with (2-[2-(2-amino-ethoxy)-ethoxy]-acetyl)2-(gamma-Glu)-CO-(CH2)18-CO 2H
  SITE 20: note = MISC_FEATURE - Xaa at position 20 is Aib
  MOD_RES 39: note = Ser at position 39 is amidated
XXEGTFTSDYSIXLDXKAQXAFIEYLIAGGPSSGAPPPS

SEQ ID NO: 362 - protein, 39 aa, synthetic construct; identical to SEQ ID NO: 361
  REGION 1..39: note = Synthetic Construct
  SITE 1: note = MISC_FEATURE - Xaa at position 1 is D-Tyr
  SITE 2: note = MISC_FEATURE - Xaa at position 2 is Aib
  SITE 13: note = MISC_FEATURE - Xaa at position 13 is alpha-methyl-Leu
  SITE 16: note = MISC_FEATURE - Xaa at position 16 is Dab
  MOD_RES 17: note = Lys at position 17 is chemically modified by conjugation of the epsilon-amino group of the Lys side chain with (2-[2-(2-amino-ethoxy)-ethoxy]-acetyl)2-(gamma-Glu)-CO-(CH2)18-CO 2H
  SITE 20: note = MISC_FEATURE - Xaa at position 20 is Aib
  MOD_RES 39: note = Ser at position 39 is amidated

SEQ ID NO: 363 - protein, 39 aa, synthetic construct; identical to SEQ ID NO: 361
  REGION 1..39: note = Synthetic Construct
  SITE 1: note = MISC_FEATURE - Xaa at position 1 is D-Tyr
  SITE 2: note = MISC_FEATURE - Xaa at position 2 is Aib
  SITE 13: note = MISC_FEATURE - Xaa at position 13 is alpha-methyl-Leu
  SITE 16: note = MISC_FEATURE - Xaa at position 16 is Dap
  MOD_RES 17: note = Lys at position 17 is chemically modified by conjugation of the epsilon-amino group of the Lys side chain with (2-[2-(2-amino-ethoxy)-ethoxy]-acetyl)2-(gamma-Glu)-CO-(CH2)18-CO 2H
  SITE 20: note = MISC_FEATURE - Xaa at position 20 is Aib
  MOD_RES 39: note = Ser at position 39 is amidated

SEQ ID NO: 364 - protein, 39 aa, synthetic construct
  REGION 1..39: note = Synthetic Construct
  SITE 1: note = MISC_FEATURE - Xaa at position 1 is D-Tyr
  SITE 2: note = MISC_FEATURE - Xaa at position 2 is Aib
  SITE 13: note = MISC_FEATURE - Xaa at position 13 is alpha-methyl-Leu
  SITE 16: note = MISC_FEATURE - Xaa at position 16 is Orn
  MOD_RES 17: note = Lys at position 17 is chemically modified by conjugation of the epsilon-amino group of the Lys side chain with (2-[2-(2-amino-ethoxy)-ethoxy]-acetyl)2-(gamma-Glu)-CO-(CH2)18-CO 2H
  SITE 20: note = MISC_FEATURE - Xaa at position 20 is Aib
  MOD_RES 39: note = Ser at position 39 is amidated
XXEGTFTSDYSIXLDXKAQXEFIEYLIAGGPSSGAPPPS

SEQ ID NO: 365 - protein, 39 aa, synthetic construct; identical to SEQ ID NO: 364
  REGION 1..39: note = Synthetic Construct
  SITE 1: note = MISC_FEATURE - Xaa at position 1 is D-Tyr
  SITE 2: note = MISC_FEATURE - Xaa at position 2 is Aib
  SITE 13: note = MISC_FEATURE - Xaa at position 13 is alpha-methyl-Leu
  SITE 16: note = MISC_FEATURE - Xaa at position 16 is Dab
  MOD_RES 17: note = Lys at position 17 is chemically modified by conjugation of the epsilon-amino group of the Lys side chain with (2-[2-(2-amino-ethoxy)-ethoxy]-acetyl)2-(gamma-Glu)-CO-(CH2)18-CO 2H
  SITE 20: note = MISC_FEATURE - Xaa at position 20 is Aib
  MOD_RES 39: note = Ser at position 39 is amidated

SEQ ID NO: 366 - protein, 39 aa, synthetic construct; identical to SEQ ID NO: 364
  REGION 1..39: note = Synthetic Construct
  SITE 1: note = MISC_FEATURE - Xaa at position 1 is D-Tyr
  SITE 2: note = MISC_FEATURE - Xaa at position 2 is Aib
  SITE 13: note = MISC_FEATURE - Xaa at position 13 is alpha-methyl-Leu
  SITE 16: note = MISC_FEATURE - Xaa at position 16 is Dap
  MOD_RES 17: note = Lys at position 17 is chemically modified by conjugation of the epsilon-amino group of the Lys side chain with (2-[2-(2-amino-ethoxy)-ethoxy]-acetyl)2-(gamma-Glu)-CO-(CH2)18-CO 2H
  SITE 20: note = MISC_FEATURE - Xaa at position 20 is Aib
  MOD_RES 39: note = Ser at position 39 is amidated

SEQ ID NO: 367 - protein, 39 aa, synthetic construct
  REGION 1..39: note = Synthetic Construct
  SITE 1: note = MISC_FEATURE - Xaa at position 1 is D-Tyr
  SITE 2: note = MISC_FEATURE - Xaa at position 2 is Aib
  SITE 13: note = MISC_FEATURE - Xaa at position 13 is alpha-methyl-Leu
  MOD_RES 17: note = Lys at position 17 is chemically modified by conjugation of the epsilon-amino group of the Lys side chain with (2-[2-(2-amino-ethoxy)-ethoxy]-acetyl)2-(gamma-Glu)-CO-(CH2)18-CO 2H
  SITE 20: note = MISC_FEATURE - Xaa at position 20 is Aib
  SITE 24: note = MISC_FEATURE - Xaa at position 24 is D-Glu
  MOD_RES 39: note = Ser at position 39 is amidated
XXEGTFTSDYSIXLDKKAQXAFIXYLIAGGPSSGAPPPS

SEQ ID NO: 368 - protein, 39 aa, synthetic construct
  REGION 1..39: note = Synthetic Construct
  SITE 1: note = MISC_FEATURE - Xaa at position 1 is D-Tyr
  SITE 2: note = MISC_FEATURE - Xaa at position 2 is Aib
  SITE 13: note = MISC_FEATURE - Xaa at position 13 is alpha-methyl-Leu
  MOD_RES 17: note = Lys at position 17 is chemically modified by conjugation of the epsilon-amino group of the Lys side chain with (2-[2-(2-amino-ethoxy)-ethoxy]-acetyl)2-(gamma-Glu)-CO-(CH2)18-CO 2H
  SITE 20: note = MISC_FEATURE - Xaa at position 20 is Aib
  SITE 24: note = MISC_FEATURE - Xaa at position 24 is D-Glu
  MOD_RES 39: note = Ser at position 39 is amidated
XXEGTFTSDYSIXLDKKAQXEFIXYLIEGGPSSGAPPPS

SEQ ID NO: 369 - protein, 39 aa, synthetic construct
  REGION 1..39: note = Synthetic Construct
  SITE 1: note = MISC_FEATURE - Xaa at position 1 is D-Tyr
  SITE 2: note = MISC_FEATURE - Xaa at position 2 is Aib
  SITE 13: note = MISC_FEATURE - Xaa at position 13 is alpha-methyl-Leu
  SITE 16: note = MISC_FEATURE - Xaa at position 16 is Orn
  MOD_RES 17: note = Lys at position 17 is chemically modified by conjugation of the epsilon-amino group of the Lys side chain with (2-[2-(2-amino-ethoxy)-ethoxy]-acetyl)2-(gamma-Glu)-CO-(CH2)18-CO 2H
  SITE 20: note = MISC_FEATURE - Xaa at position 20 is Aib
  SITE 24: note = MISC_FEATURE - Xaa at position 24 is D-Glu
  MOD_RES 39: note = Ser at position 39 is amidated
XXEGTFTSDYSIXLDXKAQXEFIXYLIAGGPSSGAPPPS

SEQ ID NO: 370 - protein, 39 aa, synthetic construct
  REGION 1..39: note = Synthetic Construct
  SITE 1: note = MISC_FEATURE - Xaa at position 1 is D-Tyr
  SITE 2: note = MISC_FEATURE - Xaa at position 2 is Aib
  SITE 13: note = MISC_FEATURE - Xaa at position 13 is alpha-methyl-Leu
  SITE 16: note = MISC_FEATURE - Xaa at position 16 is Orn
  MOD_RES 17: note = Lys at position 17 is chemically modified by conjugation of the epsilon-amino group of the Lys side chain with (2-[2-(2-amino-ethoxy)-ethoxy]-acetyl)2-(gamma-Glu)-CO-(CH2)18-CO 2H
  SITE 20: note = MISC_FEATURE - Xaa at position 20 is Aib
  SITE 24: note = MISC_FEATURE - Xaa at position 24 is D-Glu
  MOD_RES 39: note = Ser at position 39 is amidated
XXEGTFTSDYSIXLDXKAQXEFIXYLIEGGPSSGAPPPS

SEQ ID NO: 371 - protein, 39 aa, synthetic construct
  REGION 1..39: note = Synthetic Construct
  SITE 1: note = MISC_FEATURE - Xaa at position 1 is D-Tyr
  SITE 2: note = MISC_FEATURE - Xaa at position 2 is Aib
  SITE 13: note = MISC_FEATURE - Xaa at position 13 is alpha-methyl-Leu
  MOD_RES 17: note = Lys at position 17 is chemically modified by conjugation of the epsilon-amino group of the Lys side chain with (2-[2-(2-amino-ethoxy)-ethoxy]-acetyl)2-(gamma-Glu)-CO-(CH2)18-CO 2H
  SITE 20: note = MISC_FEATURE - Xaa at position 20 is Aib
  SITE 24: note = MISC_FEATURE - Xaa at position 24 is D-Glu
  MOD_RES 39: note = Ser at position 39 is amidated
XXEGTFTSDYSIXLDKKAQXAFIXYLIEGGPSSGAPPPS

SEQ ID NO: 372 - protein, 39 aa, synthetic construct
  REGION 1..39: note = Synthetic Construct
  SITE 1: note = MISC_FEATURE - Xaa at position 1 is D-Tyr
  SITE 2: note = MISC_FEATURE - Xaa at position 2 is Aib
  SITE 13: note = MISC_FEATURE - Xaa at position 13 is alpha-methyl-Leu
  SITE 16: note = MISC_FEATURE - Xaa at position 16 is Orn
  MOD_RES 17: note = Lys at position 17 is chemically modified by conjugation of the epsilon-amino group of the Lys side chain with (2-[2-(2-amino-ethoxy)-ethoxy]-acetyl)2-(gamma-Glu)-CO-(CH2)18-CO 2H
  SITE 20: note = MISC_FEATURE - Xaa at position 20 is Aib
  SITE 24: note = MISC_FEATURE - Xaa at position 24 is D-Glu
  MOD_RES 39: note = Ser at position 39 is amidated
XXEGTFTSDYSIXLDXKAQXAFIXYLIEGGPSSGAPPPS

SEQ ID NO: 373 - protein, 39 aa, synthetic construct
  REGION 1..39: note = Synthetic Construct
  SITE 1: note = MISC_FEATURE - Xaa at position 1 is D-Tyr
  SITE 2: note = MISC_FEATURE - Xaa at position 2 is Aib
  SITE 13: note = MISC_FEATURE - Xaa at position 13 is alpha-methyl-Leu
  SITE 16: note = MISC_FEATURE - Xaa at position 16 is Orn
  MOD_RES 17: note = Lys at position 17 is chemically modified by conjugation of the epsilon-amino group of the Lys side chain with (2-[2-(2-amino-ethoxy)-ethoxy]-acetyl)2-(gamma-Glu)-CO-(CH2)18-CO 2H
  SITE 20: note = MISC_FEATURE - Xaa at position 20 is Aib
  MOD_RES 39: note = Ser at position 39 is amidated
XXEGTFTSDYSIXLDXKAQXAFVEYLIAGGPSSGAPPPS

SEQ ID NO: 374 - protein, 39 aa, synthetic construct
  REGION 1..39: note = Synthetic Construct
  SITE 1: note = MISC_FEATURE - Xaa at position 1 is D-Tyr
  SITE 2: note = MISC_FEATURE - Xaa at position 2 is Aib
  SITE 13: note = MISC_FEATURE - Xaa at position 13 is alpha-methyl-Leu
  SITE 16: note = MISC_FEATURE - Xaa at position 16 is Orn
  MOD_RES 17: note = Lys at position 17 is chemically modified by conjugation of the epsilon-amino group of the Lys side chain with (2-[2-(2-amino-ethoxy)-ethoxy]-acetyl)2-(gamma-Glu)-CO-(CH2)18-CO 2H
  SITE 20: note = MISC_FEATURE - Xaa at position 20 is Aib
  MOD_RES 39: note = Ser at position 39 is amidated
XXEGTFTSDYSIXLDXKAQXEFVEYLIAGGPSSGAPPPS

SEQ ID NO: 375 - protein, 39 aa, synthetic construct
  REGION 1..39: note = Synthetic Construct
  SITE 1: note = MISC_FEATURE - Xaa at position 1 is D-Tyr
  SITE 2: note = MISC_FEATURE - Xaa at position 2 is Aib
  SITE 13: note = MISC_FEATURE - Xaa at position 13 is alpha-methyl-Leu
  SITE 16: note = MISC_FEATURE - Xaa at position 16 is Orn
  MOD_RES 17: note = Lys at position 17 is chemically modified by conjugation of the epsilon-amino group of the Lys side chain with (2-[2-(2-amino-ethoxy)-ethoxy]-acetyl)2-(gamma-Glu)-CO-(CH2)18-CO 2H
  SITE 20: note = MISC_FEATURE - Xaa at position 20 is Aib
  MOD_RES 39: note = Ser at position 39 is amidated
XXEGTFTSDYSIXLDXKAQXAFVEYLIEGGPSSGAPPPS

SEQ ID NO: 376 - protein, 39 aa, synthetic construct
  REGION 1..39: note = Synthetic Construct
  SITE 1: note = MISC_FEATURE - Xaa at position 1 is D-Tyr
  SITE 2: note = MISC_FEATURE - Xaa at position 2 is Aib
  SITE 13: note = MISC_FEATURE - Xaa at position 13 is alpha-methyl-Leu
  MOD_RES 17: note = Lys at position 17 is chemically modified by conjugation of the epsilon-amino group of the Lys side chain with (2-[2-(2-amino-ethoxy)-ethoxy]-acetyl)2-(gamma-Glu)-CO-(CH2)18-CO 2H
  SITE 20: note = MISC_FEATURE - Xaa at position 20 is Aib
  SITE 24: note = MISC_FEATURE - Xaa at position 24 is D-Glu
  MOD_RES 39: note = Ser at position 39 is amidated
XXEGTFTSDYSIXLDKKAQXAFVXYLIAGGPSSGAPPPS

SEQ ID NO: 377 - protein, 39 aa, synthetic construct
  REGION 1..39: note = Synthetic Construct
  SITE 1: note = MISC_FEATURE - Xaa at position 1 is D-Tyr
  SITE 2: note = MISC_FEATURE - Xaa at position 2 is Aib
  SITE 13: note = MISC_FEATURE - Xaa at position 13 is alpha-methyl-Leu
  SITE 16: note = MISC_FEATURE - Xaa at position 16 is Orn
  MOD_RES 17: note = Lys at position 17 is chemically modified by conjugation of the epsilon-amino group of the Lys side chain with (2-[2-(2-amino-ethoxy)-ethoxy]-acetyl)2-(gamma-Glu)-CO-(CH2)18-CO 2H
  SITE 20: note = MISC_FEATURE - Xaa at position 20 is Aib
  SITE 24: note = MISC_FEATURE - Xaa at position 24 is D-Glu
  MOD_RES 39: note = Ser at position 39 is amidated
XXEGTFTSDYSIXLDXKAQXAFVXYLIAGGPSSGAPPPS

SEQ ID NO: 378 - protein, 39 aa, synthetic construct; identical to SEQ ID NO: 306
  REGION 1..39: note = Synthetic Construct
  SITE 1: note = MISC_FEATURE - Xaa at position 1 is D-Tyr
  SITE 2: note = MISC_FEATURE - Xaa at position 2 is Aib
  SITE 13: note = MISC_FEATURE - Xaa at position 13 is alpha-methyl-Leu
  SITE 16: note = MISC_FEATURE - Xaa at position 16 is Orn
  MOD_RES 17: note = Lys at position 17 is chemically modified by conjugation of the epsilon-amino group of the Lys side chain with (2-[2-(2-amino-ethoxy)-ethoxy]-acetyl)2-(gamma-Glu)-CO-(CH2)16-CO 2H
  SITE 20: note = MISC_FEATURE - Xaa at position 20 is Aib
  SITE 24: note = MISC_FEATURE - Xaa at position 24 is D-Glu
  MOD_RES 39: note = Ser at position 39 is amidated

SEQ ID NO: 379 - protein, 39 aa, synthetic construct; identical to SEQ ID NO: 377
  REGION 1..39: note = Synthetic Construct
  SITE 1: note = MISC_FEATURE - Xaa at position 1 is D-Tyr
  SITE 2: note = MISC_FEATURE - Xaa at position 2 is Aib
  SITE 13: note = MISC_FEATURE - Xaa at position 13 is alpha-methyl-Leu
  SITE 16: note = MISC_FEATURE - Xaa at position 16 is Orn
  MOD_RES 17: note = Lys at position 17 is chemically modified by conjugation of the epsilon-amino group of the Lys side chain with (2-[2-(2-amino-ethoxy)-ethoxy]-acetyl)2-(gamma-Glu)-CO-(CH2)16-CO 2H
  SITE 20: note = MISC_FEATURE - Xaa at position 20 is Aib
  SITE 24: note = MISC_FEATURE - Xaa at position 24 is D-Glu
  MOD_RES 39: note = Ser at position 39 is amidated

SEQ ID NO: 380 - protein, 39 aa, synthetic construct
  REGION 1..39: note = Synthetic Construct
  SITE 1: note = MISC_FEATURE - Xaa at position 1 is D-Tyr
  SITE 2: note = MISC_FEATURE - Xaa at position 2 is Aib
  SITE 13: note = MISC_FEATURE - Xaa at position 13 is alpha-methyl-Leu
  MOD_RES 17: note = Lys at position 17 is chemically modified by conjugation of the epsilon-amino group of the Lys side chain with (2-[2-(2-amino-ethoxy)-ethoxy]-acetyl)2-(gamma-Glu)-CO-(CH2)18-CO 2H
  SITE 20: note = MISC_FEATURE - Xaa at position 20 is Aib
  SITE 25: note = MISC_FEATURE - Xaa at position 25 is alpha-methyl-Tyr
  MOD_RES 39: note = Ser at position 39 is amidated
XXEGTFTSDYSIXLDKKAQXAFIEXLIAGGPSSGAPPPS

SEQ ID NO: 381 - protein, 39 aa, synthetic construct
  REGION 1..39: note = Synthetic Construct
  SITE 1: note = MISC_FEATURE - Xaa at position 1 is D-Tyr
  SITE 2: note = MISC_FEATURE - Xaa at position 2 is Aib
  SITE 13: note = MISC_FEATURE - Xaa at position 13 is alpha-methyl-Leu
  SITE 16: note = MISC_FEATURE - Xaa at position 16 is Orn
  MOD_RES 17: note = Lys at position 17 is chemically modified by conjugation of the epsilon-amino group of the Lys side chain with (2-[2-(2-amino-ethoxy)-ethoxy]-acetyl)2-(gamma-Glu)-CO-(CH2)18-CO 2H
  SITE 20: note = MISC_FEATURE - Xaa at position 20 is Aib
  SITE 25: note = MISC_FEATURE - Xaa at position 25 is alpha-methyl-Tyr
  MOD_RES 39: note = Ser at position 39 is amidated
XXEGTFTSDYSIXLDXKAQXAFIEXLIAGGPSSGAPPPS

SEQ ID NO: 382 - protein, 39 aa, synthetic construct
  REGION 1..39: note = Synthetic Construct
  SITE 2: note = MISC_FEATURE - Xaa at position 2 is Aib
  SITE 13: note = MISC_FEATURE - Xaa at position 13 is alpha-methyl-Leu
  MOD_RES 17: note = Lys at position 17 is chemically modified by conjugation of the epsilon-amino group of the Lys side chain with (2-[2-(2-amino-ethoxy)-ethoxy]-acetyl)2-(gamma-Glu)-CO-(CH2)18-CO 2H
  SITE 20: note = MISC_FEATURE - Xaa at position 20 is Aib
  SITE 25: note = MISC_FEATURE - Xaa at position 25 is alpha-methyl-Tyr
  MOD_RES 39: note = Ser at position 39 is amidated
YXEGTFTSDYSIXLDKKAQXEFIEXLIAGGPSSGAPPPS

SEQ ID NO: 383 - protein, 39 aa, synthetic construct; identical to SEQ ID NO: 364
  REGION 1..39: note = Synthetic Construct
  SITE 1: note = MISC_FEATURE - Xaa at position 1 is D-Tyr
  SITE 2: note = MISC_FEATURE - Xaa at position 2 is Aib
  SITE 13: note = MISC_FEATURE - Xaa at position 13 is alpha-methyl-Leu
  SITE 16: note = MISC_FEATURE - Xaa at position 16 is Orn
  MOD_RES 17: note = Lys at position 17 is chemically modified by conjugation of the epsilon-amino group of the Lys side chain with (2-[2-(2-amino-ethoxy)-ethoxy]-acetyl)2-(gamma-Glu)-CO-(CH2)16-CO 2H
  SITE 20: note = MISC_FEATURE - Xaa at position 20 is Aib
  MOD_RES 39: note = Ser at position 39 is amidated

SEQ ID NO: 384 - protein, 39 aa, synthetic construct
  REGION 1..39: note = Synthetic Construct
  SITE 1: note = MISC_FEATURE - Xaa at position 1 is D-Tyr
  SITE 2: note = MISC_FEATURE - Xaa at position 2 is Aib
  SITE 13: note = MISC_FEATURE - Xaa at position 13 is alpha-methyl-Leu
  SITE 16: note = MISC_FEATURE - Xaa at position 16 is Orn
  MOD_RES 17: note = Lys at position 17 is chemically modified by conjugation of the epsilon-amino group of the Lys side chain with (2-[2-(2-amino-ethoxy)-ethoxy]-acetyl)2-(gamma-Glu)-CO-(CH2)18-CO 2H
  SITE 20: note = MISC_FEATURE - Xaa at position 20 is Aib
  MOD_RES 39: note = Ser at position 39 is amidated
XXEGTFTSDYSIXLDXKAQXDFIEYLIAGGPSSGAPPPS

SEQ ID NO: 385 - protein, 34 aa, synthetic construct
  REGION 1..34: note = Synthetic Construct
  SITE 1: note = MISC_FEATURE - Xaa at position 1 is D-Tyr
  SITE 2: note = MISC_FEATURE - Xaa at position 2 is Aib
  SITE 13: note = MISC_FEATURE - Xaa at position 13 is alpha-methyl-Leu
  SITE 16: note = MISC_FEATURE - Xaa at position 16 is Orn
  MOD_RES 17: note = Lys at position 17 is chemically modified by conjugation of the epsilon-amino group of the Lys side chain with (2-[2-(2-amino-ethoxy)-ethoxy]-acetyl)2-(gamma-Glu)-CO-(CH2)18-CO 2H
  SITE 20: note = MISC_FEATURE - Xaa at position 20 is Aib
  MOD_RES 34: note = Gly at position 34 is amidated
XXEGTFTSDYSIXLDXKAQXEFIEYLIAGGPSSG

SEQ ID NO: 386 - protein, 39 aa, synthetic construct; identical to SEQ ID NO: 364
  REGION 1..39: note = Synthetic Construct
  SITE 1: note = MISC_FEATURE - Xaa at position 1 is D-Tyr
  SITE 2: note = MISC_FEATURE - Xaa at position 2 is Aib
  SITE 13: note = MISC_FEATURE - Xaa at position 13 is alpha-methyl-Leu
  SITE 16: note = MISC_FEATURE - Xaa at position 16 is Orn
  MOD_RES 17: note = Lys at position 17 is chemically modified by conjugation of the epsilon-amino group of the Lys side chain with (2-[2-(2-amino-ethoxy)-ethoxy]-acetyl)-(gamma-Glu)-CO-(CH2)18-CO2 H
  SITE 20: note = MISC_FEATURE - Xaa at position 20 is Aib
  MOD_RES 39: note = Ser at position 39 is amidated

SEQ ID NO: 387 - protein, 39 aa, synthetic construct; identical to SEQ ID NO: 307
  REGION 1..39: note = Synthetic Construct
  SITE 1: note = MISC_FEATURE - Xaa at position 1 is D-Tyr
  SITE 2: note = MISC_FEATURE - Xaa at position 2 is Aib
  SITE 13: note = MISC_FEATURE - Xaa at position 13 is alpha-methyl-Leu
  MOD_RES 17: note = Lys at position 17 is chemically modified by conjugation of the epsilon-amino group of the Lys side chain with (2-[2-(2-amino-ethoxy)-ethoxy]-acetyl)-(gamma-Glu)-CO-(CH2)18-CO2 H
  SITE 20: note = MISC_FEATURE - Xaa at position 20 is Aib
  SITE 25: note = MISC_FEATURE - Xaa at position 25 is alpha-methyl-Tyr
  MOD_RES 39: note = Ser at position 39 is amidated

SEQ ID NO: 388 - protein, 39 aa, synthetic construct; identical to SEQ ID NO: 380
  REGION 1..39: note = Synthetic Construct
  SITE 1: note = MISC_FEATURE - Xaa at position 1 is D-Tyr
  SITE 2: note = MISC_FEATURE - Xaa at position 2 is Aib
  SITE 13: note = MISC_FEATURE - Xaa at position 13 is alpha-methyl-Leu
  MOD_RES 17: note = Lys at position 17 is chemically modified by conjugation of the epsilon-amino group of the Lys side chain with (2-[2-(2-amino-ethoxy)-ethoxy]-acetyl)-(gamma-Glu)-CO-(CH2)18-CO2 H
  SITE 20: note = MISC_FEATURE - Xaa at position 20 is Aib
  SITE 25: note = MISC_FEATURE - Xaa at position 25 is alpha-methyl-Tyr
  MOD_RES 39: note = Ser at position 39 is amidated

SEQ ID NO: 389 - protein, 39 aa, synthetic construct; identical to SEQ ID NO: 307
  REGION 1..39: note = Synthetic Construct
  SITE 1: note = MISC_FEATURE - Xaa at position 1 is D-Tyr
  SITE 2: note = MISC_FEATURE - Xaa at position 2 is Aib
  SITE 13: note = MISC_FEATURE - Xaa at position 13 is alpha-methyl-Leu
  MOD_RES 17: note = Lys at position 17 is chemically modified by conjugation of the epsilon-amino group of the Lys side chain with (2-[2-(2-amino-ethoxy)-ethoxy]-acetyl)2-(gamma-Glu)-CO-(CH2)16-CO 2H
  SITE 20: note = MISC_FEATURE - Xaa at position 20 is Aib
  SITE 25: note = MISC_FEATURE - Xaa at position 25 is alpha-methyl-Tyr
  MOD_RES 39: note = Ser at position 39 is amidated

SEQ ID NO: 390 - protein, 39 aa, synthetic construct; identical to SEQ ID NO: 308
  REGION 1..39: note = Synthetic Construct
  SITE 1: note = MISC_FEATURE - Xaa at position 1 is D-Tyr
  SITE 2: note = MISC_FEATURE - Xaa at position 2 is Aib
  SITE 13: note = MISC_FEATURE - Xaa at position 13 is alpha-methyl-Leu
  SITE 16: note = MISC_FEATURE - Xaa at position 16 is Orn
  MOD_RES 17: note = Lys at position 17 is chemically modified by conjugation of the epsilon-amino group of the Lys side chain with (2-[2-(2-amino-ethoxy)-ethoxy]-acetyl)2-(gamma-Glu)-CO-(CH2)16-CO 2H
  SITE 20: note = MISC_FEATURE - Xaa at position 20 is Aib
  SITE 25: note = MISC_FEATURE - Xaa at position 25 is alpha-methyl-Tyr
  MOD_RES 39: note = Ser at position 39 is amidated

SEQ ID NO: 391 - protein, 39 aa, synthetic construct; identical to SEQ ID NO: 380
  REGION 1..39: note = Synthetic Construct
  SITE 1: note = MISC_FEATURE - Xaa at position 1 is D-Tyr
  SITE 2: note = MISC_FEATURE - Xaa at position 2 is Aib
  SITE 13: note = MISC_FEATURE - Xaa at position 13 is alpha-methyl-Leu
  MOD_RES 17: note = Lys at position 17 is chemically modified by conjugation of the epsilon-amino group of the Lys side chain with (2-[2-(2-amino-ethoxy)-ethoxy]-acetyl)2-(gamma-Glu)-CO-(CH2)16-CO 2H
  SITE 20: note = MISC_FEATURE - Xaa at position 20 is Aib
  SITE 25: note = MISC_FEATURE - Xaa at position 25 is alpha-methyl-Tyr
  MOD_RES 39: note = Ser at position 39 is amidated

SEQ ID NO: 392 - protein, 39 aa, synthetic construct; identical to SEQ ID NO: 381
  REGION 1..39: note = Synthetic Construct
  SITE 1: note = MISC_FEATURE - Xaa at position 1 is D-Tyr
  SITE 2: note = MISC_FEATURE - Xaa at position 2 is Aib
  SITE 13: note = MISC_FEATURE - Xaa at position 13 is alpha-methyl-Leu
  SITE 16: note = MISC_FEATURE - Xaa at position 16 is Orn
  MOD_RES 17: note = Lys at position 17 is chemically modified by conjugation of the epsilon-amino group of the Lys side chain with (2-[2-(2-amino-ethoxy)-ethoxy]-acetyl)2-(gamma-Glu)-CO-(CH2)16-CO 2H
  SITE 20: note = MISC_FEATURE - Xaa at position 20 is Aib
  SITE 25: note = MISC_FEATURE - Xaa at position 25 is alpha-methyl-Tyr
  MOD_RES 39: note = Ser at position 39 is amidated

SEQ ID NO: 393 - protein, 39 aa, synthetic construct; identical to SEQ ID NO: 305
  REGION 1..39: note = Synthetic Construct
  SITE 1: note = MISC_FEATURE - Xaa at position 1 is D-Tyr
  SITE 2: note = MISC_FEATURE - Xaa at position 2 is Aib
  SITE 13: note = MISC_FEATURE - Xaa at position 13 is alpha-methyl-Leu
  MOD_RES 17: note = Lys at position 17 is chemically modified by conjugation of the epsilon-amino group of the Lys side chain with (2-[2-(2-amino-ethoxy)-ethoxy]-acetyl)-(gamma-Glu)-CO-(CH2)18-CO2 H
  SITE 20: note = MISC_FEATURE - Xaa at position 20 is Aib
  MOD_RES 39: note = Ser at position 39 is amidated

SEQ ID NO: 394 - protein, 39 aa, synthetic construct
  REGION 1..39: note = Synthetic Construct
  SITE 1: note = MISC_FEATURE - Xaa at position 1 is D-Tyr
  SITE 2: note = MISC_FEATURE - Xaa at position 2 is Aib
  SITE 13: note = MISC_FEATURE - Xaa at position 13 is alpha-methyl-Leu
  MOD_RES 17: note = Lys at position 17 is chemically modified by conjugation of the epsilon-amino group of the Lys side chain with (2-[2-(2-amino-ethoxy)-ethoxy]-acetyl)2-(gamma-Glu)-CO-(CH2)18-CO 2H
  SITE 20: note = MISC_FEATURE - Xaa at position 20 is Aib
  SITE 25: note = MISC_FEATURE - Xaa at position 25 is alpha-methyl-Tyr
  MOD_RES 39: note = Ser at position 39 is amidated
XXEGTFTSDYSIXLDKKAQXEFIEXLIEGGPSSGAPPPS

SEQ ID NO: 395 - protein, 39 aa, synthetic construct
  REGION 1..39: note = Synthetic Construct
  SITE 1: note = MISC_FEATURE - Xaa at position 1 is D-Tyr
  SITE 2: note = MISC_FEATURE - Xaa at position 2 is Aib
  SITE 13: note = MISC_FEATURE - Xaa at position 13 is alpha-methyl-Leu
  SITE 16: note = MISC_FEATURE - Xaa at position 16 is Orn
  MOD_RES 17: note = Lys at position 17 is chemically modified by conjugation of the epsilon-amino group of the Lys side chain with (2-[2-(2-amino-ethoxy)-ethoxy]-acetyl)2-(gamma-Glu)-CO-(CH2)18-CO 2H
  SITE 20: note = MISC_FEATURE - Xaa at position 20 is Aib
  SITE 25: note = MISC_FEATURE - Xaa at position 25 is alpha-methyl-Tyr
  MOD_RES 39: note = Ser at position 39 is amidated
XXEGTFTSDYSIXLDXKAQXEFIEXLIEGGPSSGAPPPS

SEQ ID NO: 396 - protein, 39 aa, synthetic construct
  REGION 1..39: note = Synthetic Construct
  SITE 1: note = MISC_FEATURE - Xaa at position 1 is D-Tyr
  SITE 2: note = MISC_FEATURE - Xaa at position 2 is Aib
  SITE 13: note = MISC_FEATURE - Xaa at position 13 is alpha-methyl-Leu
  MOD_RES 17: note = Lys at position 17 is chemically modified by conjugation of the epsilon-amino group of the Lys side chain with (2-[2-(2-amino-ethoxy)-ethoxy]-acetyl)2-(gamma-Glu)-CO-(CH2)18-CO 2H
  SITE 20: note = MISC_FEATURE - Xaa at position 20 is Aib
  SITE 25: note = MISC_FEATURE - Xaa at position 25 is alpha-methyl-Tyr
  MOD_RES 39: note = Ser at position 39 is amidated
XXEGTFTSDYSIXLDEKAQXAFIEXLIAGGPSSGAPPPS